European Patent Application EP 4 610 372 A2, published September 3, 2025. Title: PLANT MICROBIAL PREPARATIONS, COMPOSITIONS AND FORMULATIONS COMPRISING SAME AND USES THEREOF. Applicant: Evogene Ltd. The sequence listing filed with the application follows.

SEQUENCE LISTING (234 sequences)

SEQ ID NO: 1 - DNA, 1431 bp, Bacillus sp.
  misc_feature 1..1431: note = ribosomal RNA nucleic acid sequence
  source 1..1431: mol_type = genomic DNA
ggttactccaccgacttcgggtgttacaaactctcgtggtgtgacgggcggtgtgtacaaggcccgggaacgtattcaccgcggcatgctgatccgcgattactagcgattccagcttcatgtaggcgagttgcagcctacaatccgaactgagaatggttttatgggattggcttgacctcgcggtcttgcagccctttgtaccatccattgtagcacgtgtgtagcccaggtcataaggggcatgatgatttgacgtcatccccaccttcctccggtttgtcaccggcagtcaccttagagtgcccaactaaatgctggcaactaagatcaagggttgcgctcgttgcgggacttaacccaacatctcacgacacgagctgacgacaaccatgcaccacctgtcactctgtcccccgaaggggaacgctctatctctagagttgtcagaggatgtcaagacctggtaaggttcttcgcgttgcttcgaattaaaccacatgctccaccgcttgtgcgggcccccgtcaattcctttgagtttcagtcttgcgaccgtactccccaggcggagtgcttaatgcgttagctgcagcactaaagggcggaaaccctctaacacttagcactcatcgtttacggcgtggactaccagggtatctaatcctgtttgctccccacgctttcgcgcctcagcgtcagttacagaccaaaaagccgccttcgccactggtgttcctccacatctctacgcatttcaccgctacacgtggaattccgcttttctcttctgcactcaagttccccagtttccaatgaccctccacggttgagccgtgggctttcacatcagacttaagaaaccgcctgcgcgcgctttacgcccaataattccggataacgcttgccacctacgtattaccgcggctgctggcacgtagttagccgtggctttctggttaggtaccgtcaaggtacgagcagttactctcgtacttgttcttccctaacaacagagttttacgacccgaaagccttcatcactcacgcggcgttgctccgtcagactttcgtccattgcggaagattccctactgctgcctcccgtaggagtctgggccgtgtctcagtcccagtgtggccgatcaccctctcaggtcggctatgcatcgttgccttggtgagccgttacctcaccaactagctaatgcaccgcgggcccatctgtaagtgatagccgaaaccatctttcaatcatctcccatgaaggagaagatcctatccggtattagcttcggtttcccgaagttatcccagtcttacaggcaggttgcccacgtgttactcacccgtccgccgctaacgtcatagaagcaagcttctaatcagttcgctcgacttgcatgtattaggcacgccgccagcgttcat

SEQ ID NO: 2 - DNA, 1401 bp, Pseudomonas sp.
  misc_feature 398: note = n is a, c, g, or t
  misc_feature 1196: note = n is a, c, g, or t
  misc_feature 1..1401: note = ribosomal RNA nucleic acid sequence
  source 1..1401: mol_type = genomic DNA
agtcgagcggatgacgggagcttgctccttgattcagcggcggacgggtgagtaatgcctaggaatctgcctggtagtgggggacaacgtttcgaaaggaacgctaataccgcatacgtcctacgggagaaagcaggggaccttcgggccttgcgctatcagatgagcctaggtcggattagctagttggtggggtaatggctcaccaaggcgacgatccgtaactggtctgagaggatgatcagtcacactggaactgagacacggtccagactcctacgggaggcagcagtggggaatattggacaatgggcgaaagcctgatccagccatgccgcgtgtgtgaagaaggtcttcggattgtaaagcactttaagttgggaggaagggcagtaagntaataccttgctgttttgacgttaccgacagaataagcaccggctaactctgtgccagcagccgcggtaatacagagggtgcaagcgttaatcggaattactgggcgtaaagcgcgcgtaggtggttcgttaagttggatgtgaaagccccgggctcaacctgggaactgcatccaaaactggcgagctagagtacggtagagggtggtggaatttcctgtgtagcggtgaaatgcgtagatataggaaggaacaccagtggcgaaggcgaccacctggactgatactgacactgaggtgcgaaagcgtggggagcaaacaggattagataccctggtagtccacgccgtaaacgatgtcaactagccgttggaatccttgagattttagtggcgcagctaacgcattaagttgaccgcctggggagtacggccgcaaggttaaaactcaaatgaattgacgggggcccgcacaagcggtggagcatgtggtttaattcgaagcaacgcgaagaaccttaccaggccttgacatgcagagaactttccagagatggattggtgccttcgggaactctgacacaggtgctgcatggctgtcgtcagctcgtgtcgtgagatgttgggttaagtcccgtaacgagcgcaacccttgtccttagttaccagcacgttatggtgggcactctaaggagactgccggtgacaaaccggaggaaggtggggatgacgtcaagtcatcatggcccttacggcctgggctacacacgtgctacaatggtcggtacagagggttgcnaagccgcgaggtggagctaatctcacaaaaccgatcgtagtccggatcgcagtctgcaactcgactgcgtgaagtcggaatcgctagtaatcgcgaatcagaatgtcgcggtgaatacgttcccgggccttgtacacaccgcccgtcacaccatgggagtgggttgcaccagaagtagctagtctaaccttcgggaggacggtac

SEQ ID NO: 3 - DNA, 1520 bp, Pseudomonas sp.
  misc_feature 1..1520: note = ribosomal RNA nucleic acid sequence
  source 1..1520: mol_type = genomic DNA
aagagtttgatcatggctcagattgaacgctggcggcaggcctaacacatgcaagtcgagcggatgacgggagcttgctccttgattcagcggcggacgggtgagtaatgcctaggaatctgcctggtagtgggggacaacgtttcgaaaggaacgctaataccgcatacgtcctacgggagaaagcaggggaccttcgggccttgcgctatcagatgagcctaggtcggattagctagttggtggggtaatggctcaccaaggcgacgatccgtaactggtctgagaggatgatcagtcacactggaactgagacacggtccagactcctacgggaggcagcagtggggaatattggacaatgggcgaaagcctgatccagccatgccgcgtgtgtgaagaaggtcttcggattgtaaagcactttaagttgggaggaagggcagtaagttaataccttgctgttttgacgttaccgacagaataagcaccggctaactctgtgccagcagccgcggtaatacagagggtgcaagcgttaatcggaattactgggcgtaaagcgcgcgtaggtggttcgttaagttggatgtgaaagccccgggctcaacctgggaactgcatccaaaactggcgagctagagtacggtagagggtggtggaatttcctgtgtagcggtgaaatgcgtagatataggaaggaacaccagtggcgaaggcgaccacctggactgatactgacactgaggtgcgaaagcgtggggagcaaacaggattagataccctggtagtccacgccgtaaacgatgtcaactagccgttggaatccttgagattttagtggcgcagctaacgcattaagttgaccgcctggggagtacggccgcaaggttaaaactcaaatgaattgacgggggcccgcacaagcggtggagcatgtggtttaattcgaagcaacgcgaagaaccttaccaggccttgacatgcagagaactttccagagatggattggtgccttcgggaactctgacacaggtgctgcatggctgtcgtcagctcgtgtcgtgagatgttgggttaagtcccgtaacgagcgcaacccttgtccttagttaccagcacgttatggtgggcactctaaggagactgccggtgacaaaccggaggaaggtggggatgacgtcaagtcatcatggcccttacggcctgggctacacacgtgctacaatggtcggtacagagggttgccaagccgcgaggtggagctaatctcacaaaaccgatcgtagtccggatcgcagtctgcaactcgactgcgtgaagtcggaatcgctagtaatcgcgaatcagaatgtcgcggtgaatacgttcccgggccttgtacacaccgcccgtcacaccatgggagtgggttgcaccagaagtagctagtctaaccttcgggaggacggttaccacggtgtgattcatgactggggtgaagtcgtaacaaggtagccgtaggggaacctgcggctgga

SEQ ID NO: 4 - DNA, 1400 bp, Acinetobacter sp.
  misc_feature 378: note = n is a, c, g, or t
  misc_feature 1..1400: note = ribosomal RNA nucleic acid sequence
  source 1..1400: mol_type = genomic DNA
agtcgagcggagtgatggtgcttgcactatcacttagcggcggacgggtgagtaatgcttaggaatctgcctattagtgggggacaacatttcgaaaggaatgctaataccgcatacgtcctacgggagaaagcaggggatcttcggaccttgcgctaatagatgagcctaagtcggattagctagttggtggggtaaaggcctaccaaggcgacgatctgtagcgggtctgagaggatgatccgccacactgggactgagacacggcccagactcctacgggaggcagcagtggggaatattggacaatgggcgcaagcctgatccagccatgccgcgtgtgtgaagaaggccttatggttgtaaagcactttaagngaggaggaggctactgaagttaataccttcagatagtggacgttactcgcagaataagcaccggctaactctgtgccagcagccgcggtaatacagagggtgcaagcgttaatcggatttactgggcgtaaagcgcgcgtaggcggctaattaagtcaaatgtgaaatccccgagcttaacttgggaattgcattcgatactggttagctagagtgtgggagaggatggtagaattccaggtgtagcggtgaaatgcgtagagatctggaggaataccgatggcgaaggcagccatctggcctaacactgacgctgaggtgcgaaagcatggggagcaaacaggattagataccctggtagtccatgccgtaaacgatgtctactagccgttggggcctttgaggctttagtggcgcagctaacgcgataagtagaccgcctggggagtacggtcgcaagactaaaactcaaatgaattgacgggggcccgcacaagcggtggagcatgtggtttaattcgatgcaacgcgaagaaccttacctggccttgacatagtaagaactttccagagatggattggtgccttcgggaacttacatacaggtgctgcatggctgtcgtcagctcgtgtcgtgagatgttgggttaagtcccgcaacgagcgcaacccttttccttatttgccagcgagtaatgtcgggaactttaaggatactgccagtgacaaactggaggaaggcggggacgacgtcaagtcatcatggcccttacggccagggctacacacgtgctacaatggtcggtacaaagggttgctacctagcgataggatgctaatctcaaaaagccgatcgtagtccggattggagtctgcaactcgactccatgaagtcggaatcgctagtaatcgcggatcagaatgccgcggtgaatacgttcccgggccttgtacacaccgcccgtcacaccatgggagtttgttgcaccagaagtaggtagtctaaccgcaaggaggacgct

SEQ ID NO: 5 - DNA, 1432 bp, Microbacterium sp.
  misc_feature 1..1432: note = ribosomal RNA nucleic acid sequence
  source 1..1432: mol_type = genomic DNA
caccttcgacggctccctccacaagggttgggccaccggcttcaggtgttaccgactttcatgacttgacgggcggtgtgtacaagacccgggaacgtattcaccgcagcgttgctgatctgcgattactagcgactccgacttcatgaggtcgagttgcagacctcaatccgaactgggaccggctttttgggattcgctccacctcacggtattgcagccctttgtaccggccattgtagcatgcgtgaagcccaagacataaggggcatgatgatttgacgtcatccccaccttcctccgagttgaccccggcagtatcccatgagttcccaccattacgtgctggcaacatagaacgagggttgcgctcgttgcgggacttaacccaacatctcacgacacgagctgacgacaaccatgcaccacctgtatagagaccttgcggggcgactgtttccagacgtttcctctatatgtcaagccttggtaaggttcttcgcgttgcatcgaattaatccgcatgctccgccgcttgtgcgggtccccgtcaattcctttgagttttagccttgcggccgtactccccaggcggggaacttaatgcgttagctgcgtcacggaatccgtggaatggaccccacaactagttcccaacgtttacggggtggactaccagggtatctaagcctgtttgctccccaccctttcgctcctcagcgtcagttacggcccagagatctgccttcgccatcggtgttcctcctgatatctgcgcattccaccgctacaccaggaattccaatctcccctaccgcactctagtctgcccgtacccactgcaggcccgaggttgagcctcgggttttcacagcagacgcgacagaccgcctacgagctctttacgcccaataattccggataacgcttgcgccctacgtattaccgcggctgctggcacgtagttagccggcgctttttctgcaggtaccgtcactttcgcttcttccctgctaaaagaggtttacaacccgaaggccgtcatccctcacgcggcgttgctgcatcaggctttcgcccattgtgcaatattccccactgctgcctcccgtaggagtctgggccgtgtctcagtcccagtgtggccggtcaccctctcaggccggctacccgtcgacgccttggtgagccattacctcaccaacaagctgataggccgcgagctcatccctgaccgaaattctttccagctactgaccatgcggtcgcagctcgtatccggtattagacgccgtttccagcgcttatcccagagtcaggggcagattgctcacgtgttactcacccgttcgccactgatccacagagcaagctctgcttcaccgttcgacttgcatgtgttaagcacgccgccagcgttcatcctgagcca

SEQ ID NO: 6 - DNA, 1502 bp, Microbacterium sp.
  misc_feature 1..1502: note = ribosomal RNA nucleic acid sequence
  source 1..1502: mol_type = genomic DNA
agagtttgatcctggctcaggatgaacgctggcggcgtgcttaacacatgcaagtcgaacggtgaagcagagcttgctctgtggatcagtggcgaacgggtgagtaacacgtgagcaatctgcccctgactctgggataagcgctggaaacggcgtctaataccggatacgagctgcgaccgcatggtcagtagctggaaagaatttcggtcagggatgagctcgcggcctatcagcttgttggtgaggtaatggctcaccaaggcgtcgacgggtagccggcctgagagggtgaccggccacactgggactgagacacggcccagactcctacgggaggcagcagtggggaatattgcacaatgggcgaaagcctgatgcagcaacgccgcgtgagggatgacggccttcgggttgtaaacctcttttagcagggaagaagcgaaagtgacggtacctgcagaaaaagcgccggctaactacgtgccagcagccgcggtaatacgtagggcgcaagcgttatccggaattattgggcgtaaagagctcgtaggcggtctgtcgcgtctgctgtgaaaacccgaggctcaacctcgggcctgcagtgggtacgggcagactagagtgcggtaggggagattggaattcctggtgtagcggtggaatgcgcagatatcaggaggaacaccgatggcgaaggcagatctctgggccgtaactgacgctgaggagcgaaagggtggggagcaaacaggcttagataccctggtagtccaccccgtaaacgttgggaactagttgtggggtccattccacggattccgtgacgcagctaacgcattaagttccccgcctggggagtacggccgcaaggctaaaactcaaaggaattgacggggacccgcacaagcggcggagcatgcggattaattcgatgcaacgcgaagaaccttaccaaggcttgacatatagaggaaacgtctggaaacagtcgccccgcaaggtctctatacaggtggtgcatggttgtcgtcagctcgtgtcgtgagatgttgggttaagtcccgcaacgagcgcaaccctcgttctatgttgccagcacgtaatggtgggaactcatgggatactgccggggtcaactcggaggaaggtggggatgacgtcaaatcatcatgccccttatgtcttgggcttcacgcatgctacaatggccggtacaaagggctgcaataccgtgaggtggagcgaatcccaaaaagccggtcccagttcggattgaggtctgcaactcgacctcatgaagtcggagtcgctagtaatcgcagatcagcaacgctgcggtgaatacgttcccgggtcttgtacacaccgcccgtcaagtcatgaaagtcggtaacacctgaagccggtggcccaacccttgtggagggagccgtcgaaggtgggatcggtaattaggactaagtcgtaacaaggtagccgtaccggaaggtgcggctgga

SEQ ID NO: 7 - DNA, 1527 bp, Pseudoxanthomonas sp.
  misc_feature 1..1527: note = ribosomal RNA nucleic acid sequence
  source 1..1527: mol_type = genomic DNA
aagagtttgatcctggctcagagtgaacgctggcggtaggcctaacacatgcaagtcgaacggcagcacaggagagcttgctctctgggtggcgagtggcggacgggtgaggaatacatcggaatctaccttttcgtgggggataacgtagggaaacttacgctaataccgcatacgacctacgggtgaaagtgggggaccgcaaggcctcacgcgattagatgagccgatgtccgattagctagttggcggggtaatggcccaccaaggcgacgatcggtagctggtctgagaggatgatcagccacactggaactgagacacggtccagactcctacgggaggcagcagtggggaatattggacaatgggcgcaagcctgatccagccataccgcgtgggtgaagaaggccttcgggttgtaaagcccttttgttgggaaagaaatcctgtcgattaatactcggtggggatgacggtacccaaagaataagcaccggctaacttcgtgccagcagccgcggtaatacgaagggtgcaagcgttactcggaattactgggcgtaaagcgtgcgtaggtggtggtttaagtctgctgtgaaagccctgggctcaacctgggaattgcagtggatactggatcactagagtgtggtagagggatgcggaatttctggtgtagcagtgaaatgcgtagagatcagaaggaacatccgtggcgaaggcggcatcctgggccaacactgacactgaggcacgaaagcgtggggagcaaacaggattagataccctggtagtccacgccctaaacgatgcgaactggatgttgggtgcaacttggcacccagtatcgaagctaacgcgttaagttcgccgcctggggagtacggtcgcaagactgaaactcaaaggaattgacgggggcccgcacaagcggtggagtatgtggtttaattcgatgcaacgcgaagaaccttacctggtcttgacatccacggaactttccagagatggattggtgccttcgggaaccgtgagacaggtgctgcatggctgtcgtcagctcgtgtcgtgagatgttgggttaagtcccgcaacgagcgcaacccttgtccttagttgccagcacgtaatggtgggaactctaaggagaccgccggtgacaaaccggaggaaggtggggatgacgtcaagtcatcatggcccttacgaccagggctacacacgtactacaatggttaggacagagggctgcaaacccgcgagggtgagccaatcccagaaaccctatctcagtccggattggagtctgcaactcgactccatgaagtcggaatcgctagtaatcgcagatcagcattgctgcggtgaatacgttcccgggccttgtacacaccgcccgtcacaccatgggagtttgttgcaccagaagcaggtagcttaaccttcgggagggcgcttgccacggtgtggccgatgactggggtgaagtcgtaacaaggtagccgtatcggaaggtgcggctgg

SEQ ID NO: 8 - DNA, 1500 bp, Chryseobacterium sp.
  misc_feature 1..1500: note = ribosomal RNA nucleic acid sequence
  source 1..1500: mol_type = genomic DNA
gagagtttgatcctggctcaggatgaacgctagcgggaggcctaacacatgcaagccgagcggtagagattcttcggaatcttgagagcggcgcacgggtgcggaacacgtgtgcaacctgcctttatcaggggaatagcctttcgaaaggaagattaatgccccataatatattttctggcatcagaatatattgaaaactccggtggataaagatgggcacgcgcaggattagatagttggtagggtaacggcctaccaagtcaacgatccttagggggcctgagagggtgatcccccacactggtactgagacacggaccagactcctacgggaggcagcagtgaggaatattggacaatgggtgagagcctgatccagccatcccgcgtgaaggacgacggccctatgggttgtaaacttcttttgtacagggataaacctttccacgtgtgggaagctgaaggtactgtacgaataagcaccggctaactccgtgccagcagccgcggtaatacggagggtgcaagcgttatccggatttattgggtttaaagggtccgtaggcggactcgtaagtcagtggtgaaatctcacagcttaactgtgaaactgccattgatactgcgggtcttgagtgttgttgaagtagctggaataagtagtgtagcggtgaaatgcatagatattacttagaacaccaattgcgaaggcaggttactaagcaacaactgacgctgatggacgaaagcgtggggagcgaacaggattagataccctggtagtccacgccgtaaacgatgctaactcgtttttgggtctttaagattcagagactaagcgaaagtgataagttagccacctggggagtacgttcgcaagaatgaaactcaaaggaattgacgggggcccgcacaagcggtggattatgtggtttaattcgatgatacgcgaggaaccttaccaaggcttaaatgggaattgattggtttagaaatagaccgtccttcgggcaattttcaaggtgctgcatggttgtcgtcagctcgtgccgtgaggtgttaggttaagtcctgcaacgagcgcaacccctgtcactagttgccatcattcagttggggactctagtgagactgcctacgcaagtagagaggaaggtggggatgacgtcaaatcatcacggcccttacgccttgggccacacacgtaatacaatggccggtacagagggcagctacacagcgatgtgatgcaaatctcgaaagccggtctcagttcggattggagtctgcaactcgactctatgaagctggaatcgctagtaatcgcgcatcagccatggcgcggtgaatacgttcccgggccttgtacacaccgcccgtcaagccatggaagtctggggtacctgaagtcggtgaccgtaacaggagctgcctagggtaaaacaggtaactagggctaagtcgtaacaaggtagccgtaccggaaggtgcggctgg

SEQ ID NO: 9 - DNA, 1523 bp, Erwinia sp.
  misc_feature 1..1523: note = ribosomal RNA nucleic acid sequence
  source 1..1523: mol_type = genomic DNA
agagtttgatcatggctcagattgaacgctggcggcaggcctaacacatgcaagtcgaacggtagcacagagagcttgctcttgggtgacgagtggcggacgggtgagtaatgtctgggaaactgcccgatggagggggataactactggaaacggtagctaataccgcataacgtcttcggaccaaagtgggggaccttcgggcctcacaccatcggatgtgcccagatgggattagctagtaggtggggtaacggctcacctaggcgacgatccctagctggtctgagaggatgaccagccacactggaactgagacacggtccagactcctacgggaggcagcagtggggaatattgcacaatgggcgcaagcctgatgcagccatgccgcgtgtatgaagaaggccttcgggttgtaaagtactttcagtggggaggaaggcgaagaggttaataaccttttcgattgacgttacccgcagaagaagcaccggctaactccgtgccagcagccgcggtaatacggagggtgcaagcgttaatcggaattactgggcgtaaagcgcacgcaggcggtctgtcaagtcggatgtgaaatccccgggctcaacctgggaactgcattcgaaactggcaggctagagtcttgtagaggggggtagaattccaggtgtagcggtgaaatgcgtagagatctggaggaataccggtggcgaaggcggccccctggacaaagactgacgctcaggtgcgaaagcgtggggagcaaacaggattagataccctggtagtccacgccgtaaacgatgtcgacttggaggttgtgcccttgaggcgtggcttccggagctaacgcgttaagtcgaccgcctggggagtacggccgcaaggttaaaactcaaatgaattgacgggggcccgcacaagcggtggagcatgtggtttaattcgatgcaacgcgaagaaccttacctggccttgacatccacggaattcggcagagatgccttagtgccttcgggaaccgtgagacaggtgctgcatggctgtcgtcagctcgtgttgtgaaatgttgggttaagtcccgcaacgagcgcaacccttatcctttgttgccagcacgtaatggtgggaactcaaaggagactgccggtgataaaccggaggaaggtggggatgacgtcaagtcatcatggcccttacggccagggctacacacgtgctacaatggcgcatacaaagagaagcgacctcgcgagagcaagcggacctcataaagtgcgtcgtagtccggatcggagtctgcaactcgactccgtgaagtcggaatcgctagtaatcgtagatcagaatgctacggtgaatacgttcccgggccttgtacacaccgcccgtcacaccatgggagtgggttgcaaaagaagtaggtagcttaaccttcgggagggcgcttaccactttgtgattcatgactggggtgaagtcgtaacaaggtaaccgtaggggaacctgcggttgga

SEQ ID NO: 10 - DNA, 1406 bp, Erwinia sp.
  misc_feature 446: note = n is a, c, g, or t
  misc_feature 448..449: note = n is a, c, g, or t
  misc_feature 457: note = n is a, c, g, or t
  misc_feature 459: note = n is a, c, g, or t
  misc_feature 461..462: note = n is a, c, g, or t
  misc_feature 1121..1122: note = n is a, c, g, or t
  misc_feature 1125: note = n is a, c, g, or t
  misc_feature 1129..1130: note = n is a, c, g, or t
  misc_feature 1..1406: note = ribosomal RNA nucleic acid sequence
  source 1..1406: mol_type = genomic DNA
tttgattcatggctcagattgaacgctggcggcaggcctaacacatgcaagtcgaacggtagcacagagagcttgctcttgggtgacgagtggcggacgggtgagtaatgtctgggaaactgcccgatggagggggataactactggaaacggtagctaataccgcataacgtcttcggaccaaagtgggggaccttcgggcctcacaccatcggatgtgcccagatgggattagctagtaggtggggtaacggctcacctaggcgacgatccctagctggtctgagaggatgaccagccacactggaactgagacacggtccagactcctacgggaggcagcagtggggaatattgcacaatgggcgcaagcctgatgcagccatgccgcgtgtatgaagaaggccttcgggttgtaaagtactttcagtggggaggaaggcgangnngttaatancntnntcgattgacgttacccgcagaagaagcaccggctaactccgtgccagcagccgcggtaatacggagggtgcaagcgttaatcggaattactgggcgtaaagcgcacgcaggcggtctgtcaagtcggatgtgaaatccccgggctcaacctgggaactgcattcgaaactggcaggctagagtcttgtagaggggggtagaattccaggtgtagcggtgaaatgcgtagagatctggaggaataccggtggcgaaggcggccccctggacaaagactgacgctcaggtgcgaaagcgtggggagcaaacaggattagataccctggtagtccacgccgtaaacgatgtcgacttggaggttgtgcccttgaggcgtggcttccggagctaacgcgttaagtcgaccgcctggggagtacggccgcaaggttaaaactcaaatgaattgacgggggcccgcacaagcggtggagcatgtggtttaattcgatgcaacgcgaagaaccttacctggccttgacatccacggaattcggcagagatgccttagtgccttcgggaaccgtgagacaggtgctgcatggctgtcgtcagctcgtgttgtgaaatgttgggttaagtcccgcaacgagcgcaacccttatcctttgttgccagcnngtnatgnngggaactcaaaggagactgccggtgataaaccggaggaaggtggggatgacgtcaagtcatcatggcccttacggccagggctacacacgtgctacaatggcgcatacaaagagaagcgacctcgcgagagcaagcggacctcataaagtgcgtcgtagtccggatcggagtctgcaactcgactccgtgaagtcggaatcgctagtaatcgtagatcagaatgctacggtgaatacgttcccgggccttgtacacaccgcccgtcacaccatggg

SEQ ID NO: 11 - DNA, 1520 bp, Pseudomonas sp.
  misc_feature 1..1520: note = ribosomal RNA nucleic acid sequence
  source 1..1520: mol_type = genomic DNA
aagagtttgatcatggctcagattgaacgctggcggcaggcctaacacatgcaagtcgagcggatgacgggagcttgctccttgattcagcggcggacgggtgagtaatgcctaggaatctgcctggtagtgggggacaacgtttcgaaaggaacgctaataccgcatacgtcctacgggagaaagcaggggaccttcgggccttgcgctatcagatgagcctaggtcggattagctagttggtgaggtaatggctcaccaaggcgacgatccgtaactggtctgagaggatgatcagtcacactggaactgagacacggtccagactcctacgggaggcagcagtggggaatattggacaatgggcgaaagcctgatccagccatgccgcgtgtgtgaagaaggtcttcggattgtaaagcactttaagttgggaggaagggcagtaagttaataccttgctgttttgacgttaccgacagaataagcaccggctaactctgtgccagcagccgcggtaatacagagggtgcaagcgttaatcggaattactgggcgtaaagcgcgcgtaggtggttcgttaagttggatgtgaaagccccgggctcaacctgggaactgcatccaaaactggcgagctagagtacggtagagggtggtggaatttcctgtgtagcggtgaaatgcgtagatataggaaggaacaccagtggcgaaggcgaccacctggactgatactgacactgaggtgcgaaagcgtggggagcaaacaggattagataccctggtagtccacgccgtaaacgatgtcaactagccgttggaatccttgagattttagtggcgcagctaacgcattaagttgaccgcctggggagtacggccgcaaggttaaaactcaaatgaattgacgggggcccgcacaagcggtggagcatgtggtttaattcgaagcaacgcgaagaaccttaccaggccttgacatgcagagaactttccagagatggattggtgccttcgggaactctgacacaggtgctgcatggctgtcgtcagctcgtgtcgtgagatgttgggttaagtcccgtaacgagcgcaacccttgtccttagttaccagcacgttatggtgggcactctaaggagactgccggtgacaaaccggaggaaggtggggatgacgtcaagtcatcatggcccttacggcctgggctacacacgtgctacaatggtcggtacagagggttgccaagccgcgaggtggagctaatctcacaaaaccgatcgtagtccggatcgcagtctgcaactcgactgcgtgaagtcggaatcgctagtaatcgcgaatcagaatgtcgcggtgaatacgttcccgggccttgtacacaccgcccgtcacaccatgggagtgggttgcaccagaagtagctagtctaaccttcgggaggacggttaccacggtgtgattcatgactggggtgaagtcgtaacaaggtagccgtaggggaacctgcggctgga

SEQ ID NO: 12 - DNA, 1520 bp, Pseudomonas sp.
  misc_feature 1..1520: note = ribosomal RNA nucleic acid sequence
  source 1..1520: mol_type = genomic DNA
aagagtttgatcatggctcagattgaacgctggcggcaggcctaacacatgcaagtcgagcggtagagggtagcttgctactcttgagagcggcggacgggtgagtaatgcctaggaatctgcctagtggtgggggataacgttcggaaacggacgctaataccgcatacgtcctacgggagaaagcgggggaccttcgggcctcgcgccattagatgagcctaggtcggattagctagttggtgaggtaaaggctcaccaaggcgacgatccgtaactggtctgagaggatgatcagtcacactggaactgagacacggtccagactcctacgggaggcagcagtggggaatattggacaatgggcgaaagcctgatccagccatgccgcgtgtgtgaagaaggtcttcggattgtaaagcactttaagttgggaggaagggtagtaacttaatacgttgctattttgacgttaccgacagaataagcaccggctaactctgtgccagcagccgcggtaatacagagggtgcaagcgttaatcggaattactgggcgtaaagcgcgcgtaggtggtttgttaagttggatgtgaaagccccgggctcaacctgggaactgcatccaaaactggcaagctagagtacggtagagggtggtggaatttcctgtgtagcggtgaaatgcgtagatataggaaggaacaccagtggcgaaggcgaccacctggactgatactgacactgaggtgcgaaagcgtggggagcaaacaggattagataccctggtagtccacgccgtaaacgatgtcaactagccgttggattccttgagaatttagtggcgcagctaacgcattaagttgaccgcctggggagtacggccgcaaggttaaaactcaaatgaattgacgggggcccgcacaagcggtggagcatgtggtttaattcgaagcaacgcgaagaaccttacctggccttgacatgctgagaactttccagagatggattggtgccttcgggaactcagacacaggtgctgcatggctgtcgtcagctcgtgtcgtgagatgttgggttaagtcccgtaacgagcgcaacccttgtccttagttaccagcacgttatggtgggaactctaaggagactgccggtgacaaaccggaggaaggtggggatgacgtcaagtcatcatggcccttacggccagggctacacacgtgctacaatggtcggtacaaagggttgccaagccgcgaggtggagctaatcccataaaaccgatcgtagtccggatcgcagtctgcaactcgactgcgtgaagtcggaatcgctagtaatcgtgaatcagaatgtcacggtgaatacgttcccgggccttgtacacaccgcccgtcacaccatgggagtgggttgcaccagaagtagctagtctaaccttcggggggacggttaccacggtgtgattcatgactggggtgaagtcgtaacaaggtagccgtaggggaacctgcggctgga

SEQ ID NO: 13 - DNA, 1405 bp, Pseudomonas sp.
  misc_feature 1..1405: note = ribosomal RNA nucleic acid sequence
  source 1..1405: mol_type = genomic DNA
tgcagtcgagcggtagagggtagcttgctactcttgagagcggcggacgggtgagtaatgcctaggaatctgcctagtggtgggggataacgttcggaaacggacgctaataccgcatacgtcctacgggagaaagcgggggaccttcgggcctcgcgccattagatgagcctaggtcggattagctagttggtgaggtaaaggctcaccaaggcgacgatccgtaactggtctgagaggatgatcagtcacactggaactgagacacggtccagactcctacgggaggcagcagtggggaatattggacaatgggcgaaagcctgatccagccatgccgcgtgtgtgaagaaggtcttcggattgtaaagcactttaagttgggaggaagggtagtaacttaatacgttgctattttgacgttaccgacagaataagcaccggctaactctgtgccagcagccgcggtaatacagagggtgcaagcgttaatcggaattactgggcgtaaagcgcgcgtaggtggtttgttaagttggatgtgaaagccccgggctcaacctgggaactgcatccaaaactggcaagctagagtacggtagagggtggtggaatttcctgtgtagcggtgaaatgcgtagatataggaaggaacaccagtggcgaaggcgaccacctggactgatactgacactgaggtgcgaaagcgtggggagcaaacaggattagataccctggtagtccacgccgtaaacgatgtcaactagccgttggattccttgagaatttagtggcgcagctaacgcattaagttgaccgcctggggagtacggccgcaaggttaaaactcaaatgaattgacgggggcccgcacaagcggtggagcatgtggtttaattcgaagcaacgcgaagaaccttacctggccttgacatgctgagaactttccagagatggattggtgccttcgggaactcagacacaggtgctgcatggctgtcgtcagctcgtgtcgtgagatgttgggttaagtcccgtaacgagcgcaacccttgtccttagttaccagcacgttatggtgggaactctaaggagactgccggtgacaaaccggaggaaggtggggatgacgtcaagtcatcatggcccttacggccagggctacacacgtgctacaatggtcggtacaaagggttgccaagccgcgaggtggagctaatcccataaaaccgatcgtagtccggatcgcagtctgcaactcgactgcgtgaagtcggaatcgctagtaatcgtgaatcagaatgtcacggtgaatacgttcccgggccttgtacacaccgcccgtcacaccatgggagtgggttgcaccagaagtagctagtctaacctttcgggggggacggta

SEQ ID NO: 14 - DNA, 1510 bp, Arthrobacter sp.
  misc_feature 1..1510: note = ribosomal RNA nucleic acid sequence
  source 1..1510: mol_type = genomic DNA
ggagagtttgatcctggctcaggatgaacgctggcggcgtgcttaacacatgcaagtcgaacgatgatccggtgcttgcaccggggattagtggcgaacgggtgagtaacacgtgagtaacctgcccttaactctgggataagcctgggaaactgggtctaataccggatatgactgaccgtcgcatggtggttggtggaaagctttattgtggttttggatggactcgcggcctatcagcttgttggtgaggtaatggcttaccaaggcgacgacgggtagccggcctgagagggtgaccggccacactgggactgagacacggcccagactcctacgggaggcagcagtggggaatattgcacaatgggcgcaagcctgatgcagcgacgccgcgtgagggatgacggccttcgggttgtaaacctctttcagtagggaagaagcgaaagtgacggtacctgcagaagaagcgccggctaactacgtgccagcagccgcggtaatacgtagggcgcaagcgttatccggaattattgggcgtaaagagctcgtaggcggtttgtcgcgtctgccgtgaaagtccggggctcaactccggatctgcggtgggtacgggcagactagagtgatgtaggggagactggaattcctggtgtagcggtgaaatgcgcagatatcaggaggaacaccgatggcgaaggcaggtctctgggcattaactgacgctgaggagcgaaagcatggggagcgaacaggattagataccctggtagtccatgccgtaaacgttgggcactaggtgtgggggacattccacgttttccgcgccgtagctaacgcattaagtgccccgcctggggagtacggccgcaaggctaaaactcaaaggaattgacgggggcccgcacaagcggcggagcatgcggattaattcgatgcaacgcgaagaaccttaccaaggcttgacatggaccggaccgccgcagagatgtggtttcccctttggggctggttcacaggtggtgcatggttgtcgtcagctcgtgtcgtgagatgttgggttaagtcccgcaacgagcgcaaccctcgttctatgttgccagcacgtgatggtggggactcataggagactgccggggtcaactcggaggaaggtggggacgacgtcaaatcatcatgccccttatgtcttgggcttcacgcatgctacaatggccggtacaaagggttgcgatactgtgaggtggagctaatcccaaaaagccggtctcagttcggattggggtctgcaactcgaccccatgaagtcggagtcgctagtaatcgcagatcagcaacgctgcggtgaatacgttcccgggccttgtacacaccgcccgtcaagtcacgaaagttggtaacacccgaagccggtggcctaaccccttgtgggagggagctgtcgaaggtgggactggcgattgggactaagtcgtaacaaggtagccgtaccggaaggtgcggctgg

SEQ ID NO: 15 - DNA, 1509 bp, Kocuria sp.
  misc_feature 1..1509: note = ribosomal RNA nucleic acid sequence
  source 1..1509: mol_type = genomic DNA
agagtttgatcctggctcaggacgaacgctggcggcgtgcttaacacatgcaagtcgaacgctgaagcaccagcttgctggtgtggatgagtggcgaacgggtgagtaatacgtgagtaacctgcccttgactctgggataagcccgggaaactgggtctaatactggatgctacatgtcaccgcatggtggtgtgtggaaagggtttactggtcttggatgggctcacggcctatcagcttgttggtgaggtaatggctcaccaaggcgacgacgggtagccggcctgagagggtgaccggccacactgggactgagacacggcccagactcctacgggaggcagcagtggggaatattgcacaatgggcgaaagcctgatgcagcgacgccgcgtgagggatgacggccttcgggttgtaaacctctttcagcagggaagaagccacaagtgacggtacctgcagaagaagcgccggctaactacgtgccagcagccgcggtaatacgtagggcgcaagcgttgtccggaattattgggcgtaaagagctcgtaggcggtttgtcgcgtctgctgtgaaagcccggggcttaaccccgggtgtgcagtgggtacgggcagactagagtgcagtaggggagactggaattcctggtgtagcggtggaatgcgcagatatcaggaggaacaccgatggcgaaggcaggtctctgggctgttactgacgctgaggagcgaaagcatggggagcgaacaggattagataccctggtagtccatgccgtaaacgttgggcactaggtgtgggggacattccacgttttccgcgccgtagctaacgcattaagtgccccgcctggggagtacggccgcaaggctaaaactcaaaggaattgacgggggcccgcacaagcggcggagcatgcggattaattcgatgcaacgcgaagaaccttaccaaggcttgacatataccggatcgttccagagatggttcttcccctttggggtcggtatacaggtggtgcatggttgtcgtcagctcgtgtcgtgagatgttgggttaagtcccgcaacgagcgcaaccctcgttccatgttgccagcacgtgatggtggggactcatgggagactgccggggtcaactcggaggaaggtggggatgacgtcaaatcatcatgccccttatgtcttgggcttcacgcatgctacaatggccggtacaaagggttgcgatactgtgaggtggagctaatcccaaaaagccggtctcagttcggattgaggtctgcaactcgacctcatgaagtcggagtcgctagtaatcgcagatcagcaacgctgcggtgaatacgttcccgggccttgtacacaccgcccgtcaagtcacgaaagtcggtaacacccgaagccggtggcccaacccttgtggagggagccgtcgaaggtgggactggcgattgggactaagtcgtaacaaggtagccgtaccggaaggtgcggctgga

SEQ ID NO: 16 - DNA, 1371 bp, Pseudomonas sp.
  misc_feature 1..1371: note = ribosomal RNA nucleic acid sequence
  source 1..1371: mol_type = genomic DNA
aggagcttgctcctggattcagcggcggacgggtgagtaatgcctaggaatctgcctggtagtgggggacaacgtttcgaaaggaacgctaataccgcatacgtcctacgggagaaagcaggggaccttcgggccttgcgctatcagatgagcctaggtcggattagctagttggtgaggtaatggctcaccaaggcgacgatccgtaactggtctgagaggatgatcagtcacactggaactgagacacggtccagactcctacgggaggcagcagtggggaatattggacaatgggcgaaagcctgatccagccatgccgcgtgtgtgaagaaggtcttcggattgtaaagcactttaagttgggaggaagggcagtaaattaatactttgctgttttgacgttaccgacagaataagcaccggctaactctgtgccagcagccgcggtaatacagagggtgcaagcgttaatcggaattactgggcgtaaagcgcgcgtaggtggtttgttaagttggatgtgaaatccccgggctcaacctgggaactgcatccaaaactggcaagctagagtatggtagagggtggtggaatttcctgtgtagcggtgaaatgcgtagatataggaaggaacaccagtggcgaaggcgaccacctggactgatactgacactgaggtgcgaaagcgtggggagcaaacaggattagataccctggtagtccacgccgtaaacgatgtcaactagccgttgggagccttgagctcttagtggcgcagctaacgcattaagttgaccgcctggggagtacggccgcaaggttaaaactcaaatgaattgacgggggcccgcacaagcggtggagcatgtggtttaattcgaagcaacgcgaagaaccttaccaggccttgacatccaatgaactttccagagatggattggtgccttcgggaacattgagacaggtgctgcatggctgtcgtcagctcgtgtcgtgagatgttgggttaagtcccgtaacgagcgcaacccttgtccttagttaccagcacgtaatggtgggcactctaaggagactgccggtgacaaaccggaggaaggtggggatgacgtcaagtcatcatggcccttacggcctgggctacacacgtgctacaatggtcggtacaaagggttgccaagccgcgaggtggagctaatcccataaaaccgatcgtagtccggatcgcagtctgcaactcgactgcgtgaagtcggaatcgctagtaatcgcgaatcagaatgtcgcggtgaatacgttcccgggccttgtacacaccgcccgtcacaccatgggagtgggttgcaccagaagtagctagtctaacct

SEQ ID NO: 17 - DNA, 1524 bp, Erwinia sp.
  misc_feature 1..1524: note = ribosomal RNA nucleic acid sequence
  source 1..1524: mol_type = genomic DNA
agagtttgatcatggctcagattgaacgctggcggcaggcctaacacatgcaagtcgaacggtagcacagaggagcttgctcctcgggtgacgagtggcggacgggtgagtaatgtctggggatctgcccgatggagggggataaccactggaaacggtggctaataccgcataacgtcgcaagaccaaagtgggggaccttcgggcctcacaccatcggatgaacccagatgggattagctagtaggtggggtaacggctcacctaggcgacgatccctagctggtctgagaggatgaccagccacactggaactgagacacggtccagactcctacgggaggcagcagtggggaatattgcacaatgggcgcaagcctgatgcagccatgccgcgtgtatgaagaaggccttcgggttgtaaagtactttcagcggggaggaaggggatgaggttaataacctcgttcattgacgttacccgcagaagaagcaccggctaactccgtgccagcagccgcggtaatacggagggtgcaagcgttaatcggaattactgggcgtaaagcgcacgcaggcggtctgttaagtcagatgtgaaatccccgggcttaacctgggaactgcatttgaaactggcaggcttgagtcttgtagaggggggtagaattccaggtgtagcggtgaaatgcgtagagatctggaggaataccggtggcgaaggcggccccctggacaaagactgacgctcaggtgcgaaagcgtggggagcaaacaggattagataccctggtagtccacgccgtaaacgatgtcgacttggaggctgtgagcatgactcgtggcttccggagctaacgcgttaagtcgaccgcctggggagtacggccgcaaggttaaaactcaaatgaattgacgggggcccgcacaagcggtggagcatgtggtttaattcgatgcaacgcgaagaaccttacctgctcttgacatccacggaattcggcagagatgccttagtgccttcgggaaccgtgagacaggtgctgcatggctgtcgtcagctcgtgttgtgaaatgttgggttaagtcccgcaacgagcgcaacccttatcctttgttgccagcgattcggtcgggaactcaaaggagactgccggtgataaaccggaggaaggtggggatgacgtcaagtcatcatggcccttacgagcagggctacacacgtgctacaatggcgcatacaaagagaagcgacctcgcgagagcaagcggacctcacaaagtgcgtcgtagtccggatcggagtctgcaactcgactccgtgaagtcggaatcgctagtaatcgtggatcagaatgccacggtgaatacgttcccgggccttgtacacaccgcccgtcacaccatgggagtgggttgcaaaagaagtaggtagcttaaccttcgggagggcgcttaccactttgtgattcatgactggggtgaagtcgtaacaaggtaaccgtaggggaacctgcggttgga

SEQ ID NO: 18 - DNA, 1383 bp, Paraburkholderia sp.
  misc_feature 1..1383: note = ribosomal RNA nucleic acid sequence
  source 1..1383: mol_type = genomic DNA
ggcagcacgggggcaaccctggtggcgagtggcgaacgggtgagtaatacatcggaacgtgtcctgtagtgggggatagcccggcgaaagccggattaataccgcatacgatctgtggatgaaagcgggggatccttcgggacctcgcgctacaggggcggccgatggcagattagctagttggtggggtaaaggcctaccaaggcgacgatctgtagctggtctgagaggacgaccagccacactgggactgagacacggcccagactcctacgggaggcagcagtggggaattttggacaatgggcgaaagcctgatccagcaatgccgcgtgtgtgaagaaggccttcgggttgtaaagcacttttgtccggaaagaaaacctcgtggttaatacccgtgggggatgacggtaccggaagaataagcaccggctaactacgtgccagcagccgcggtaatacgtagggtgcaagcgttaatcggaattactgggcgtaaagcgtgcgcaggcggtccgctaagacagatgtgaaatccccgggcttaacctgggaactgcatttgtgactggcgggctagagtatggcagaggggggtagaattccacgtgtagcagtgaaatgcgtagagatgtggaggaataccgatggcgaaggcagccccctgggccaatactgacgctcatgcacgaaagcgtggggagcaaacaggattagataccctggtagtccacgccctaaacgatgtcaactagttgttggggattcatttccttagtaacgtagctaacgcgtgaagttgaccgcctggggagtacggtcgcaagattaaaactcaaaggaattgacggggacccgcacaagcggtggatgatgtggattaattcgatgcaacgcgaaaaaccttacctacccttgacatgtatggaatcctgctgagaggtgggagtgcccgaaagggagccataacacaggtgctgcatggctgtcgtcagctcgtgtcgtgagatgttgggttaagtcccgcaacgagcgcaacccttgtccctagttgctacgcaagagcactctagggagactgccggtgacaaaccggaggaaggtggggatgacgtcaagtcctcatggcccttatgggtagggcttcacacgtcatacaatggtcggaacagagggtcgccaacccgcgagggggagccaatcccagaaaaccgatcgtagtccggatcgcactctgcaactcgagtgcgtgaagctggaatcgctagtaatcgcggatcagcatgccgcggtgaatacgttcccgggtcttgtacacaccgcccgtcacaccatgggagtgggtttaccagaagtggctagtctaaccgcaaggaggac

SEQ ID NO: 19 - DNA, 1520 bp, Pseudomonas sp.
  misc_feature 1..1520: note = ribosomal RNA nucleic acid sequence
  source 1..1520: mol_type = genomic DNA
aagagtttgatcatggctcagattgaacgctggcggcaggcctaacacatgcaagtcgagcggtagagagaagcttgcttctcttgagagcggcggacgggtgagtaatgcctaggaatctgcctggtagtgggggataacgttcggaaacggacgctaataccgcatacgtcctacgggagaaagcaggggaccttcgggccttgcgctatcagatgagcctaggtcggattagctagttggtgaggtaatggctcaccaaggcgacgatccgtaactggtctgagaggatgatcagtcacactggaactgagacacggtccagactcctacgggaggcagcagtggggaatattggacaatgggcgaaagcctgatccagccatgccgcgtgtgtgaagaaggtcttcggattgtaaagcactttaagttgggaggaagggttgtagattaatactctgcaattttgacgttaccgacagaataagcaccggctaactctgtgccagcagccgcggtaatacagagggtgcaagcgttaatcggaattactgggcgtaaagcgcgcgtaggtggtttgttaagttggatgtgaaatccccgggctcaacctgggaactgcattcaaaactgactgactagagtatggtagagggtggtggaatttcctgtgtagcggtgaaatgcgtagatataggaaggaacaccagtggcgaaggcgaccacctggactgatactgacactgaggtgcgaaagcgtggggagcaaacaggattagataccctggtagtccacgccgtaaacgatgtcaactagccgttggaagccttgagcttttagtggcgcagctaacgcattaagttgaccgcctggggagtacggccgcaaggttaaaactcaaatgaattgacgggggcccgcacaagcggtggagcatgtggtttaattcgaagcaacgcgaagaaccttaccaggccttgacatccaatgaactttccagagatggattggtgccttcgggaacattgagacaggtgctgcatggctgtcgtcagctcgtgtcgtgagatgttgggttaagtcccgtaacgagcgcaacccttgtccttagttaccagcacgtaatggtgggcactctaaggagactgccggtgacaaaccggaggaaggtggggatgacgtcaagtcatcatggcccttacggcctgggctacacacgtgctacaatggtcggtacagagggttgccaagccgcgaggtggagctaatcccataaaaccgatcgtagtccggatcgcagtctgcaactcgactgcgtgaagtcggaatcgctagtaatcgcgaatcagaatgtcgcggtgaatacgttcccgggccttgtacacaccgcccgtcacaccatgggagtgggttgcaccagaagtagctagtctaaccttcgggaggacggttaccacggtgtgattcatgactggggtgaagtcgtaacaaggtagccgtaggggaacctgcggctgga

SEQ ID NO: 20 - DNA, 1389 bp, Pseudomonas sp.
  misc_feature 1..1389: note = ribosomal RNA nucleic acid sequence
  source 1..1389: mol_type = genomic DNA
aggttagactagctacttctggtgcaacccactcccatggtgtgacgggcggtgtgtacaaggcccgggaacgtattcaccgcgacattctgattcgcgattactagcgattccgacttcacgcagtcgagttgcagactgcgatccggactacgatcggttttatgggattagctccacctcgcggcttggcaaccctctgtaccgaccattgtagcacgtgtgtagcccaggccgtaagggccatgatgacttgacgtcatccccaccttcctccggtttgtcaccggcagtctccttagagtgcccaccattacgtgctggtaactaaggacaagggttgcgctcgttacgggacttaacccaacatctcacgacacgagctgacgacagccatgcagcacctgtctcaatgttcccgaaggcaccaatccatctctggaaagttcattggatgtcaaggcctggtaaggttcttcgcgttgcttcgaattaaaccacatgctccaccgcttgtgcgggcccccgtcaattcatttgagttttaaccttgcggccgtactccccaggcggtcaacttaatgcgttagctgcgccactaaaagctcaaggcttccaacggctagttgacatcgtttacggcgtggactaccagggtatctaatcctgtttgctccccacgctttcgcacctcagtgtcagtatcagtccaggtggtcgccttcgccactggtgttccttcctatatctacgcatttcaccgctacacaggaaattccaccaccctctaccatactctagtcagtcagttttgaatgcagttcccaggttgagcccggggatttcacatccaacttaacaaaccacctacgcgcgctttacgcccagtaattccgattaacgcttgcaccctctgtattaccgcggctgctggcacagagttagccggtgcttattctgtcggtaacgtcaaaattgcagagtattaatctacaacccttcctcccaacttaaagtgctttacaatccgaagaccttcttcacacacgcggcatggctggatcaggctttcgcccattgtccaatattccccactgctgcctcccgtaggagtctggaccgtgtctcagttccagtgtgactgatcatcctctcagaccagttacggatcgtcgccttggtgagccattacctcaccaactagctaatccgacctaggctcatctgatagcgcaaggcccgaaggtcccctgctttctcccgtaggacgtatgcggtattagcgtccgtttccgaacgttatcccccactaccaggcagattcctaggcattactcacccgtccgccgctctcaagagaagcaagcttctctctaccgctcgactgca

SEQ ID NO: 21 - DNA, 1391 bp, Pseudomonas sp.
  misc_feature 1..1391: note = ribosomal RNA nucleic acid sequence
  source 1..1391: mol_type = genomic DNA
aggttagactagctacttctggtgcaacccactcccatggtgtgacgggcggtgtgtacaaggcccgggaacgtattcaccgcgacattctgattcgcgattactagcgattccgacttcacgcagtcgagttgcagactgcgatccggactacgatcggttttgtgggattagctccacctcgcggcttggcaaccctctgtaccgaccattgtagcacgtgtgtagcccaggccgtaagggccatgatgacttgacgtcatccccaccttcctccggtttgtcaccggcagtctccttagagtgcccaccataacgtgctggtaactaaggacaagggttgcgctcgttacgggacttaacccaacatctcacgacacgagctgacgacagccatgcagcacctgtctcaatgttcccgaaggcaccaatccatctctggaaagttcattggatgtcaaggcctggtaaggttcttcgcgttgcttcgaattaaaccacatgctccaccgcttgtgcgggcccccgtcaattcatttgagttttaaccttgcggccgtactccccaggcggtcaacttaatgcgttagctgcgccactaagagctcaaggctcccaacggctagttgacatcgtttacggcgtggactaccagggtatctaatcctgtttgctccccacgctttcgcacctcagtgtcagtatcagtccaggtggtcgccttcgccactggtgttccttcctatatctacgcatttcaccgctacacaggaaattccaccaccctctaccatactctagctcgacagttttgaatgcagttcccaggttgagcccggggatttcacatccaacttaacgaaccacctacgcgcgctttacgcccagtaattccgattaacgcttgcaccctctgtattaccgcggctgctggcacagagttagccggtgcttattctgtcggtaacgtcaaaacaattacgtattaggtaactgcccttcctcccaacttaaagtgctttacaatccgaagaccttcttcacacacgcggcatggctggatcaggctttcgcccattgtccaatattccccactgctgcctcccgtaggagtctggaccgtgtctcagttccagtgtgactgatcatcctctcagaccagttacggatcgtcgccttggtgagccattacctcaccaactagctaatccgacctaggctcatctgatagcgcaaggcccgaaggtcccctgctttctcccgtaggacgtatgcggtattagcgtccgtttccgagcgttatcccccactaccaggcagattcctaggcattactcacccgtccgccgctcgccaccaggtacaagtacccgtgctgccgctcgactgca

SEQ ID NO: 22 - DNA, 1522 bp, Pseudomonas sp.
  misc_feature 1..1522: note = ribosomal RNA nucleic acid sequence
  source 1..1522: mol_type = genomic DNA
aagagtttgatcatggctcagattgaacgctggcggcaggcctaacacatgcaagtcgagcggcagcacgggtacttgtacctggtggcgagcggcggacgggtgagtaatgcctaggaatctgcctggtagtgggggataacgctcggaaacggacgctaataccgcatacgtcctacgggagaaagcaggggaccttcgggccttgcgctatcagatgagcctaggtcggattagctagttggtgaggtaatggctcaccaaggcgacgatccgtaactggtctgagaggatgatcagtcacactggaactgagacacggtccagactcctacgggaggcagcagtggggaatattggacaatgggcgaaagcctgatccagccatgccgcgtgtgtgaagaaggtcttcggattgtaaagcactttaagttgggaggaagggcagttacctaatacgtaattgttttgacgttaccgacagaataagcaccggctaactctgtgccagcagccgcggtaatacagagggtgcaagcgttaatcggaattactgggcgtaaagcgcgcgtaggtggttcgttaagttggatgtgaaatccccgggctcaacctgggaactgcattcaaaactgtcgagctagagtatggtagagggtggtggaatttcctgtgtagcggtgaaatgcgtagatataggaaggaacaccagtggcgaaggcgaccacctggactgatactgacactgaggtgcgaaagcgtggggagcaaacaggattagataccctggtagtccacgccgtaaacgatgtcaactagccgttgggagccttgagctcttagtggcgcagctaacgcattaagttgaccgcctggggagtacggccgcaaggttaaaactcaaatgaattgacgggggcccgcacaagcggtggagcatgtggtttaattcgaagcaacgcgaagaaccttaccaggccttgacatccaatgaactttccagagatggattggtgccttcgggaacattgagacaggtgctgcatggctgtcgtcagctcgtgtcgtgagatgttgggttaagtcccgtaacgagcgcaacccttgtccttagttaccagcacgttatggtgggcactctaaggagactgccggtgacaaaccggaggaaggtggggatgacgtcaagtcatcatggcccttacggcctgggctacacacgtgctacaatggtcggtacagagggttgccaagccgcgaggtggagctaatcccacaaaaccgatcgtagtccggatcgcagtctgcaactcgactgcgtgaagtcggaatcgctagtaatcgcgaatcagaatgtcgcggtgaatacgttcccgggccttgtacacaccgcccgtcacaccatgggagtgggttgcaccagaagtagctagtctaaccttcgggaggacggttaccacggtgtgattcatgactggggtgaagtcgtaacaaggtagccgtaggggaacctgcggctgga

SEQ ID NO: 23 - DNA, 1497 bp, Flavobacterium sp.
  misc_feature 1..1497: note = ribosomal RNA nucleic acid sequence
  source 1..1497: mol_type = genomic DNA
gaagagtttgatcctggctcaggatgaacgctagcggcaggcttaacacatgcaagtcgaggggtattagttttcggactaagagaccggcgcacgggtgcgtaacgcgtatgcaatctaccttttacagagggatagcccagagaaatttggattaatacctcatagtatatagacctggcatcaggattatattaaagtcacaacggtaaaagatgagcatgcgtcccattagctagttggtaaggtaacggcttaccaaggcaacgatgggtaggggtcctgagagggagatcccccacactggtactgagacacggaccagactcctacgggaggcagcagtgaggaatattggacaatgggcgcaagcctgatccagccatgccgcgtgcaggatgacggtcctatggattgtaaactgcttttgtacgagaagaaacactccttcgtgaaggagcttgacggtatcgtaagaataaggatcggctaactccgtgccagcagccgcggtaatacggaggatccaagcgttatccggaatcattgggtttaaagggtccgtaggcggtttagtaagtcagtggtgaaagcccatcgctcaacggtggaacggccattgatactgctaaacttgaattattaggaagtaactagaatatgtagtgtagcggtgaaatgcttagagattacatggaataccaattgcgaaggcaggttactactaatggattgacgctgatggacgaaagcgtgggtagcgaacaggattagataccctggtagtccacgccgtaaacgatggatactagctgttggaagcaatttcagtggctaagcgaaagtgataagtatcccacctggggagtacgttcgcaagaatgaaactcaaaggaattgacgggggcccgcacaagcggtggagcatgtggtttaattcgatgatacgcgaggaaccttaccaaggcttaaatgtagattgaccgatttggaaacagatctttcgcaagacaatttacaaggtgctgcatggttgtcgtcagctcgtgccgtgaggtgtcaggttaagtcctataacgagcgcaacccctgttgttagttgccagcgagtagtgtcgggaactctaacaagactgccagtgcaaactgtgaggaaggtggggatgacgtcaaatcatcacggcccttacgccttgggctacacacgtgctacaatggccggtacagagagcagccactgggcgaccaggagcgaatctataaaaccggtcacagttcggatcggagtctgcaactcgactccgtgaagctggaatcgctagtaatcggatatcagccatgatccggtgaatacgttcccgggccttgtacacaccgcccgtcaagccatggaagctgggggtgcctgaagtcggtgaccgcaaggagctgcctagggtaaaactggtaactagggctaagtcgtaacaaggtagccgtaccggaaggtgcggctgg

SEQ ID NO: 24 - DNA, 1516 bp, Acidovorax sp.
  misc_feature 1..1516: note = ribosomal RNA nucleic acid sequence
  source 1..1516: mol_type = genomic DNA
tagagtttgatcctggctcagattgaacgctggcggcatgccttacacatgcaagtcgaacggtaacaggtcttcggatgctgacgagtggcgaacgggtgagtaatacatcggaacgtgcccgatcgtgggggataacggagcgaaagctttgctaataccgcatacgatctacggatgaaagcaggggaccgcaaggccttgcgcggacggagcggccgatggcagattaggtagttggtgggataaaagctcaccaagccgacgatctgtagctggtctgagaggacgaccagccacactgggactgagacacggcccagactcctacgggaggcagcagtggggaattttggacaatgggcgaaagcctgatccagccatgccgcgtgcaggatgaaggccttcgggttgtaaactgcttttgtacggaacgaaaagactccttctaataaagggggtccatgacggtaccgtaagaataagcaccggctaactacgtgccagcagccgcggtaatacgtagggtgcaagcgttaatcggaattactgggcgtaaagcgtgcgcaggcggttatataagacagatgtgaaatccccgggctcaacctgggaactgcatttgtgactgtatagctagagtacggtagagggggatggaattccgcgtgtagcagtgaaatgcgtagatatgcggaggaacaccgatggcgaaggcaatcccctggacctgtactgacgctcatgcacgaaagcgtggggagcaaacaggattagataccctggtagtccacgccctaaacgatgtcaactggttgttgggtcttcactgactcagtaacgaagctaacgcgtgaagttgaccgcctggggagtacggccgcaaggttgaaactcaaaggaattgacggggacccgcacaagcggtggatgatgtggtttaattcgatgcaacgcgaaaaaccttacccacctttgacatgtacggaatcctttagagatagaggagtgctcgaaagagaaccgtaacacaggtgctgcatggctgtcgtcagctcgtgtcgtgagatgttgggttaagtcccgcaacgagcgcaacccttgtcattagttgctacatttagttgggcactctaatgagactgccggtgacaaaccggaggaaggtggggatgacgtcaagtcctcatggcccttataggtggggctacacacgtcatacaatggctggtacagagggttgccaacccgcgagggggagccaatcccataaagccagtcgtagtccggatcgcagtctgcaactcgactgcgtgaagtcggaatcgctagtaatcgcggatcagaatgtcgcggtgaatacgttcccgggtcttgtacacaccgcccgtcacaccatgggagcgggttctgccagaagtaggtagcctaaccgtaaggagggcgcttaccacggcagggttcgtgactggggtgaagtcgtaacaaggtagccgtatcggaaggtgcggctgga

SEQ ID NO: 25 - DNA, 1417 bp, Bacillus sp.
  misc_feature 144: note = n is a, c, g, or t
  misc_feature 214: note = n is a, c, g, or t
  misc_feature 1392..1393: note = n is a, c, g, or t
  misc_feature 1..1417: note = ribosomal RNA nucleic acid sequence
  source 1..1417: mol_type = genomic DNA
tgcagtcgagcggatcgatgggagcttgctccctgagatcagcggcggacgggtgagtaacacgtgggtaacctgcctgtaagactgggataactccgggaaaccggggctaataccggataacacctacccccgcatgggggnaggttgaaaggtggcttcggctatcacttacagatggacccgcggcgcattagctagttggtgaggtaanggctcaccaaggcgacgatgcgtagccgacctgagagggtgatcggccacactgggactgagacacggcccagactcctacgggaggcagcagtagggaatcttccgcaatggacgaaagtctgacggagcaacgccgcgtgagtgaagaaggttttcggatcgtaaaactctgttgttagggaagaacaagtgccgttcgaatagggcggcgccttgacggtacctaaccagaaagccacggctaactacgtgccagcagccgcggtaatacgtaggtggcaagcgttgtccggaattattgggcgtaaagcgcgcgcaggtggtttcttaagtctgatgtgaaagcccacggctcaaccgtggagggtcattggaaactggggaacttgagtgcagaagaggaaagtggaattccaagtgtagcggtgaaatgcgtagatatttggaggaacaccagtggcgaaggcgactttctggtctgtaactgacactgaggcgcgaaagcgtggggagcaaacaggattagataccctggtagtccacgccgtaaacgatgagtgctaagtgttagagggtttccgccctttagtgctgcagctaacgcattaagcactccgcctggggagtacggtcgcaagactgaaactcaaaggaattgacgggggcccgcacaagcggtggagcatgtggtttaattcgaagcaacgcgaagaaccttaccaggtcttgacatcctctgacaaccctagagatagggctttccccttcgggggacagagtgacaggtggtgcatggttgtcgtcagctcgtgtcgtgagatgttgggttaagtcccgcaacgagcgcaacccttgatcttagttgccagcattcagttgggcactctaagatgactgccggtgacaaaccggaggaaggtggggatgacgtcaaatcatcatgccccttatgacctgggctacacacgtgctacaatggacggtacaaagggctgcaagaccgcgaggtttagccaatcccataaaaccgttctcagttcggattgtaggctgcaactcgcctacatgaagctggaatcgctagtaatcgcggatcagcatgccgcggtgaatacgttcccgggccttgtacacaccgcccgtcacaccacgagagtttgtaacacccgaagtcgnngaggtaacctttggagccagccgc

SEQ ID NO: 26 - DNA, 1366 bp, Enterobacter sp.
  misc_feature 312..313: note = n is a, c, g, or t
  misc_feature 1267: note = n is a, c, g, or t
  misc_feature 1329: note = n is a, c, g, or t
  misc_feature 1..1366: note = ribosomal RNA nucleic acid sequence
  source 1..1366: mol_type = genomic DNA
ttaagctacctacttcttttagcaacccactcccatggtgtgacgggcggtgtgtacaaggcccgggaacgtattcaccgtagcattctgatctacgattactagcgattccgacttcatggagtcgagttgcagactccaatccggactacgacgcactttatgaggtccgcttgctctcgcgaggtcgcttctctttgtatgcgccattgtagcacgtgtgtagccctactcgtaagggccatgatgacttgacgtcatccccaccttcctccagtttatcactggcagtctcctttgagttcccggccnnaccgctggcaacaaaggataagggttgcgctcgttgcgggacttaacccaacatttcacaacacgagctgacgacagccatgcagcacctgtctcagagttcccgaaggcaccaatccatctctggaaagttctctggatgtcaagagtaggtaaggttcttcgcgttgcatcgaattaaaccacatgctccaccgcttgtgcgggcccccgtcaattcatttgagttttaaccttgcggccgtactccccaggcggtcgacttaacgcgttagctccggaagccacgcctcaagggcacaacctccaagtcgacatcgtttacggcgtggactaccagggtatctaatcctgtttgctccccacgctttcgcacctgagcgtcagtctttgtccagggggccgccttcgccaccggtattcctccagatctctacgcatttcaccgctacacctggaattctacccccctctacaagactctagcctgccagtttcgaatgcagttcccaggttgagcccggggatttcacatccgacttgacagaccgcctgcgtgcgctttacgcccagtaattccgattaacgcttgcaccctccgtattaccgcggctgctggcacggagttagccggtgcttcttctgcgggtaacgtcaatcgacaaggttattaaccttatcgccttcctccccgctgaaagtactttacaacccgaaggccttcttcatacacgcggcatggctgcatcaggcttgcgcccattgtgcaatattccccactgctgcctcccgtaggagtctggaccgtgtctcagttccagtgtggctggtcatcctctcagaccagctagggatcgtcgcctaggtgagccgttaccccacctactagctaatcccatctgggcacatctgatggcaagaggcccgaaggtccccctctttggtcttgcgacgntatgcggtattagctaccgtttccagtagttatccccctccatcaggcagtttcccagacantactcacccgtccgccgctcgccggcaaagtagcaag

SEQ ID NO: 27 - DNA, 1524 bp, Enterobacter sp.
  misc_feature 1..1524: note = ribosomal RNA nucleic acid sequence
  source 1..1524: mol_type = genomic DNA
agagtttgatcatggctcagattgaacgctggcggcaggcctaacacatgcaagtcgagcggcagcggaaagtagcttgctactttgccggcgagcggcggacgggtgagtaatgtctgggaaactgcctgatggagggggataactactggaaacggtagctaataccgcataacgtcgcaagaccaaagagggggaccttcgggcctcttgccatcagatgtgcccagatgggattagctagtaggtggggtaacggctcacctaggcgacgatccctagctggtctgagaggatgaccagccacactggaactgagacacggtccagactcctacgggaggcagcagtggggaatattgcacaatgggcgcaagcctgatgcagccatgccgcgtgtatgaagaaggccttcgggttgtaaagtactttcagcggggaggaaggcgataaggttaataaccttgtcgattgacgttacccgcagaagaagcaccggctaactccgtgccagcagccgcggtaatacggagggtgcaagcgttaatcggaattactgggcgtaaagcgcacgcaggcggtctgtcaagtcggatgtgaaatccccgggctcaacctgggaactgcattcgaaactggcaggctagagtcttgtagaggggggtagaattccaggtgtagcggtgaaatgcgtagagatctggaggaataccggtggcgaaggcggccccctggacaaagactgacgctcaggtgcgaaagcgtggggagcaaacaggattagataccctggtagtccacgccgtaaacgatgtcgacttggaggttgtgcccttgaggcgtggcttccggagctaacgcgttaagtcgaccgcctggggagtacggccgcaaggttaaaactcaaatgaattgacgggggcccgcacaagcggtggagcatgtggtttaattcgatgcaacgcgaagaaccttacctactcttgacatccagagaactttccagagatggattggtgccttcgggaactctgagacaggtgctgcatggctgtcgtcagctcgtgttgtgaaatgttgggttaagtcccgcaacgagcgcaacccttatcctttgttgccagcggttaggccgggaactcaaaggagactgccagtgataaactggaggaaggtggggatgacgtcaagtcatcatggcccttacgagtagggctacacacgtgctacaatggcgcatacaaagagaagcgacctcgcgagagcaagcggacctcataaagtgcgtcgtagtccggattggagtctgcaactcgactccatgaagtcggaatcgctagtaatcgtagatcagaatgctacggtgaatacgttcccgggccttgtacacaccgcccgtcacaccatgggagtgggttgcaaaagaagtaggtagcttaaccttcgggagggcgcttaccactttgtgattcatgactggggtgaagtcgtaacaaggtaaccgtaggggaacctgcggttgga

SEQ ID NO: 28 - DNA, 1518 bp, Variovorax sp.
  misc_feature 1..1518: note = ribosomal RNA nucleic acid sequence
  source 1..1518: mol_type = genomic DNA
tagagtttgatcctggctcagattgaacgctggcggcatgccttacacatgcaagtcgaacggcagcgcgggagcaatcctggcggcgagtggcgaacgggtgagtaatacatcggaacgtgcccaatcgtgggggataacgcagcgaaagctgtgctaataccgcatacgatctacggatgaaagcaggggatcgcaagaccttgcgcgaatggagcggccgatggcagattaggtagttggtgaggtaaaggctcaccaagccttcgatctgtagctggtctgagaggacgaccagccacactgggactgagacacggcccagactcctacgggaggcagcagtggggaattttggacaatgggcgaaagcctgatccagccatgccgcgtgcaggatgaaggccttcgggttgtaaactgcttttgtacggaacgaaacggccttttctaataaagagggctaatgacggtaccgtaagaataagcaccggctaactacgtgccagcagccgcggtaatacgtagggtgcaagcgttaatcggaattactgggcgtaaagcgtgcgcaggcggttatgtaagacagttgtgaaatccccgggctcaacctgggaactgcatctgtgactgcatagctagagtacggtagagggggatggaattccgcgtgtagcagtgaaatgcgtagatatgcggaggaacaccgatggcgaaggcaatcccctggacctgtactgacgctcatgcacgaaagcgtggggagcaaacaggattagataccctggtagtccacgccctaaacgatgtcaactggttgttgggtcttcactgactcagtaacgaagctaacgcgtgaagttgaccgcctggggagtacggccgcaaggttgaaactcaaaggaattgacggggacccgcacaagcggtggatgatgtggtttaattcgatgcaacgcgaaaaaccttacccacctttgacatgtacggaattcgccagagatggcttagtgctcgaaagagagccgtaacacaggtgctgcatggctgtcgtcagctcgtgtcgtgagatgttgggttaagtcccgcaacgagcgcaacccttgtcattagttgctacattcagttgggcactctaatgagactgccggtgacaaaccggaggaaggtggggatgacgtcaagtcctcatggcccttataggtggggctacacacgtcatacaatggctggtacaaagggttgccaacccgcgagggggagctaatcccataaaaccagtcgtagtccggatcgcagtctgcaactcgactgcgtgaagtcggaatcgctagtaatcgtggatcagaatgtcacggtgaatacgttcccgggtcttgtacacaccgcccgtcacaccatgggagcgggttctgccagaagtagttagcttaaccgcaaggagggcgattaccacggcagggttcgtgactggggtgaagtcgtaacaaggtagccgtatcggaaggtgcggctgga

SEQ ID NO: 29 - DNA, 1441 bp, Variovorax sp.
  misc_feature 1..1441: note = ribosomal RNA nucleic acid sequence
  source 1..1441: mol_type = genomic DNA
tatcgccctccttgcggttaagctaactacttctggcagaacccgctcccatggtgtgacgggcggtgtgtacaagacccgggaacgtattcaccgtgacattctgatccacgattactagcgattccgacttcacgcagtcgagttgcagactgcgatccggactacgactggttttatgggattagctccccctcgcgggttggcaaccctttgtaccagccattgtatgacgtgtgtagccccacctataagggccatgaggacttgacgtcatccccaccttcctccggtttgtcaccggcagtctcattagagtgcccaactgaatgtagcaactaatgacaagggttgcgctcgttgcgggacttaacccaacatctcacgacacgagctgacgacagccatgcagcacctgtgttacggctctctttcgagcactaagccatctctggcgaattccgtacatgtcaaaggtgggtaaggtttttcgcgttgcatcgaattaaaccacatcatccaccgcttgtgcgggtccccgtcaattcctttgagtttcaaccttgcggccgtactccccaggcggtcaacttcacgcgttagcttcgttactgagtcagtgaagacccaacaaccagttgacatcgtttagggcgtggactaccagggtatctaatcctgtttgctccccacgctttcgtgcatgagcgtcagtacaggtccaggggattgccttcgccatcggtgttcctccgcatatctacgcatttcactgctacacgcggaattccatccccctctaccgtactctagctatgcagtcacagatgcagttcccaggttgagcccggggatttcacaactgtcttacataaccgcctgcgcacgctttacgcccagtaattccgattaacgcttgcaccctacgtattaccgcggctgctggcacgtagttagccggtgcttattcttacggtaccgtcattagccctctttattagaaaaggccgtttcgttccgtacaaaagcagtttacaacccgaaggccttcatcctgcacgcggcatggctggatcaggctttcgcccattgtccaaaattccccactgctgcctcccgtaggagtctgggccgtgtctcagtcccagtgtggctggtcgtcctctcagaccagctacagatcgaaggcttggtgagcctttacctcaccaactacctaatctgccatcggccgctccattcgcgcaaggtcttgcgatcccctgctttcatccgtagatcgtatgcggtattagcacagctttcgctgcgttatcccccacgattgggcacgttccgatgtattactcacccgttcgccactcgccgccaggattgctcccgcgctgccgttcgacttgcatgtgtaaggcatgccgccagcgttcaatctgagccatga

SEQ ID NO: 30 - DNA, 1512 bp, Acidovorax sp.
  misc_feature 1..1512: note = ribosomal RNA nucleic acid sequence
  source 1..1512: mol_type = genomic DNA
tagagtttgatcctggctcagattgaacgctggcggcatgccttacacatgcaagtcgaacggtaacaggtcttcggatgctgacgagtggcgaacgggtgagtaatacatcggaacgtgcccgatcgtgggggataacggagcgaaagctttgctaataccgcatacgatctacggatgaaagcaggggaccgcaaggccttgcgcggacggagcggccgatggcagattaggtagttggtgggataaaagcttaccaagccgacgatctgtagctggtctgagaggacgaccagccacactgggactgagacacggcccagactcctacgggaggcagcagtggggaattttggacaatgggcgaaagcctgatccagccatgccgcgtgcaggatgaaggccttcgggttgtaaactgcttttgtacggaacgaaaagactccttctaataaagggggtccatgacggtaccgtaagaataagcaccggctaactacgtgccagcagccgcggtaatacgtagggtgcaagcgttaatcggaattactgggcgtaaagcgtgcgcaggcggttatgtaagacagatgtgaaatccccgggctcaacctgggaactgcatttgtgactgcatagctagagtacggcagagggggatggaattccgcgtgtagcagtgaaatgcgtagatatgcggaggaacaccgatggcgaaggcaatcccctgggcctgtactgacgctcatgcacgaaagcgtggggagcaaacaggattagataccctggtagtccacgccctaaacgatgtcaactggttgttgggtcttcactgactcagtaacgaagctaacgcgtgaagttgaccgcctggggagtacggccgcaaggttgaaactcaaaggaattgacggggacccgcacaagcggtggatgatgtggtttaattcgatgcaacgcgaaaaaccttacccacctttgacatgtacggaatcctttagagatagaggagtgctcgaaagagaaccgtaacacaggtgctgcatggctgtcgtcagctcgtgtcgtgagatgttgggttaagtcccgcaacgagcgcaacccttgccattagttgctacgaaagggcactctaatgggactgccggtgacaaaccggaggaaggtggggatgacgtcaagtcctcatggcccttataggtggggctacacacgtcatacaatggctggtacagagggttgccaacccgcgagggggagccaatcccataaagccagtcgtagtccggatcgcagtctgcaactcgactgcgtgaagtcggaatcgctagtaatcgcggatcagaatgtcgcggtgaatacgttcccgggtcttgtacacaccgcccgtcacaccatgggagcgggttctgccagaagtagttagcctaaccgcaaggagggcgattaccacggcagggttcgtgactggggtgaagtcgtaacaaggtagccgtatcggaaggtgcggctgga

SEQ ID NO: 31 - DNA, 1520 bp, Pseudomonas sp.
  misc_feature 1..1520: note = ribosomal RNA nucleic acid sequence
  source 1..1520: mol_type = genomic DNA
aagagtttgatcatggctcagattgaacgctggcggcaggcctaacacatgcaagtcgagcggtagagaggtgcttgcacctcttgagagcggcggacgggtgagtaatgcctaggaatctgcctggtagtgggggataacgctcggaaacggacgctaataccgcatacgtcctacgggagaaagcaggggaccttcgggccttgcgctatcagatgagcctaggtcggattagctagttggtgaggtaatggctcaccaaggcgacgatccgtaactggtctgagaggatgatcagtcacactggaactgagacacggtccagactcctacgggaggcagcagtggggaatattggacaatgggcgaaagcctgatccagccatgccgcgtgtgtgaagaaggtcttcggattgtaaagcactttaagttgggaggaagggcattaacctaatacgttagtgttttgacgttaccgacagaataagcaccggctaactctgtgccagcagccgcggtaatacagagggtgcaagcgttaatcggaattactgggcgtaaagcgcgcgtaggtggttcgttaagttggatgtgaaatccccgggctcaacctgggaactgcattcaaaactgtcgagctagagtatggtagagggtggtggaatttcctgtgtagcggtgaaatgcgtagatataggaaggaacaccagtggcgaaggcgaccacctggactgatactgacactgaggtgcgaaagcgtggggagcaaacaggattagataccctggtagtccacgccgtaaacgatgtcaactagccgttgggagccttgagctcttagtggcgcagctaacgcattaagttgaccgcctggggagtacggccgcaaggttaaaactcaaatgaattgacgggggcccgcacaagcggtggagcatgtggtttaattcgaagcaacgcgaagaaccttaccaggccttgacatccaatgaactttccagagatggattggtgccttcgggaacattgagacaggtgctgcatggctgtcgtcagctcgtgtcgtgagatgttgggttaagtcccgtaacgagcgcaacccttgtccttagttaccagcacgttatggtgggcactctaaggagactgccggtgacaaaccggaggaaggtggggatgacgtcaagtcatcatggcccttacggcctgggctacacacgtgctacaatggtcggtacagagggttgccaagccgcgaggtggagctaatcccacaaaaccgatcgtagtccggatcgcagtctgcaactcgactgcgtgaagtcggaatcgctagtaatcgcgaatcagaatgtcgcggtgaatacgttcccgggccttgtacacaccgcccgtcacaccatgggagtgggttgcaccagaagtagctagtctaaccttcggggggacggttaccacggtgtgattcatgactggggtgaagtcgtaacaaggtagccgtaggggaacctgcggctgga

SEQ ID NO: 32 - DNA, 1535 bp, Bacillus sp.
  misc_feature 1..1535: note = ribosomal RNA nucleic acid sequence
  source 1..1535: mol_type = genomic DNA
ggagagtttgatcctggctcaggacgaacgctggcggcgtgcctaatacatgcaagtcgagcggacagaagggagcttgctcccggatgttagcggcggacgggtgagtaacacgtgggtaacctgcctgtaagactgggataactccgggaaaccggagctaataccggatagttccttgaaccgcatggttcaaggatgaaagacggtttcggctgtcacttacagatggacccgcggcgcattagctagttggtggggtaatggctcaccaaggcgacgatgcgtagccgacctgagagggtgatcggccacactgggactgagacacggcccagactcctacgggaggcagcagtagggaatcttccgcaatggacgaaagtctgacggagcaacgccgcgtgagtgatgaaggttttcggatcgtaaagctctgttgttagggaagaacaagtgcgagagtaactgctcgcaccttgacggtacctaaccagaaagccacggctaactacgtgccagcagccgcggtaatacgtaggtggcaagcgttgtccggaattattgggcgtaaagggctcgcaggcggtttcttaagtctgatgtgaaagcccccggctcaaccggggagggtcattggaaactgggaaacttgagtgcagaagaggagagtggaattccacgtgtagcggtgaaatgcgtagagatgtggaggaacaccagtggcgaaggcgactctctggtctgtaactgacgctgaggagcgaaagcgtggggagcgaacaggattagataccctggtagtccacgccgtaaacgatgagtgctaagtgttagggggtttccgccccttagtgctgcagctaacgcattaagcactccgcctggggagtacggtcgcaagactgaaactcaaaggaattgacgggggcccgcacaagcggtggagcatgtggtttaattcgaagcaacgcgaagaaccttaccaggtcttgacatcctctgacaatcctagagataggacgtccccttcgggggcagagtgacaggtggtgcatggttgtcgtcagctcgtgtcgtgagatgttgggttaagtcccgcaacgagcgcaacccttgatcttagttgccagcattcagttgggcactctaaggtgactgccggtgacaaaccggaggaaggtggggatgacgtcaaatcatcatgccccttatgacctgggctacacacgtgctacaatggacagaacaaagggcagcgaaaccgcgaggttaagccaatcccacaaatctgttctcagttcggatcgcagtctgcaactcgactgcgtgaagctggaatcgctagtaatcgcggatcagcatgccgcggtgaatacgttcccgggccttgtacacaccgcccgtcacaccacgagagtttgtaacacccgaagtcggtgaggtaaccttttaggagccagccgccgaaggtgggacagatgattggggtgaagtcgtaacaaggtagccgtatcggaaggtgcggctggatc

SEQ ID NO: 33 - DNA, 1415 bp, Curtobacterium sp.
  misc_feature 1386: note = n is a, c, g, or t
  misc_feature 1..1415: note = ribosomal RNA nucleic acid sequence
  source 1..1415: mol_type = genomic DNA
ggttaggccaccggcttcgggtgttaccgactttcatgacttgacgggcggtgtgtacaaggcccgggaacgtattcaccgcagcgttgctgatctgcgattactagcgactccgacttcatgaggtcgagttgcagacctcaatccgaactgagaccggctttttgggattcgctccaccttacggtatcgcagccctttgtaccggccattgtagcatgcgtgaagcccaagacataaggggcatgatgatttgacgtcatccccaccttcctccgagttgaccccggcagtctcctatgagtccccggcataacccgctggcaacatagaacgagggttgcgctcgttgcgggacttaacccaacatctcacgacacgagctgacgacaaccatgcaccacctgtacaccgaccacaagggggcgaccatctctggccgtttccggtgtatgtcaagccttggtaaggttcttcgcgttgcatcgaattaatccgcatgctccgccgcttgtgcgggcccccgtcaattcctttgagttttagccttgcggccgtactccccaggcggggcgcttaatgcgttagctacgacacagaaaccgtggaaaggtccctacatctagcgcccaacgtttacggcatggactaccagggtatctaatcctgttcgctccccatgctttcgctcctcagcgtcagttacggcccagagatctgccttcgccatcggtgttcctcctgatatctgcgcattccaccgctacaccaggaattccaatctcccctaccgcactctagtctgcccgtacccactgcaagcccgaggttgagcctcgggatttcacagcagacgcgacaaaccgcctacgagctctttacgcccaataattccggacaacgcttgcaccctacgtattaccgcggctgctggcacgtagttagccggtgctttttctgcaggtaccgtcactttcgcttcttccctactaaaagaggtttacaacccgaaggccgtcatccctcacgcggcgttgctgcatcaggctttcgcccattgtgcaatattccccactgctgcctcccgtaggagtctgggccgtgtctcagtcccagtgtggccggtcaccctctcaggccggctacccgtcgtcgccttggtgagccattacctcaccaacaagctgataggccgcgagtccatccccaaccaaaaaatctttccaccaccagaccatgcggccagtgatcatatccagtattagacgtcgtttccaacgcttatcccagagtcaggggcaggttactcacgtgttactcacccgttcgccactaatccacccagcaagctgggcatcatcgttcgacttgcatgtgttaagcacnccgccagcgttcgtcctgagccatgattc

SEQ ID NO: 34 - DNA, 1375 bp, Paenibacillus sp.
  misc_feature 423: note = n is a, c, g, or t
  misc_feature 438: note = n is a, c, g, or t
  misc_feature 1361: note = n is a, c, g, or t
  misc_feature 1..1375: note = ribosomal RNA nucleic acid sequence
  source 1..1375: mol_type = genomic DNA
caccgacttcgggtgttgtaaactctcgtggtgtgacgggcggtgtgtacaagacccgggaacgtattcaccgcggcatgctgatccgcgattactagcaattccgacttcatgtaggcgagttgcagcctacaatccgaactgagaccggcttttctaggattggctccacctcgcgatttcgcttcccgttgtaccggccattgtagtacgtgtgtagcccaggtcataaggggcatgatgatttgacgtcatccccaccttcctccggtttgtcaccggcagtctgcttagagtgcccagcttgacctgctggcaactaagcataagggttgcgctcgttgcgggacttaacccaacatctcacgacacgagctgacgacaaccatgcaccacctgtctcctctgtcccgaaggaaaggnctatctctagaccgntcagagggatgtcaagacctggtaaggttcttcgcgttgcttcgaattaaaccacatactccactgcttgtgcgggtccccgtcaattcctttgagtttcagtcttgcgaccgtactccccaggcggaatgcttaatgtgttaacttcggcaccaagggtatcgaaacccctaacacctagcattcatcgtttacggcgtggactaccagggtatctaatcctgtttgctccccacgctttcgcgcctcagcgtcagttacagcccagagagtcgccttcgccactggtgttcctccacatctctacgcatttcaccgctacacgtggaattccactctcctcttctgcactcaagctccccagtttccagtgcgacccgaagttgagcctcgggattaaacaccagacttaaagagccgcctgcgcgcgctttacgcccaataattccggacaacgcttgccccctacgtattaccgcggctgctggcacgtagttagccggggctttcttctcaggtaccgtcactcttgtagcagttactctacaagacgttcttccctggcaacagagctttacgatccgaaaaccttcatcactcacgcggcgttgctccgtcaggctttcgcccattgcggaagattccctactgctgcctcccgtaggagtctgggccgtgtctcagtcccagtgtggccgatcaccctctcaggtcggctacgcatcgtcgccttggtaggcctttaccccaccaactagctaatgcgccgcaggcccatccacaagtgacagattgctccgtctttcctccttctcccatgcaggaaaaggatgtatcgggtattagctaccgtttccggtagttatccctgtcttgtgggcaggttgcctacgtgttactcacccgtccgccgctaggttatntagaagcaagcttc

SEQ ID NO: 35 - DNA, 1433 bp, Bacillus sp.
  misc_feature 307: note = n is a, c, g, or t
  misc_feature 980: note = n is a, c, g, or t
  misc_feature 1..1433: note = ribosomal RNA nucleic acid sequence
  source 1..1433: mol_type = genomic DNA
ctcaccgacttcgggtgttacaaactctcgtggtgtgacgggcggtgtgtacaagacccgggaacgtattcaccgcggcatgctgatccgcgattactagcgattccggcttcatgtaggcgagttgcagcctacaatccgaactgagaatggttttatgggattggcttaacctcgcggttttgcagccctttgtaccatccattgtagcacgtgtgtagcccaggtcataaggggcatgatgatttgacgtcatccccaccttcctccggtttgtcaccggcagtcaccttagagtgcccaactnaatgctggcaactaagatcaagggttgcgctcgttgcgggacttaacccaacatctcacgacacgagctgacgacaaccatgcaccacctgtcactctgtccccgaagggaaccttctatctctagaagtagcagaggatgtcaagacctggtaaggttcttcgcgttgcttcgaattaaaccacatgctccaccgcttgtgcgggtccccgtcaattcctttgagtttcagtcttgcgaccgtactccccaggcggagtgcttaatgcgtttgctgcagcactaaagggcggaaaccctctaacacttagcactcatcgtttacggcgtggactaccagggtatctaatcctgttcgctccccacgctttcgcgcctcagcgtcagttacagaccagagagccgccttcgccactggtgttcctccacatctctacgcatttcaccgctacacgtggaattccgctctcctcttctgcactcaagttccccagtttccaatgaccctccacggttgagccgtgggctttcacatcagacttaaggaaccgcctgcgcgcgctttacgcccaataattccggacaacgcttgccacctacgtattaccgcggctgctggcacgtagttagccgtggctttctggttaggtaccgtcaaggtacctgcttattnaacaggtacttgttcttccctaacaacagagctttacgatccgaaaaccttcatcactcacgcggcgttgctccgtcagactttcgtccattgcggaagattccctactgctgcctcccgtaggagtctgggccgtgtctcagtcccagtgtggccgatcaccctctcaggtcggctacgcatcgtcgccttggtgagccgttacctcaccaactagctaatgcgccgcgggcccatccttgagtggtagctaaaagccaccttctaacatatcctcatgcgaagatatgtgttatccggtattagctccggtttcccggagttatccccgtctcaagggcaggttgcccacgtgttactcacccgtccgccgctaagttttgaaaagcaagcttttcaaaactccgctcgacttgcatgtattaggcacgccgccagcgttcgtcctgagcc

SEQ ID NO: 36 - DNA, 1468 bp, Bacillus sp.
  misc_feature 472: note = n is a, c, g, or t
  misc_feature 1..1468: note = ribosomal RNA nucleic acid sequence
  source 1..1468: mol_type = genomic DNA
ccaccttaggcggctggctccatgaaggttacctcaccgacttcgggtgttacaaactctcgtggtgtgacgggcggtgtgtacaaggcccgggaacgtattcaccgcggcatgctgatccgcgattactagcgattccggcttcatgcaggcgagttgcagcctgcaatccgaactgagaatggctttatgggattcgcttaccttcgcaggtttgcagccctttgtaccatccattgtagcacgtgtgtagcccaggtcataaggggcatgatgatttgacgtcatccccaccttcctccggtttgtcaccggcagtcaccttagagtgcccaactgaatgctggcaactaagatcaagggttgcgctcgttgcgggacttaacccaacatctcacgacacgagctgacgacaaccatgcaccacctgtcactctgtcccccgaaggggaaagccctatctctagggttntcagaggatgtcaagacctggtaaggttcttcgcgttgcttcgaattaaaccacatgctccaccgcttgtgcgggcccccgtcaattcctttgagtttcagccttgcggccgtactccccaggcggagtgcttaatgcgttagctgcagcactaaagggcggaaaccctctaacacttagcactcatcgtttacggcgtggactaccagggtatctaatcctgtttgctccccacgctttcgcgcctcagtgtcagttacagaccagaaagtcgccttcgccactggtgttcctccaaatctctacgcatttcaccgctacacttggaattccactttcctcttctgcactcaagttccccagtttccaatgaccctccacggttgagccgtgggctttcacatcagacttaaggaaccacctgcgcgcgctttacgcccaataattccggacaacgcttgccacctacgtattaccgcggctgctggcacgtagttagccgtggctttctggttaggtaccgtcaaggtaccagcagttactctggtacttgttcttccctaacaacagaactttacgacccgaaggccttcttcgttcacgcggcgttgctccgtcagactttcgtccattgcggaagattccctactgctgcctcccgtaggagtctgggccgtgtctcagtcccagtgtggccgatcaccctctcaggtcggctacgcatcgtcgccttggtgagccattacctcaccaactagctaatgcgccgcgggcccatctataagtgacagcgtaaaccgtctttccatcttctctcatgcgagaaaagaacgtatccggtattagctccggtttcccgaagttatcccagtcttataggcaggttgcccacgtgttactcacccgtccgccgctaatctcagggagcaagctcccatcgattcgctcgacttgcatgtattaggcacgccgccagcgttcgtcctgagccatgat

SEQ ID NO: 37 - DNA, 491 bp, Bacillus sp.
  misc_feature 1..491: note = Marker nucleic acid sequence
  source 1..491: mol_type = genomic DNA
atgataattaggtgaggggggaagttggtgtatttctaagtagagtcgattataaaattagtttttaaatttatatgcattagtatatccattagataactagaacaaaatataattagaataccttccgacgttggtattcgtagcactattttctgattttctatataaaaaacctactgttggcgaaagatgaacagtaggttttttcctttttaggttttatataatattcatttcttgttcacataaaacacatttattagaagtttggaatttagatatactcactcttttttacatgattaaactgaccgatacttctaaattttttatgacgctgatttacaagttcttctgaagataataataagagttcatgcagtgaagctttaattgtattttcaatttctttagcttgtttttcaatatcattatgggcgccaccttgaacttcagatatcacactatctataatccctaattttttt

SEQ ID NO: 38 - DNA, 398 bp, Bacillus sp.
  misc_feature 1..398: note = Marker nucleic acid sequence
  source 1..398: mol_type = genomic DNA
gcttctctaactaactcagtaggtttgaccttgtattcgatataatatgccaacaataatgcttttattttcttgcttaaatcatctttatctgtatttgtcagactttcagttctactaaataaggcattgtttaaatttttcacactactcttgacaactgtatcaacacttgcatacagatctccccgcacattttccaataatttatcgtctaattgtttgcaaaattgaaacattgctgttctatcatctttaacaacaggtttttgtaaggatacaccaagggtattgaaaacttttgttatggcttttttgtggagttgatgaatagttgtatctgtatctgaggtttctttttttatttcagttacatttttcatcatggtggtagctaa

SEQ ID NO: 39 - DNA, 443 bp, Bacillus sp.
  misc_feature 1..443: note = Marker nucleic acid sequence
  source 1..443: mol_type = genomic DNA
ctgcagggggaattttcacacattctaaattaaatttgtattatttctaacaaaaaagagattgagacatcaatacatcaatccaatctaaagacgaataaatgggatgatctatgacaccgctgttaatttctgtgtcagagttcgcttttcgcgggcggcctatgagcttcctcgtcgctcgcgctcctgtgggggctcatcctttccgcttttcccgcagggccctccaatcaaccgctagaagtaactacatacatgaaatctgcgttcaatttacctagttattatctatttggatttaacaagtcatttatcatttcctcgtaagttattttaaagctgatataaaatggttaaaatttaaaaaatattaaacagtaccttgcaataaacaatagctgatgatatattgtaattattaggaaatcattgtaagtcac

SEQ ID NO: 40 - DNA, 386 bp, Bacillus sp.
  misc_feature 1..386: note = Marker nucleic acid sequence
  source 1..386: mol_type = genomic DNA
tattggtagacatgctttatccccctattggtttttcgttagttctcgatacaactctattaatgtgaataattaaatacattttttcgtcgttagaaatcgtgtattcaaaattggtacgaatatatttttgaattttttcaacacacttgacttcctgtgggtactttcggttaatttggtcaagtagatcattatcacctgtgcttaacatcttattatcaagtaaacgttctacaaaaaattgcaggtgtgtaagaaacctagaaaaattgatagtatccgtaggaatatcaaccttatagtgaaatttaataatgtttagaatgtccttaaccgtatttgtcattagtaatatgtggtttgaattatcttcattttgttgt

SEQ ID NO: 41 - DNA, 323 bp, Bacillus sp.
  misc_feature 1..323: note = Marker nucleic acid sequence
  source 1..323: mol_type = genomic DNA
gactgaggatagcgttgaggtgaataaaaagtcacctgcaagcaactgatgttgctgatgcttaaatgacaaaaaagacaggaagaagtagactctttctgtcttttttgtttaacataaaatcgattatgtttagcggagttttcttgctaagacagctaactgtaagcatatatattttcttgcttataattagaactcattcctatgtccaaacttgattatggtagatagaaatgaattcttatatgaacaataggtttgattgtatgttaaattttaaaggaataaacgagtctcatcaattattgagactcgtttat

SEQ ID NO: 42 - DNA, 483 bp, Pseudomonas sp.
  misc_feature 1..483: note = Marker nucleic acid sequence
  source 1..483: mol_type = genomic DNA
aacaggaagggtatgggtttgctccgaaaggcctgtcacctagcttcagttcgctacgggcccagtgtggttggcagttcggcaatattcaagatttcgcgtatcggtagcaggggatctcattatccataagcggcttaagaatgcaacgcaggtgctgcgactcgctgaccattttctactatggcagtggacacaagcgaatgcagggtccaatgctgctctggaaaaaatgaactatttcaccttgagcttgtcgcctttttcgatgctatctctagtgctgcgaaaaaacagttcagtcgcaagcattaccagtgaaagcttatgaagctcttccgttttggacctgcacacttaaagcgcatagctaagtgctccgcatatctatgggggcacggagcactcgtatcaccatcggattcaggcttgggccgggtgctgatcggggcagattttcggagatttggatgtttttcccat

SEQ ID NO: 43 - DNA, 474 bp, Pseudomonas sp.
  misc_feature 1..474: note = Marker nucleic acid sequence
  source 1..474: mol_type = genomic DNA
gcgcaggttggtgttgttgcaggacctggttgctgccaaggagtgatcagttaggggtatggcccaaggagttcgaagatatgcccataaaacccaggcccttcacttttgagtgtgaaggttgtggttggacaaagaccgtggcgccgcagagcgatgcgttagcgccgggcgagtggattgatcagtgcccaaagtgtggcgaaaaaaggctgaaagtgcacgcagcggggtggctcgcggcgtttttggccgggttttgggcacggcggcggtaaagccattttcggtcaatatgccttttggatcagtgctcaggagaatggcaaacaaagatggctatatgccattctcctgggagcgtttaccatgcccgaaggcagcggtgaaggttttcagagccaagcctctttggcgctagcttgagagcatcccaactaatgaacgctcaggactcatagctcgttgagtcca

SEQ ID NO: 44 - DNA, 472 bp, Pseudomonas sp.
  misc_feature 1..472: note = Marker nucleic acid sequence
  source 1..472: mol_type = genomic DNA
acgcgcatgctcgctcagcgatgtatgcacgcgcaggccttcggccacgatctgcagtacgctcatgcgcgggctcaaactgccgtaagggtcttggaaaacgatctgcaggcgtttgcgccaagatttcatccgcgccggttgcagcggcaccccagcgaactccacctgccccttggcctcgatcaacccgaggatggcctgaccgagtgttgacttaccggaacccgattccccgactatgcccagggtcgtgccacgtcggatcgacaagtcaacgtcgtgcaccgcctgcagataacggcgcttccaaaaatggccaccaagcgcaaaccgtacgttgagcgcacggacgttcaacagtactggtgcattggcttgcgcaggctgctggatgccaggctcggcatccagcaactggcgggtgtaggcatgccgggaatgctgaaacaacacctcactgtcacctttt

SEQ ID NO: 45 - DNA, 472 bp, Pseudomonas sp.
  misc_feature 1..472: note = Marker nucleic acid sequence
  source 1..472: mol_type = genomic DNA
agcacgcccgcttccacagggaccgcacagatttcaaatactgtgctgatcctgtgggagcgggcgtgcccgcgaagcgttcaacgcgtgtgatgctggggctacagcaaccgctccctggcttgttgcatgcagtagcggcggcaactcttttcatttgtacctatcagttttgtcaggtttcagcccccgccaactcttatagcatgcgcaaaaactgtagttgccaaacttcgacgcccacagtttgaaacacactcgataacgtgatcttcacgttattggctgcccctgagcgtatcaaagaccgacaccgcaatcactgcactcatgcaaggacaagccatgaccctgcaatccaacgcattcaatttcgcaagttccacccgcagcgacgtcgacccgcgtaccgggctgtgcggcttcaccctagaagttccaccgctcaacgccaacttcctgcaaggccctg

SEQ ID NO: 46 - DNA, 488 bp, Pseudomonas sp.
  misc_feature 1..488: note = Marker nucleic acid sequence
  source 1..488: mol_type = genomic DNA
caggaaggatgaatcatgcggatgtggatgagagacccggggcggcttatcagccgattgataatggcgagtatttgcgttatcgcggtaatcgttgacacgcgggtattagccacacctcaggtcactgaagaaatcaggggactcctggattttgtagaacacagtgactgcaagtttgttcgcaacggcgtcgaatactcaggccccagggctcgagcgcatctggagcagaagctgaattatcttgaaggcaagaacctggtgaaaagcacggaagaattcattgatcttgccgccactaaaagcagtttgagtggccgtgcttatgaggtgcgatgcgcaaaaggtgtagaaccggcaggtatctggttgcgcagagagctgcagaggcaacgacatggaacggcaacgtgaatcccaagtagtcgacgaagcttcgcaagcggtacaagacgaagataaccggatgaccgaagtcaaccgcc

SEQ ID NO: 47 - DNA, 429 bp, Acinetobacter sp.
  misc_feature 1..429: note = Marker nucleic acid sequence
  source 1..429: mol_type = genomic DNA
ctttttattctaaaattaaacaataaaaatttatctatatttttatattaaataatgaactaaataacaggctttaactcctattaaattttctcaaagcaaaccttaaaaagagaacaaaaaccacccaaacagaatttatattctcaaaaataaacatcaactgattaaattttaattcatttattaaaacttaattatattaagctatttaaattattatttagtttctccatctaaaaattcatacaattccattttttaaataataccttttacaatcaatatattataaataccaaatagtaaataaagcccccattacacccattattttttgattttataatgataaaaaaatcatttgttttctttatataaaaaagtaaaaaaatcgagataaattagaaaaacttaatagattttttt

SEQ ID NO: 48 - DNA, 492 bp, Acinetobacter sp.
  misc_feature 1..492: note = Marker nucleic acid sequence
  source 1..492: mol_type = genomic DNA
ataaataagaaaagattactttgacaacatataggaaaattatgctatttctgaaattatcactgaaatataaattttggtttatataataaaaatgcaccttaaataaggtgcattttcttaattatattatctttgataattataatgtagtaatcgtacctgctgttggtgtgcctccaccggtacaacccttaggaataaacttatcatccgtagtaggaatatctgtcgaacaactccagccaccatctgcagtacgacttaatgataagatttttccagaaattttaggattaccttgaagcgtacaagtgattgcatttgttactgccccattagttgctgtaaatgctgtaacaccgtaagcgctacatgcatttgaatttgccgcagtaaagcccacgtcacctaaagctgctgggattttcccttcatttactgcgtcttcataacctgttttcactgcactaatctcagaatatccagcat

SEQ ID NO: 49 - DNA, 446 bp, Acinetobacter sp.
  misc_feature 1..446: note = Marker nucleic acid sequence
  source 1..446: mol_type = genomic DNA
taactttccactggtggcactattatcagttgcataaacgattgagttcttgctggtgtaaacgatttgctccgttttactgagatttccagtagtagagttataactccatgcaattacccccataaaattggcacgggttgaggtgtaatacggtaaaaataactccgttcctgttaagcctccacgggtaaccacaatggaaggtccataacctgctacaaatggatttgtataaataatggatggtgcatttttaaatcgagttttttgcatacctgacttataaataacatccagatcagtttcggtttctgaagctggcgatgctccatagcccatattagcaacaccataagatccaaaagtagcaacttctccagcttcagtaccggaatttcttgttgcggcactaccaagtcctgtcacctgcgtccagtcgggtg

SEQ ID NO: 50 - DNA, 428 bp, Acinetobacter sp.
  misc_feature 1..428: note = Marker nucleic acid sequence
  source 1..428: mol_type = genomic DNA
acctttttttgtgaataccgcagtgaaaaaaggtgaacaggctaaagttggtgatgtttccattaaaacagttaaagatagtatgtccaaagatatggatcctaatttatctacgttctttatagatttcttggataaacttggaagaaagactttacctggagaattaagtggtaatgcgaatatttatggattagatcaatgggataatccaggtacaggcttggaagcggatgatgttacaactttagggattatgaccaattatttttttacagataatatctcgctagaaataaaggccggcgtacctccaaaagtagacttacagggcaaaggtaaaatttatgccccactaaaagcccaagctcatccatcaattgaacttcctgtaattggaggaattggcttaccttcaattgatttag

SEQ ID NO: 51 - DNA, 255 bp, Acinetobacter sp.
  misc_feature 1..255: note = Marker nucleic acid sequence
  source 1..255: mol_type = genomic DNA
catgatactttaactagtaaaaattcccttaatctataatagttatctgttaaaaagcctcttcaaaggggcttttaattctttcttttgctctgtcactttcatttgatagtaattgattagttttctttacacataacagatttttacatccgtactagttcttctttatttgcttttgtccaagtctttctatttataagcttaaagactttataaactggtttaataaattaattctaaatataaaaacta

SEQ ID NO: 52 - DNA, 497 bp, Microbacterium sp.
  misc_feature 1..497: note = Marker nucleic acid sequence
  source 1..497: mol_type = genomic DNA
tctgaagcgcttcggcggtgtcgacagcgacgtcgtcgtcgcggcagccggcgccgacgagacgccggacggcacgggatggcgcacgcgcgtgagcctccacgtcgacgggcatggacgcatcgggcccttcgccgcgcgctcgcaccgcgtcgtcgaggtcgacgacctgccactcgccaccccggcgatcgccgaatcggtagcccgcggccggtcggccgctcccgggcgcctcgacctcgtgcagccctccgacgggcgcgtgcgagccctggcccgcccggagacgccccgccgtcgaggtcggggcggtccgcgtccggtggccgacccggcgctgcgcgaaaccgtgatcgagagggtcggcgaccgggagttccgcgtcgacgccggagggttctggcaggtgcaccggctcgcgccggtcgcgctgcgcgacgcggtccacagcggcctgcgatccgccggccgcaccgtcgatcccgacgcatggc

SEQ ID NO: 53 - DNA, 476 bp, Microbacterium sp.
  misc_feature 1..476: note = Marker nucleic acid sequence
  source 1..476: mol_type = genomic DNA
gcacgaccttcgctgaccctcgacgctccggcgtcgggggtctgtcttttaccgggcggcgttacgcgtcggggccggccggggcggcggtcgcgcgggcgctctcgatcaccgcggcgacgcgggcgggcgtccgcgaggagaacacccagtgggtgaccggatcgtcgtcgtcttcgatcgcgatccgtacgactccgtcgatgccgccacgcagaaggtgccaggagctcgacgacaggccgggcccgcgtgcctgccgcgcggcgtcgccggtgaacgtctcgatctcgccgaggtaggtgagctcgatgctcgcgcgcccgactcggagccgctcgccggtgacttcgatcaccggcgagagggcgatgagtcccgccacgacgagggctcccacggcgatgccggcgatgagcccgaccaccgagtcgagcggggcgagcacgagagcgaccatcggcccgcagacggcg

SEQ ID NO: 54 - DNA, 489 bp, Microbacterium sp.
  misc_feature 1..489: note = Marker nucleic acid sequence
  source 1..489: mol_type = genomic DNA
tcgcgccgccctcgtgctcgccgacgccgcgcagcgttcgctcgccgagcgcgcggccgtcgccgtctcgttcgactgacgcgcgaccgcccgcccggatcgggtcagccgactgcgtcagcggatgcggcgcagccgcacctcggcgcggccgggcgtcgtgccggtgaggtagacgcgcggcccgccgagggcatcggtgccgccgaggtacgtgtagtcctcacccgggaggtagccggcggctccgggcaccccgcggtcgacgccggccgcgatgccgaactcgatcgcctcgtcaccgacgcggtagcgcgcggtgcccgcgcccaggacgccggtcccgtcgggtgccaggtcgaggccctcgaaggctccgccgggccggaaggcgagttccaggctccacgtgcagagcggcccctcggtatcgatcacgaggtcggcgccggtctcggaggggcgcaccgcgatgcgggtgtgcagggc

SEQ ID NO: 55 - DNA, 499 bp, Microbacterium sp.
  misc_feature 1..499: note = Marker nucleic acid sequence
  source 1..499: mol_type = genomic DNA
gaggcggtcccacatccgctggctgtcgccggtctcgacgggggaggtctggtcggccgcgacgttgatcagggcgtgcgaggtgaggatgaccgggacgtccgggtgcgcgtcgagcacgctctgggcccaggcgagcgttgcgtccgaggcgttccaggcgacggcgagcgacatgaaccgctggccctcggcctcgaagatgtggaactggctcagccccagcgggtcgctgccgccgtacgtgctctgcgtcgccgcccgtgtcgcaccgaaccagcggttgaagggctcgttcgcgatgtcgagctggtcatcgcggacgccgctgttgagcacgtcgtggttgccgggcaggatcgaatacggcgcagcggcctcatccatggtgcgcatggcggcgtcggccgcacgccactcggcctcgaccccggcgcggtcgacgatgtccccgaggtgcagcgtgaagggaatgcgcaggtcgtccgcgtgagccgtc

SEQ ID NO: 56 - DNA, 423 bp, Microbacterium sp.
  misc_feature 1..423: note = Marker nucleic acid sequence
  source 1..423: mol_type = genomic DNA
ccttcctgcgggtagcgcacgccgatctgatcgcggatatcgtcgagcacgcccatgatcgcgacggtctctgcgatcggcagaacgtcgccgtcggtccgtccggcggcgacgagggcctccgcctcgagggcctggaactgcatgccgcgcccctcgatctccgagcggtactcctcgaggatcgtgccgtcgtgcgatacgacgcggaagtcggtggccgcgtaccagacgcccgagatctcgacccgcgcttcggtcccgacgatgtgagcggtgttcggcccggccccgcgggaagacgacacggtcgtcgagaccgcacccgaggggtgggtcatgaccgtcgcgacctcggcgtcggcgcccgtctccatcagccgcgcgagcgccctcacctgcgtcgggagcccgaggaggtcg

SEQ ID NO: 57 - DNA, 500 bp, Pseudoxanthomonas sp.
  misc_feature 1..500: note = Marker nucleic acid sequence
  source 1..500: mol_type = genomic DNA
tcggaactccaatgtcaggcgccgcctcgatggaatcacgcgagcgccgtcgcgccgaaggggtggggcgctcgcgatccgatcgcgccgatcgctggttgtatgcaatcgagacggtcgtacttgggctgccgaccctcggcgttgccattccggggctgctggcgctcggattcatggtcgtggcggtcgtcttgaccgagtttggcctgacggcgctgtgggcggggttgatgttcgcgggcggcgccatcggcgtgacatcctggttcgtactgtctggtcttgtgttgcttgagggaaggaaaggattgcagcgtgcgaacccggcgtggtggctgggtcttctcgcgggcattgctacgtcgggctcggtcggctggccgatggtgatcgacgtgtttgccggcctgcaggagcacgtcgtattcggcctcttggcgtcgggtcttctgttgtggatcccttccctccatttgattctgatgcggttgaggacg

SEQ ID NO: 58 - DNA, 499 bp, Pseudoxanthomonas sp.
  misc_feature 1..499: note = Marker nucleic acid sequence
  source 1..499: mol_type = genomic DNA
cgccgagggtggcgttggcgcgccaataatcgttcatccacaccacggcggcgaaagccgtgctggccatggtgaccgcgaccaccaggtagcggttgccatagcgcagaccgttgcccacggtgatccacatcagcaccacgtaggcccacgacagcggctcgcccatgccgttcatcgcggcggccagcaggccgtagtcggcgatcatgcccagcccgcgccgcacgtgcgacttgcccggctgcaccaacagccaggcaatgatgcccaggccgttgaccaagcccgagacgatgatggtcaggacgatggagtattcgtcagcgggcagcgccgcgcgcgacgagggcagcagcgcgtagaccaggatgatggaaatcagcgcgacacggatcagcgcctggccgtgctcgctgtcgccgcgatgctcaaggcgggatttgacccaggtaaggacgttggacatggctcactccatccctggacggctctgcac

SEQ ID NO: 59 - DNA, 498 bp, Pseudoxanthomonas sp.
  misc_feature 1..498: note = Marker nucleic acid sequence
  source 1..498: mol_type = genomic DNA
aggagggcgaggaaggggtgcccgtcggcactacgccagcgacaccgccggcatcgccgacaccggcgccggcgcagccgacgaatgcgaatccgagcccgggccaggttccgagccaggttccgagcccctctcccgccgggagaggggttggggtgaggggcgacggagaggggatgggcggaggcgttcatggcgtggccgcgctcgtaccttttcgctcgaacatgccggccatcgcgcctgtcctgaccctcacccccacccctctctcccacggggacttccttcggtcgccgcagggagaggggcttgaagtcgcctctgcgtcgaggaggtcggcatgaccgaactcctgcgctggggcgtcgatctgctgcgccacctgctgcgcacgctcgactggccgttgctgggcgcgctgctggcgctgatggcgatcggcctggccgtgctgtacagcgcgggaggcgaagcactcggttcgcacctggtgtt

SEQ ID NO: 60 - DNA, 496 bp, Pseudoxanthomonas sp.
  misc_feature 1..496: note = Marker nucleic acid sequence
  source 1..496: mol_type = genomic DNA
ggccgccgcgccaccgacgaacgtcgcggggggatttgtccggttcgttcgtcctgatgtccagaaggcgccattccgagcgccccggggagagtcgtccatgcggtatccaatgcgagtcctgctgttgagcatggcctgtagcgcggcgctgtccgcgcaggcccaggcggcccccggccgcatcgacctgcccgccggcgagctggccacggcgctgaacacgctggccaagcagtccggcacgcagctggtgtaccgcgccgaccagatgaagggccgtcgcaccacgggcgtgcagggcgccgcgaacaccgaccaggcgctggaacggctgctcaagggcagcggcttcgaagccaagcgcgacgcctccggcgcggtgctgatcgtgcaggccgccaccaccccgcgtcgtgccccggcgccgcgtcccgcgcctcaggaggcgcctcccgggggcggtgccgcgcaggccgaagaacccgtaacccag

SEQ ID NO: 61 - DNA, 492 bp, Pseudoxanthomonas sp.
  misc_feature 1..492: note = Marker nucleic acid sequence
  source 1..492: mol_type = genomic DNA
gcgaacgacacctgcaagggtcgcttcggcgacgacctgcgcgggcagctgcgcacgttgatgacgcgcctggcggccgcgccggcgaacaccgagtaccgcgatccctccactggcgaactgctcaccggcgaggtcaacgccggcacggtggccggcatcacccgcatgtattcgtactacccgcagggcgccgcgctgctgccgctggtcctcaacgaagcccagcagggccgctacggctcactgatgtcgctgtccaagctgctggaagcgcaggtgggcgaccagttcatgcacgggatgcagctgtcggtgatctgcgccgaggacgccgatctcttcaagaccgacccggccgacggcgacaccgtgctgggcagtgcaatgggcgacacgctgaaggcgcagtgcgcggcatggcccaccggcaagcggccggcggatttccacaccgcatggacgtcggacatccccacgctgctgacctca

SEQ ID NO: 62 - DNA, 493 bp, Chryseobacterium sp.
  misc_feature 1..493: note = Marker nucleic acid sequence
  source 1..493: mol_type = genomic DNA
ggtagtgacagccgaatggaaccacgttttatctctaagcctgtaaaacccgatagcttttcctttgggaatgatagcataaccatcccacttgtcgcccgcaggatagttgaatttattgagccatccctgtgcgcggaactgtacaagttcatccggagatatagctgcacctctcatatacagggcataagctaccacatcgtggcatacgcccttgttgtaattagccatctcgtcctgcccggaaagcaggccattggatatcagtgatttttttactggttcgaattgcccaacctgggctccttttggtgtgatcatttcaatatttttaagtgattaagtgtgtgatgtttggtacttaaagatataaaataaattttaaatcgtattttaattttaattgaatggcaaccggaggcttagatttttctcagtcaacctataaataatgaaatttttaaacatgaatctgtaataaaccgttgaa

SEQ ID NO: 63 - DNA, 497 bp, Chryseobacterium sp.
  misc_feature 1..497: note = Marker nucleic acid sequence
  source 1..497: mol_type = genomic DNA
cactccagaatctattgattcagtggaaaaagttatcccttacattaccgatgaagtaatgataggacatgcattatccatttccattcccaaaaatgtaaaaaagattaaagatggagcttttcaatattcagggatgggctatcagattattgaagtgaactttaatgaaggccttgaggaaattgggattggtgtattttcatcccaaaatataaaaaaggttaaaactccttcaacattgagaattattggtagtggtgctttcagtggacaagctagtcttgtaaatggagttatgacaaatgaatcatactcattagaagagattatcctaaatgaaggattaatacgaattaacgattatgcttttaattcctcacaagctacagttaagaatgtttatatcccaagttcagtccaatttgttggacaaaatgcatttgccattccttcgctacaaactgtttcagccctaagcggattagaccttacca

SEQ ID NO: 64 - DNA, 478 bp, Chryseobacterium sp.
  misc_feature 1..478: note = Marker nucleic acid sequence
  source 1..478: mol_type = genomic DNA
gagtaccatataatgctgttgttttagatgctgccaaagcacaagcattaaacactttactttacggaccttttaaggctgtacttactgcttatgggcagggaaacagacttaatttagtagcagccgggaacaatcctgttcttattaaagataataaacttaccaatctttctgtacagcttacggcagctttagcggctaacgggtatacgcctaccgaggcagctttccttggaaatgcttttgggcaggctcgtcaggcgaaacagggagagttaattcttcttacagcaagtaaagttcttggacttgatgcgctgaccaatctacccgctacgccaacttcaaagtttatctatggagcgagtttcccaatcggggaccaactttcattaacagctgatgaagtagcaaatatcggaaatgcagttaaatcatataacgcttccataaagacaatggctgattcttatgg

SEQ ID NO: 65 - DNA, 491 bp, Chryseobacterium sp.
  misc_feature 1..491: note = Marker nucleic acid sequence
  source 1..491: mol_type = genomic DNA
ggagccatagggaatatctcacctgggtttccgcctccgcccgaacttacggtttccttatgatggtactggaagccatcaagataatctgtttcctccgtaatggtagtagaggtattgtaaccagagactacattgatggtgtttttctttaccttaaatccatctgcactatagaggtattctgtagtgtaagagcctccattgtacatttcaattatttggggaagattcagatggttgtattgtatggaggaaattccttttcctggcatattggtcatattaccgttggcatcatagtttatggcagtagaaaatgaacttgcggcttcataaccacttgggtttcctgatgcgtcatccagctgggtaagcctgtttccctggtaagtatactgcaggttgtctatcaccgttgccgtggtatttccgcctattacagatgttctgtacagggaggtaatgtttccattgagatcatacgccag

SEQ ID NO: 66 - DNA, 490 bp, Chryseobacterium sp.
  misc_feature 1..490: note = Marker nucleic acid sequence
  source 1..490: mol_type = genomic DNA
ggtaatacattaaaaaatactctgtaaggtgatatagatatttccacaaggtagttgatgttatgaattatcctttaatttactgttattcctaaagtctatgatggaatattcctatatttgaaaataatgttgtgaactgatgaaatttggaatcagtacaatgcaggctaatttgatatttactatagaaataacgtctataagatttttcacagaccttatagaaaataaataccatgagaggaatcaattatgaagactaaaaatagagcatttagatctgatctgatcgttaattcacctatattgggcaggcaatatggaaactagatataagtggttcaatggttacagcattgttaccggggccgttcgctacgcagacctctgctatttgattacggctaacgatgctgctatgagtgaagggtacacagattcgtcaatactgtacagtctttatcgtggaacctggtatgctgatgca

SEQ ID NO: 67 - DNA, 497 bp, Erwinia sp.
  misc_feature 1..497: note = Marker nucleic acid sequence
  source 1..497: mol_type = genomic DNA
tgccagccaggcgcctgtgccgactgaccatttttcagccttaacggataatttatcttcagacatcgatcttgcgactccctgatagttgcaaaaataaacaaaatagctttctggcaatttttgttccgcatagtggaattaattacctattcaggctaaaaatagaggggccgttgccgatatttagccacccccctgatacggactgcagggatcgtgccagaaataagtgggttattttattgcggcaatagatcgcggcagcaacgggaaatttggctacgcgggcagggttaaaaaagttaatttattttcactggtgaaataaaagacgctttttttctcatcctgccagggatattcttagcggggcggcagtgagacaccaccatggatcagttgcaccagcgtggggcaaacgttcgggaaagttggagagagcgatgtcagaggtgttgagagaggtcaaagcggtgtcgcgcacagcgtccggc

SEQ ID NO: 68 - DNA, 500 bp, Erwinia sp.
  misc_feature 1..500: note = Marker nucleic acid sequence
  source 1..500: mol_type = genomic DNA
tggcggcgacggcggcccagctcagctacttcccctcagcctccagcgggctgacgctctggcaggcggtgggctgcgaacgctgccatcacagcggctatcgtggccgtatcggtattcatgaactgttaatcattgatgaccgcctgcgtcgggcgataagccacccgcacagcgaacaaccgctgcatcaactggtcagcgctgactatcagaccctgcagcaggatggcctgcaaaaagcgcaggaaggggtcaccacgctggaagagatcctgcgcgtcacacggaatgaaagctaagatgcgttttcgttatcaggccgttaaccgccaggggcagcgcgtgcgcggggagctggaagccgacactgcgcagctggcacgccagcggctgcgcgaacagcagctacagccgctgcagttacgggttcagcgggcaggcccggggctgcacctcaagcgcagcacgctctccgccggggagcgcgtgctgctgat

SEQ ID NO: 69 - DNA, 497 bp, Erwinia sp.
  misc_feature 1..497: note = Marker nucleic acid sequence
  source 1..497: mol_type = genomic DNA
agtaagtaaggggttaacgaatgaggaaaatgtcctgcatcgtcgtggttttgccattggccagctgcagcaccgcgccctgagcaccgaaggaaaccccttcaattttctcggcgattaaaccggcgatctcaggggcatccccttcagcggcagtggcgctataggtgacgctgtattccacatctgcctctggctgagagggtttaaagttctccaggtcatcaaggctgaattcattgatcccggccctggtcttcgagcctttcagctcggcggtataggccttgcctgacgcatcggtcagcgtcacggtgaccttctctgcttcgccgccgagtgcaaacttcagtggcttatcggcattgatggaattctggctccaggtgactttctgttcgccctcaaccatcacctcacggcccacccaggaggcggaactcatctgctgcatgctcagcagcagccccccgacggagttgaccgttttattcagg

SEQ ID NO: 70 - DNA, 498 bp, Erwinia sp.
  misc_feature 1..498: note = Marker nucleic acid sequence
  source 1..498: mol_type = genomic DNA
cgcgaggccgcagcggaaaaacaccgcgataacgccagccatcagcagcatctcagcgcggtgttcgctgccttcccggatgatgccgcaaccttacggcgcgagcagctggcgtggtatcgctaccggcgtaatcagcaggtcagcgcgcagccgggcgaagatctggaaagcctgattgcccgtggcgcggtgacggccgagccgattatctacgaggattttttgccggtgagcgcggcggggattttccagtcgaatctgggcagcgatgccagttcagtgggcagcggcaaccccagccaggcggaatttgaacgggcgctgggtgccgccgtgattgatgagttcagcctgtaccagcagctgcagcaggattccatcgagggtttgttcacgtaggggcgcggcatgccgcgcccggggtgattgcgcgcagatagcgggccaggcgtgcctggcccctacggccatcaaggatgaaacggagccgttccg

SEQ ID NO: 71 - DNA, 498 bp, Erwinia sp.
  misc_feature 1..498: note = Marker nucleic acid sequence
  source 1..498: mol_type = genomic DNA
gctgggcatggccgataacctcaatgacgtcagtaatctgcagaacgacccgctgcgcgatgccctgcatctcaacgagggtgccagctggacgcgggccatgagctggacggaaaacggccagccgcgcgccggaaccgcaacctcccactttacccgcctgaaggatgaggtgctgcagctggccggtgagccggtggcgtgccgcgtgtggcaggaagaggtcagcgccgacgacggccagtcctggcgcaatacgttctggattgataccaccagcgggcaggttcgtcaggcccggcagatgctgggtgcggacattatcccggttgaattcactatcctgaagcctgcgaaatcatgaaaaaaaccatcacaactcttctcgcagggatagtggcatcgctgtcgctgcaggctctggcggatagtcaggtcacggtattttatcccgggaacacggcatcggtgacgatcggccatgccgaaaatctcgcg

SEQ ID NO: 72 - DNA, 492 bp, Pseudomonas sp.
  misc_feature 1..492: note = Marker nucleic acid sequence
  source 1..492: mol_type = genomic DNA
tatccagatataggcggttctcgcatgggggcgtcgatcatggactatttgctcggtttgttgggtcgggtgacggacagtgaggcactggcacgtctgctgattgttggtgcaattgggatgagcacggtcatcgcagtgatcactgtgacgttactcgttttgggcctgcggagccctctgcaacgccgtcttgcattgatcaagcgtggccactccagcgttgcagccggacgtgaggcgccaggaaacctgcaactgttactggaacgggtcggtcggcgcgttactccgtctgcggaggggcaggtgtcggccacccgagccctgttggcccacgcgggttacggctcggcttcagcggtacaggtgtactgggcagtgcgtttgctactgccgttgatgatgtcaggtatctcgctgttggtactgcccctggttccgaaactctccctgatgacgggtataggtttggtagtcatcggggccgtg

SEQ ID NO: 73 - DNA, 489 bp, Pseudomonas sp.
  misc_feature 1..489: note = Marker nucleic acid sequence
  source 1..489: mol_type = genomic DNA
ttctgaagtctcagaaggcggcgctgaccgcagagcgaatggcactcgaagaggatgcccagcttaccggcgatgcatgtaagccacgtcttgcgaagatcaaggcgcaacaggttcaacttgaaagtcagcagtccgcgttggagctgcagtaccagcaagaactcgacctcacccaccggttgctcaatgctcgtcaggccgagcaggtcgatacagccgcctgcactcagcttcaacaagacctcagctacgtgcaggggagtcgaccactgctgtcgctcgacgtatgtacccgcagtgtggctgaggtgatcgccgactggacgggcgtgcctctcggcaatttgctgaaggacgaacacgcaagcttgttgaacctggaggaccagttggccgcgcgtgttgtcggtcaagagccagccttgcttgcacttgcccaacggctacgtgccgctcgaacgggcctcactgacgacaaggcaccga

SEQ ID NO: 74 - DNA, 451 bp, Pseudomonas sp.
  misc_feature 1..451: note = Marker nucleic acid sequence
  source 1..451: mol_type = genomic DNA
agagccccagaacagctgggcggatctcgtcaaacatgatttgggcatgcttctgcagcgtctgccggggctggagatgctctattggaatgacggctcggcatttgctgaagaagccacgcgagaatggatcaaccagcaggtcagtggtaaccgcccggaacagtggctgcccgcagctgcacctgccacatcgacgggggcatgcgaaatactcgctttggagcccgaagcactggcacaagcggatgccgacggtgtggagcaggcgctggcctggttggcgagccggccggctgtacagaccgggcggcagcgctggctcctgcgtttgctgatggcgcgagtggcggagcagtgcggcaaggctgagctggccatccatctgttcacggagctggatactgctgcgcaacgccacacctttgccgactgggagccggacctgctc

SEQ ID NO: 75 - DNA, 448 bp, Pseudomonas sp.
  misc_feature 1..448: note = Marker nucleic acid sequence
  source 1..448: mol_type = genomic DNA
agagctcaaccgcacctatttcaacctgtcccagggcggtgaaatgcgaggggcgtggaaccaggggcaggactggatttatgtcgacgagcctcaaccggcggtagacggcggcgatggctctgccagcatccagctggacgagcacagtgcgtcggtggtcgaggcaatgaagcttcgcacccagtcgaacccggaggcgcaaccgctgactggagcggagctgggcaaggtcaacagcggacagcaatgagaaatgcccgcgtcggagttgatccgtcgcgggcagcacacttagcgcttggctgtggcgtcagggtcggccgagcgggccagaaacgcccgggtgacctccggcagatgttccttcagccattcggccatggcgacttcttccttcagaatcgaacgacatgcctgtgcagtggcgctgtccccggccgcctcg

SEQ ID NO: 76 - DNA, 345 bp, Pseudomonas sp.
  misc_feature 1..345: note = Marker nucleic acid sequence
  source 1..345: mol_type = genomic DNA
tggaggattggagatttctctgtgggagcggccttgtgccgcgaaagggccgcgttagcggccccatccatttctgcagtgactaaaaacccggggccgctgcgcagccctttcgcgacacaaggccgctcccacattccgtactcagaaccgagcgagtgcttttgcccaccaaatctgttcgtcaaggtgtggataaagtgtttgtgcttcgctgcaggcctctggattcaagcgttacgaagatttgggcaaaaagtgatcatgatctgcttctgctctacagatgtggcaaggatcgaggttttctcgcgttatccacaagcactttcagtcgcgcgaagt

SEQ ID NO: 77 - DNA, 497 bp, Pseudomonas sp.
  misc_feature 1..497: note = Marker nucleic acid sequence
  source 1..497: mol_type = genomic DNA
atgaattatgcgaactggcgagtgggcacccctcgctgcaggtggagctgctctgcgcggcagaattgcctgcggctttggccgaactgaagcttgttgcgcgacaaaccatcgccttactctgcggcaacccgaataacgtcgaaagttttacccggcgcctttatttggccggtatgccgcgcaatcagatgttttccgacctgttcctgccgcacgcctgacgcgcggcgggagcactcgagtcaagccagttcctgcgggtctgcccctgtctgtcgttgcacaccgcctttcggtgcgccgccgtacgacctttatatccattgggcccctttgcccgccccattaggacatgccatgaacgatcacctgctggttgaccgcgagcacgggttggtaaccctgcgcttgaaccgtttggacaagaaaaatgccctgacccgcgcgatgtatggcgccttggccgaagccttgaatcaggccgatcaggataa

SEQ ID NO: 78 - DNA, 500 bp, Pseudomonas sp.
  misc_feature 1..500: note = Marker nucleic acid sequence
  source 1..500: mol_type = genomic DNA
ccgaacgaccttaatgcggcggcaatagcgagcagactaacggaatacagggacgttcggcagtcggctgcggacaccaatctgcaccgctgacagcgctatggcgcgatgagcttcatagattaaatatgccaggcctgcgaaatcgtagggcggacatgccgcaggcttgtccgccatctgggccgtcaacggtggacaaggcttcgccatgtccatccaaatcggctcctaacgcccggattgcgcagtgttccggtttcataggtttagctgtcgcggctcttatgcagaggttttgcccctgaccagttaccttgaacttgccgcaccgcctgggggacttatcaatatgcagccgccgcgctccagccttatgcagtccactcaggcgtttcaatccaagtggctgccctggaggactcgtgaggggttcgttactgcgccattggttgctggcgctgggcctgctgctggtatcggttgggctgctggccgca

SEQ ID NO: 79 - DNA, 498 bp, Pseudomonas sp.
  misc_feature 1..498: note = Marker nucleic acid sequence
  source 1..498: mol_type = genomic DNA
tgaacgacaccgcgcctttagttgacgcatgctttcgcggtttgatttgcgattggtagggcctacaaccttgtagggcggacatgccgaaggcttgtccccatccaggcgtcgcgtcagcggcggacaaagcttcgctatgtccaccctacaaaagcgcgcctcgcccggatgcaatccggaaaatcgaatctatcaagccagcccagcaccataccccgcctcggcaatcgcgatgatcagctcgtcgctcgacagtctactgctcacccgcacttcaccgccggccaacttgaccttcacatcggcggccggatcgcgcgcctgcaaggcttcggtgatggtcttgacgcagtgctcgcatgtcatgcctagcacgttgagcgtatgaacctgtggtgcttgcatcgataaactcctgattgaaagtaagtcgccgctgtgggacggcggccagtgtcaggcttaccccatgggtaaggtcaagcgataaaaagc

SEQ ID NO: 80 - DNA, 497 bp, Pseudomonas sp.
  misc_feature 1..497: note = Marker nucleic acid sequence
  source 1..497: mol_type = genomic DNA
gcaagctgttgtttttccgcgaggccagcactgctttggatcaactcgtcccaggcctggatgcgctgcttggccgcgcccagattgccgtagcggttttgtgctttctcgatgatcagagcgaattcccagttggccagggcgctgcccaagccgatcagcagcaacgcgcaggcgagcagcagcacagcactgcgtgtcgctcggccgggttggcgctggcgtgactgcatcggccgtgcctctgctggggatgcggaaagtctaggcgttacccaaggcttttgctgggtgtttgcagtggcattgtgcgattgcggcgcgaccggtaaagcgcccccggattacctccgggctacaaggctggcttttgtagggtgtgacatggcgaagccttgtccaccgctggctgcccaatggcggacaagccttcggcatgtccgccctacgggacttgcggcttatcaccgactatttaccgatcaatcggggggttg

SEQ ID NO: 81 - DNA, 498 bp, Pseudomonas sp.
  misc_feature 1..498: note = Marker nucleic acid sequence
  source 1..498: mol_type = genomic DNA
ggactcggcaggatttttcttgccacctgtcggtcgctcgggcggctccgtggtgatctgaaagttgcgtttgcgactgtattcgctcgatggctcagccatgggaaaaatcctcccgcgagtctggttcgaggtattcagcggctggcggacttagccgatttcttgcgcgaacctttgccgggtttgaccgacgcttcgccatcgtccccagctgtttggcccttggcgccgccgctgaggctgcgtttgagcaactcggtcaggtcgtaaatatcggcgctggcgcgttcctgctcatcggccggggcctcgatctcttcgaccttacccttgcgcgccttctcatcgaccagttgcatgatcttctccgtgaaggtgtcctgatattcctcgggctgccagggcgcgaccatgtcttcgaccaggcgcttggccatggccagttcgcccttggcgagttcggcatcgctgaccttggcgctcagttcaaggcta

SEQ ID NO: 82 - DNA, 494 bp, Arthrobacter sp.
  misc_feature 1..494: note = Marker nucleic acid sequence
  source 1..494: mol_type = genomic DNA
atggtgggagcccggcgcggctttggctgagtcagacccacacttggtagccggtggacttgtcgaagagccggcgggtgctgataccggcgccggcgatccacaggaccgaatcgtcttccgcggcctggtcaaccacccctgtgatgacatgctcccccagcagccacacctctacggtgtgaccggtcaggcgcgcccagtcaccgcgaagcccacgcgcgtttttttgggctgtcggcttctttgccggctccttcttggccggggcgcggctgccgccagccgtggccgtacctgcggatgcgcctggtttcatgtgttcctccacgggccgggcaccaagcaccattgtcttgggccaccatacgagctgatatttcattgatatatcaaaagccagctcaagtatgttgcaggtcacatttcctgtcaatgaatgcccttggggcgcaggagcgaaccttggcaggaagcggagtacgtgccgcgac

SEQ ID NO: 83 - DNA, 497 bp, Arthrobacter sp.
  misc_feature 1..497: note = Marker nucleic acid sequence
  source 1..497: mol_type = genomic DNA
agttacgctgcgtccacggagagtgcgaaagcctcctcgtcgtagcatttgacccgttacgctcatccctaaagacttggattggtcttggcagtagccaggattcatccgggaaggattggactcgacacttgagccaatcaggtcgaataacctcatctagccgcaacacccgtgtggggacgtggaatcaattcaggatgcacaatgatcaccgacaatgacgtcgtacctgctgccgacaccctcactgcctggattggcggcgtctccaccgagatcggagaactttccgtaaaggttgcctcgctgcttgaagagaacctcgccggcaggtccaaggtcagcaaagctgcactggtcggactggatgaccttgcacgtgaattcttggggaagaactcttttgccgtcggagcaggaacctttttcgctggcgactttgctgaggagggcggccgggctttggagtggtggttccggaagaacgacggctc

SEQ ID NO: 84 - DNA, 497 bp, Arthrobacter sp.
  misc_feature 1..497: note = Marker nucleic acid sequence
  source 1..497: mol_type = genomic DNA
cgatccaagccctctatcagcccgttacccactgctcccgcctctgaacgcggcgcggaagatctggaaaggcttccatcctaagaagcgggtcacccaactggggcccgccctggaggccgcagttgggctaatgctgccggaatggcatcgaagaggacggaaggcaggccggtcaatccggcctgccttcctgtctttgatccccgtggtgtggctcgacgtggccgagcgtcagccaacgcccggaagaacgcaaatgaaacgtcttattaaacttttttccaaaagagtctggactagatgtattagctgggcgtagctttactagtgggacgcacgcagtgactcgcatcacaaaatcagaagagttcagcgtgaagcccggttcgaatcctcaagcaaacgggggaaagccccgggtttgcgacgatcccttccaaacgtcaacaaagggcattccaactctttcgtaacgctgtcccgtatgcgacaga

SEQ ID NO: 85 - DNA, 499 bp, Arthrobacter sp.
  misc_feature 1..499: note = Marker nucleic acid sequence
  source 1..499: mol_type = genomic DNA
agcgagcgacaacgtcgtcacacggcgctccgcagcgcgcagcaccagccaggagacccacacatcatgaacaccaaaacccagcccacaccaggcgccctagcactggacctgcaggacgaaaggctccaggaccggacaggtctgcgcggacagtacaaagcattcctggaccgcacccgttccggggacctcggcgtcctgcccgtcatcggcgggctggtggtcatctgggcggtcctccaaatcctcaaccccatattcctttcccctgccaacctggtcaacctggccatggaaagctccgcggtcggcattatcgccctcggcatcgtcaccgtccttctcgtcgcccagatcgatctctccgtcggctccgtcagcggcctgtccgccgccgtcgtagcagtcacctctgtgaatatgggctggccggtctggttggtcatcctcacgaccatcggcctcggagctgtcatcggatgggtctacggccaaa

SEQ ID NO: 86 - DNA, 496 bp, Arthrobacter sp.
  misc_feature 1..496: note = Marker nucleic acid sequence
  source 1..496: mol_type = genomic DNA
tgcgtcggtccttgcaactgtgacaaatgctgatccgttgggcatctcgacggcgcttccggtggagtccgagtctttgtcggctccggacttcgtggtttccggtgcggccttctgcactgccgttaccaggacatcgtggaacaggagacctgtggactgcttccagcccttgacctcttctggaacgcgtgcgttctcgggcattccgtcttcagacttgaaggaggtatatacggtgaccgtgtcgcctgcttcaatacgcccgcccaagaggcgttccggtgagagaaggagcgtcacttcctccatcccgtcgggtaccgggacggtccctggcaccagttcgcgcgggtccaccagccgcgacgttaggagttgctcgcctggttctaacgcaaccgatgtaacttttcctgtctgatcgccaagaccttcaagcgccccttctggaactgctgactgtgggatagctgccagttcaacgtagttattt

SEQ ID NO: 87 - DNA, 471 bp, Kocuria sp.
  misc_feature 1..471: note = Marker nucleic acid sequence
  source 1..471: mol_type = genomic DNA
atgcattcctggccgtcgaagacggacgctggcacggcggccgggtcctcgtcgcggctgaaacgccctgggcttcgttccgcggttagggcaccgcgggcgcggtcacgtcggcctcagtgaaagcagcctcgacctcgaccggggtccggtactccggtccttcgtggagccgcgtctcgatcttggcaactaccgccgccggggacgcggcggcgccatggtggggtgtcgaggattggtcgagcagaccgagctcaccgtgcgcccgccatctgttgacgcacgtgcttgtgcaggcacaggagaggcccatctcagccacggcgtgggcgatgggtctcgtgcggcatcgctcgatgagccaacagcgcccttcgaccgtcagaggcgcattcttgcgcgtcactaggccgcgccgggcgcggacgctcggcgcgcggtgtcgcggttgtcgatgccctggtgggc

SEQ ID NO: 88 - DNA, 428 bp, Kocuria sp.
  misc_feature 1..428: note = Marker nucleic acid sequence
  source 1..428: mol_type = genomic DNA
gaggtgcgccccgacggcaccgtcccggcgaccgatcggccactgcgccggtctccggagatggtcggggtggccaccgcggagatcgaccgggtcgtgctcgacgccggcacggggaggcaccccacaggcgaggaggacgcccagggcggcgcgatcgacgacagcatggaaagcaccacggaggaggcgcaatgagcgctcagcacacggaccaggacaccgcagggcaggagctgctcgggcagtacgggcagcacctgctcaacgtcttcggcgcgccccaggcggtgctcgtgcgcggacagggtgccgaggtctgggatgccgacggcaaccggctgctggatctgctcggagggattgcggtcaacgcgctgggccacgcccacccggcctgggcgcgcgctgtcagtgagcaggccgcg

SEQ ID NO: 89 - DNA, 484 bp, Kocuria sp.
  misc_feature 1..484: note = Marker nucleic acid sequence
  source 1..484: mol_type = genomic DNA
gacataggccgggctcgactcgtcgatgcgccggtcgccgatgcgcagctcggccgggcggtcgatcgcgatcgccgtgatccgcccgcgctcatccagcaccggcaggtggctggcgccggcgggcagcgccgcgcgcatctgctcctcggtggcctccgggccgaccgtggccggatgcggattggccacctgctggacggcgacctccagatctgcctccgggtgggccacgatccagcgtcggaagtccccgtcggtcagcgagcccagcagctgcccggtcccgtcgacgacgaacacgatccgctccgcattgcccgtcatcttgcgcagggcgaccacgacggactcgtcgtggaagaccaggtacggggtgaggcggcgttcgatgatcacgggggggtccttggttcgggggggggtgcggatggggcgggagatgagcccctcagtctgccagtcgggcgcggtgggccctgac

SEQ ID NO: 90 - DNA, 443 bp, Kocuria sp.
  misc_feature 1..443: note = Marker nucleic acid sequence
  source 1..443: mol_type = genomic DNA
ccagtgcttcggccaggtgcgcaccgcggcctccccggccgccttggactggccgtagacggacagcggggccacggggtgctcgggggcgtgctcctgatccagcggcagggagccgtcgaagacgtagtcggtcgacacgtgcgtcagggggacgtcgtgatcgcggcaggcggcggcaagcgcgcccacggccgtggcgttgacctgccaggctcgggagcggccctcggcggtctcggcctcgtcgaccgcagtgaacgccgacgcgttgagcaccgcgcgggcggtctccagctcgctgagcggccagctgcccgggtcctccatgtcccattcgccccgggtcagggcccggtgcgcgatcccgcgacgacggcaggccgccaccagggcacggccgagctgcccagcggcaccgaggatgagcacgggcgaggccc

SEQ ID NO: 91 - DNA, 479 bp, Kocuria sp.
  misc_feature 1..479: note = Marker nucleic acid sequence
  source 1..479: mol_type = genomic DNA
atcgcatccgtcgtcagatcgcgaacctgccgcgctgagcaggtccctgggcggcacacgcagcagcccccgtcgggtcgtcccgacgggggctgcgctggtcttcatcaggggcggcgccgcagccggcctcagtcgtgcaggtccggcagcacgcgcgcggcccactcctccacggaggactcccacctctgcgggtccacgttccactccttggtgtggcgggcgcgctggaagcccaccatctcgacccggtcgctgagttccgccaagcgcttggaggcggtgtccgggacgaactcgtcgtcggcggagtgcaggatcagcgtgggggtctgcagctgatcggcgcgcgtgatccagtccagcgagcccaggtccagcggtgcggccaggcccgtgagccacagcccgcgcggcgaggtgatcagggactgggccatggtggtgatcgctgaggggatgtgtcgcgacgccgt

SEQ ID NO: 92 - DNA, 491 bp, Pseudomonas sp.
  misc_feature 1..491: note = Marker nucleic acid sequence
  source 1..491: mol_type = genomic DNA
gaatttacttttgcgatttccaggctggccgcgaggtgctcaaactgattattctcaggtgccgatacttcaccaacgaggtccatgttggattcagacattttattttccttcaacggattaaatagaatccgaagtaggcgatagaacacgctttaatttgaaggccagaagtattaccaataaatcatatcagagccgccagacaccatttaaataccaaacttatcaagtatatgaccgagtgaatgttgccaaacaatagaccaaccaaagtcagccatacccattcactctaaaaccggcatcaggcgtggaaacttacaacatgaaaatacttgcaaagctgcctcttgaaattacaaacgggagcctcacgattactgttacaacaaaaaaagatcgctttctgcaacaatatccacattacttacaatgtagaaactcctgcaggcagcgaccttttccggaggtcttgcgcgtttaataac

SEQ ID NO: 93 - DNA, 468 bp, Pseudomonas sp.
  misc_feature 1..468: note = Marker nucleic acid sequence
  source 1..468: mol_type = genomic DNA
gcggttcacgccgaggggagacatccgttagaacgcgttgcgagctttaccttgaatcgattatcggcgacggcgttgtgcgggttttgtgatggccgcggtcagcaagcgaaccaactgcgcgctgtcgtctttgcggcccaaaaccaggatggatgagccttgcaagcaggcatcgatggcaggccacgaaatgtccttcgcgccttcgatatcaaaagaatcatccaccgcgccgtcgacctcaaaacctcccgtcagcaagcctcgtgaattgcccgaggtttgcccgaccgcgacgatccgtccgtcgtcgatatcattcagcgcgaagcctgccttccaactcctgagatcgagtgtctgtattgcgggggtgatcacaggattctcgaacgctgtatccatctgaccggcgtcggtgataccgctgatcacaccatgctggagcttcataccttgcgttga

SEQ ID NO: 94 - DNA, 446 bp, Pseudomonas sp.
  misc_feature 1..446: note = Marker nucleic acid sequence
  source 1..446: mol_type = genomic DNA
cttgacccggccggcactggcctatcgcctgaagaaaagcggcttgttgcatgacgagagtcttgagtgactttgcgtggccgcctggcggttcaccgtggaccacgcttgagctggattgatcaaatcaacaaaacctcgccgagacttcatcaaatgatcaaacaagcccttcgataaactccgagcccgatactcgcgacatcacattaagttatatgtcattgataaatatcgatttatataagttttataaaattggcatagcccttgctccagtaccaattgtcgcttttcgacgcgtagcaatttgcaacatgggttggatgaccgcgaatcgcaaaatcgtactcataaatggagagttcatgaatactcgaagcatcaaattgatcactgcagcaatggcgctcgcctcatggttagtaacaatcactccagcgtcg

SEQ ID NO: 95 - DNA, 471 bp, Pseudomonas sp.
  misc_feature 1..471: note = Marker nucleic acid sequence
  source 1..471: mol_type = genomic DNA
tgctaaataaatccgttatgcaagagctgtcgcgcagggctgacgcgatagctccacccatcggcgctattgtccaaaacacgaggtggagcatgaggatgtatgcagtttaaaagtccagtcagacgtgagtaaccggttcgcaaggttcgctattccctgaaggccctggaaacgggctttatatctgtgaggcctctacctatgacatcgcgccgaaaacttctccaggccgcctccaccttagcgttagggggtgtctttggacgcagcgctttttccgaaacgctaagtagggaagggcccaatatgaccgattcaattccggacatcattttccacaatggcgagatcactacactggatcgcgccaacccagtcgcccacgccgttgcaatcaaagacggcaagtttctggctgtagggtcagaccaggaagtcatggcgctggctggctcagccacaaaagtt

SEQ ID NO: 96 - DNA, 441 bp, Pseudomonas sp.
  misc_feature 1..441: note = Marker nucleic acid sequence
  source 1..441: mol_type = genomic DNA
ttttttttgcctgcgatttggcatttggcaatccgtcgctccaccacctccgagcgaggcgccgttttttcgactactaatgactggccgattttcgactctttatagaggagcgcgtcgatgctgagtcagtggattcttgcggcgattcacctgtttgcgtttgccttggccttttgggcagtgctggcgcgtggcagagcgtccagcttattggcgtcgggtacgggagcggccaagcgcgttctgctcgccgataacctgtgggggctttcggcgttgacgctgctggtcaccggagcgatgcgtgcgtttggcgggtacgagaaaaggcgaaattctccgcgctctatcggaaacgtccgacagccagctccagaagtgaaaggtaatatcggcgcaagaaaagagggagaggcaagtgaaaggagtcagcatgct

SEQ ID NO: 97 - DNA, 463 bp, Erwinia sp.
  misc_feature 1..463: note = Marker nucleic acid sequence
  source 1..463: mol_type = genomic DNA
gcagctccggatgacctgctggcagtagtggacggcgcgctcaatgatgaaagtgtgcgcccggtagccgaccgggtgatggttcagggcgcaacgattttcaactatcgcgtggaggccaggctgcatctgtttgacggcgtggtggccggtccatgtctggaagcggcgaacggtgcgttggctgcctatctcgctgaacagcgaaagctggggcgcagtgttcgacgagactcttatggggcagtgctacgtgtggcgggcgttgattgggtggagatgctccagccggccagcgacatcattatggacaggacgcaggcgggctactgcacaggcacgcaggtcatggtggccgatgatgacagaggattcactccatgagcatgaatgacagtctgttgccacccggttcatctgcacttgagtgccggctggccacagcttgcagcgacctatccac

SEQ ID NO: 98 - DNA, 460 bp, Erwinia sp.
  misc_feature 1..460: note = Marker nucleic acid sequence
  source 1..460: mol_type = genomic DNA
aacggtaatcggcgcgtcgatatgaatttgcggcgcatggcttaccggctgaggacggatagcttcattccggtaagcctgtgccggcaggctcatcggatgcaatggtgcagcgtcggcaggtgatcctgcgctgcccatggtcagggcggccatggcagccagcgcggcggttttacggcgcgacgttacactgaccggcccgttaatcagctccggtccgttctcgcccaccacgccaaactggcctgacggaatgtagccaccgttatcatgcatccccgcaaaagccatccccgcgtaaggcccgtaaagctgcggctgcattacgcgcgattgcgcgctgcccggcgcaaggttcgtcggtagcgtcttcgccttttcgctgacgaggcccattttctccagcagccagccaacgcccgatttcaccgagtccagtggatgcagcaccttattg

SEQ ID NO: 99 - DNA, 467 bp, Erwinia sp.
  misc_feature 1..467: note = Marker nucleic acid sequence
  source 1..467: mol_type = genomic DNA
ttttccagtgaacgggcgtgccgatcccgcacggcgtttaccctcgcctgctgttcgccaagacgtttcagggattgctgctgcctgtctagcgccgcacgtgcttcatctgcctgaccttttagctcacgctgtgcctgactcagctttttggtatcaatgccggactgactcagcgcctcgcgctggcgctgcactgacaggcgtaacgcattgtatttctgctgcaaaccggcggcgctggcctttgccttgtccagctcccgtgcctgctgcgcggtgggcttactggtactggcaaactgcatcgccagccgggcggcctcctctttggctgccttcaggctgcgggaggtcatgcccagctgggtattggttttgcggaacccgtcaatgcgggcggcctgcccattcagctctttgaggcgctggcggctggcttgcaactctgaggccagcgacttcgt

SEQ ID NO: 100 - DNA, 457 bp, Erwinia sp.
  misc_feature 1..457: note = Marker nucleic acid sequence
  source 1..457: mol_type = genomic DNA
gctccttcagggtgcaaaaatatccgttcagggttgttctgaattcgcaccctgccgaaatttcctggccgagaaaggcctcagtgccctgcttggtatagcgacggctaaaaccgtgctggataatctctctgactctgaaaaggagtacgtgtttaacgttgcaagatcgggcaaggctgatctgatagagaaattgacgcctgaagagcgagatgcctaccattatatggtaggtcaggatcagaagggattgatcaccatatttccacaaccagacagagatttaacaattgggaaactcgaaaacccaaggtacttagatagccaggatactgtcctaaccacaccggatcaacgtgataaaaatggttccagccataccggtaataatgagggaatccctgatataggcggtaatacaacggtaacgccaataccagagggatcaaacaaa

SEQ ID NO: 101 - DNA, 445 bp, Erwinia sp.
  misc_feature 1..445: note = Marker nucleic acid sequence
  source 1..445: mol_type = genomic DNA
caaagcggcaacgggtcgtaattttggcgcactactcattctcggtacatcaaccgttatccctgtgtcagaacgcatccgtctttattcccgacaggaagatattgcggctgactttggtgaagacagccctgagaacgaggcagctctcatttacttttcacagtcgccaaagccaactcaggcttatgtggggcgatgggccaaagcgctggcaaccggcgaagccggaagcgtggaaacgctggcgcaggcaatcacggcagtattgcagttcacgaactggtacgggcttggcattgctgatgaagacgatttgacggaggcagaggtgctggcaacggcggctgccgttcaggcatccagcctcagccgggtattcgcatacacctcagcggattccggcatcatcgacccggcatcggtcaataacattggccgacag

SEQ ID NO: 102 - DNA, 493 bp, Paraburkholderia sp.
  misc_feature 1..493: note = Marker nucleic acid sequence
  source 1..493: mol_type = genomic DNA
cgatgttgcctcatgtggtggcttacggacgtgtgttcgcaccaaatgaaagcgttccgtgacctcgcgtaaatgcgttctgggtaggggcagaatcccgtcaaacccttgccggacgtggcgcggaacgcttctactgtgcgctgtgtaatcggcaaaaaatcagggccttcgacccccggttttgagaacaatcgcggggctgtagcgcacacggaacgcttatgcttccaggtataggcgtgattcaactcctgcggcggatttgcccgaaaatagccgggacgcgaaccggtagactggaacctccacaactttccgagaatcttgcgcatacagctctttcggcaagctggtgtcccacttccgttgcaacagcctagcggctatcgtcagcgccgcgactgctgagatgcgttattttcggttacgtggctcttccgggccgccgagccttccttggcaagcggtaaccagaattaatacccaaggg

SEQ ID NO: 103 - DNA, 499 bp, Paraburkholderia sp.
  misc_feature 1..499: note = Marker nucleic acid sequence
  source 1..499: mol_type = genomic DNA
tcacaaggcatcattggtatccgtggcgcacccagaaacgcaccaacgggtgtcccaaccatgaccgcctttcgtctcaatagcgtcatgaccgtctctatccgtatcgctggccaagaccgcgtacggcaacaacaccgctttgccaataaaacgcaagcgcgctaaatattcgcgtcgatacaacacgcattgattgtagggaataacccgtagtaggattcgcgactcaattaataatgattcgcatttcgacaagggttcttcgatgcgcttccgccagatccatgccgcacttctgattgccttctttgcggcgcccacgctcgtcttcgcgcaagccgccgcgccggatgcagcgagtcgcaccacccagaacgcaccgaaagccggaaccggcacatccgccaacacgcccgcgagtacgggcagtacgcagaacacggcagacccggccgaattgcccgtcgtgaagatcaccgcgagcggcgtgtctggg

SEQ ID NO: 104 - DNA, 492 bp, Paraburkholderia sp.
  misc_feature 1..492: note = Marker nucleic acid sequence
  source 1..492: mol_type = genomic DNA
tgcactcttcgcgccggcgcaaggggcacacgtgttcacgctcgcaggggagatcgccgcggtcgataccgtgatcgagctgctgtccgcgttggcgcccggcgcccgcctcgatagtgccgggccgccattgcccatcgccaccgaattcccgagcgatccggcgctcggccgtctgcttccaggtttgcccgctacgtcgctggaagacgggttgcgacagacgttcgctttctaccgctcgcggcgatagattgggctccgcttgttcttgcgctgatcggttggttcatttggggctcgtgttaatcagcgcggtggctttgcggagcgaggcatcgtatattttgattcctgaggatcgctggcgcattgaattgcgcgaagacggtcgtgcaacgaagaacttcgcatgagccccgtagtcaaggatggatgcaacctaacgcatggagcgtcgaaggcaatcagatggaacgtttcgattacgca

SEQ ID NO: 105 - DNA, 500 bp, Paraburkholderia sp.
  misc_feature 1..500: note = Marker nucleic acid sequence
  source 1..500: mol_type = genomic DNA
gatacgaagtgaccaacagctgatcaactggcgatttgtgcagggcgagctgaccaagcttcaatcgtggacgacgcatacgggtgacggggcgcacgccgggcgcacgcgcgccccatgtccatcgcgcccggccatcgtgtgtacctgccgcaagcagcatagttcgattcatggtgtgaatttcctggggagggagccgcgtcgcgcggcgggattactgccggggaggttatttgttggaggtggccgcgtggtcgcgatgacaccgtcgaccggcgtcttgccgacgaatgcgaagccgcgccaaaccacgaggatgccggcggccgcgagatatttcttcgtatctgactgcatgaatgctcctattgctggcggtgaatcacttcggtgccggagaattgataaccttccttgccgcacttttgcgcgatccagatagggaagggcagcgtgtgcaggccttcgtcttttccgatgtggtgcgccttgcaaag

SEQ ID NO: 106 - DNA, 494 bp, Paraburkholderia sp.
  misc_feature 1..494: note = Marker nucleic acid sequence
  source 1..494: mol_type = genomic DNA
ggaaggcggtctgctgtccggtcacgtgcacgcggccaacgggactctgtttccgcagccccgtgtcgcacatggcgactcgcatacgctgttcgacgtcgtggtgggggaaggctggcgcgtggtaacacttggcggcgcgccggcaacgcaacaggtgcacgcggcggctgaaaggctcggtgcacgtttgatcgagttggcgcccgatggtgacgtgcatcatgccgtgatcgaaaacgggcgtcccgcgttgatcgaactcgatggcgtactggcgggttggttcgatcggcagggctgctgtgcggcgatcgtgcgccccgatcattacgtgtatggcgtggcaggtagcgcgagcgcactcgaagccgaactcgcgcaactggaagcaacccttcgcggataagcatccggatggccgcttcgtgcggccatccgaccgggaagaacgaaggccaagtcgcagacagaagcgacgcctgaaaaaatta

SEQ ID NO: 107 - DNA, 434 bp, Pseudomonas sp.
  misc_feature 1..434: note = Marker nucleic acid sequence
  source 1..434: mol_type = genomic DNA
gccctggccggaagtcacttggaaacggccgttggtgaacgatgcagtaccaccagtacctgcagcggttgtcagactagtaacgacgctcgcaatggtggcgtttgcagcccaagtcacgttattgccgtttacagaaacggagccggcagcagccagtgtggtaggggtagcggcagcggtggtaccagcggtcaagccgagagcggttgggccggtagcaggagtagcgccaatggtaatcgagctgctggaagacagagttacgataccagtagcatcagcactagcagtaacgccggtagtagctgtctgcgcgttgatcgctgtcacggaggcgttagcagcagctgtaccggcagccacaacaccagaggccagggtaatcgaggtaccgttaatggtgatggcatcaccagctgcaagggcagtag

SEQ ID NO: 108 - DNA, 463 bp, Pseudomonas sp.
  misc_feature 1..463: note = Marker nucleic acid sequence
  source 1..463: mol_type = genomic DNA
agcacgctctgcctcggcgcgctcatcagcttcgcgtcgggctttctcggcggccgcctgcgcgatggcggcgtcgcgctcttgctgttcacgaactaatttctcggcgttgaacttttcaatttctgcaagttcggcttcgtgcttagtacgatcggcgtgcatggcgcgcaacagcgagaggctgcggtctttcgcctgggcggcttctgccaggaactcttcccaagagtcgcctagctcaatcgcttccagttgggcaatggtttgggccagggcggcagcggtcggcgtcgcgccaaatacctccagatccttgatcgcctggatgttgtcgacgtggcggtccttgcgggcctgctcggcgttttcccagtcagtcagcggctggcgaatctcgtcacgaagagcattcgccccatcgacgaattgcttcaactcctgctcaattaccttcggcagt

SEQ ID NO: 109 - DNA, 498 bp, Pseudomonas sp.
  misc_feature 1..498: note = Marker nucleic acid sequence
  source 1..498: mol_type = genomic DNA
agacacagtggtgatcgtttgcatcaaccatgggtactgcggccagaagcccaacagcacaaccatcaggcacaaattaccgaggttgtaggccagggcagtgacggcgaagcgcaaccatcgctggctgtcggccggggccgcgtttattgcaaacgtccaccgtttattaccttggtagctcacccaggtccccaacaaagcaccgatcagcgtagaaaccaataccggcactaccagggacaataataagagtgttatgtaatgggttccggtggccagtaacccgaccaatagataacaaggcagacatgacagcgagcggccaataagaggtaattgcggcatatatgtcggcacgttagttgttcaacgaatacacccactgggcataggctgcgatactatcgagcagccgatcagcccatgtgaaaaaatcgtcaaccacgtcaaacattactaaagtgtaataacactgcaagccatgtgttaatgaca

SEQ ID NO: 110 - DNA, 487 bp, Pseudomonas sp.
  misc_feature 1..487: note = Marker nucleic acid sequence
  source 1..487: mol_type = genomic DNA
cacagtcggaaaaggaaaaacgacgttttaagatcattcgagtcaaagggtataacgtacacgatgccgccatagaggtcgccgagaaccggacagctatcccgttcgaacctcacgcctgcagtcctccgagcaatatatcaccgtattataaccatcgcctagttttccagactggacgcttcccatctagttggctatgtgtagacggtaatgggacagcccggagtcccgccttcttggcccttgatactccttgataataagtccagaattaagtcttttcctgctcaggaaagggaaagaaaccctttgaatttcaataggtcggacaccagacgcacgtctcgtttcccgttccaagcattaagaaaaagccacttaatcgagtggctttttttttgcctgcgatttgtgaaatgggcgcttcggcgcctttttcgttccgccagaatccatcgaaagccatgggtgtccggacgtgttg

SEQ ID NO: 111 - DNA, 447 bp, Pseudomonas sp.
  misc_feature 1..447: note = Marker nucleic acid sequence
  source 1..447: mol_type = genomic DNA
gacaagaatgtcgtgcagtagggtttttcgcttttgcctttaatccttatgtgatggagcaacttccctatcagggattgttgttccatcagcaaatacataaaaacaactaaagaacaattaaacccacttagcgcacggaaaaatcccaccaatagccgggtaacttaccgcacacaaaaatatcggcaaaaacatataatacatttgtataccgattcaaacagttaatcagcttattatcttcacccagcaagccacgccttcccaaaccgctgcggtcgcctatttaaaagatagcgccgtgcgcgtggtcgcggtccagttactcttatacctacaactataatattccaatactgcttttatagcacttgcaacaactataggcgtcaaccatgcaccaacatttacttgagcaaaaaaaacaaaaacttttcggtcacc

SEQ ID NO: 112 - DNA, 497 bp, Pseudomonas sp.
  misc_feature 1..497: note = Marker nucleic acid sequence
  source 1..497: mol_type = genomic DNA
tctgcagtaatgaaagggcggcaatgatgtcgccctttttttgtgctcggggcgtttccgagacggacagaatcagtcacgtatcataatggcacgtcgtctcccgtgactttcattcgatggaaacctggcgaggtgggcgtctaccctcgcctgaagattacggatatgaatagtgataactgcgcttcttttttgttgataagcatttgtcatttcgattgcgtgagcaggaacgattccattcatgcggccccgtgctgcggatttgaggctatctattgaggcttctccaagttccggtttgaaaaggcggacaggtgatttggccatcgaatagacttcttgtttcatggcccgtgatgtcttagcaagcgaggccatgtccgatccgggtaaatagctgaagatttcatcatagacaacttgtactcccttgatcttttcaaacgctccaaggggtgttctatagcgttgagctgtccttagcccgataa

SEQ ID NO: 113 - DNA, 497 bp, Pseudomonas sp.
  misc_feature 1..497: note = Marker nucleic acid sequence
  source 1..497: mol_type = genomic DNA
cctggccgtggcgatcgagagcggaatcgccgaaggctccctggagtccgttgccgagcctcatgcggtcgcgcaaagtctctatcagctgtgggtcggtgccagtgtcatggtcaagatcaccaagagtgtccagcctttcgagacggcgatagcgacgacccgtcagattctcagccttacctgatcgataccgctgcgtccttcatcaagatctgcctatccctactcatctgaagcgtgccctgcgcagcttcagcctgtctgcaccctcctccaaaaaaaccgtgatgcgaaaaaacaaaaattttactagacgactggtctaatttgaaattaaggtagccacacgttctacgcatcgcaaagcagcagctcgcgaaagccacccactcagaggtttgggcgatgccttttgcagcttgatttttttgctcagacgctagacgactggtctattcaaactaatgcagcacactctcaaacaggacaaccga

SEQ ID NO: 114 - DNA, 497 bp, Pseudomonas sp.
  misc_feature 1..497: note = Marker nucleic acid sequence
  source 1..497: mol_type = genomic DNA
gttggcaagcgcagaacttgagcgttgctgcaccggtctggtcggtgcgggggaagcacttgccggcgccctggtgcggggtcgacatgcccaggatgaagtgattgaaacgttcgccgcgttgattcgcggcgtgttgagtccgcctgaataagtgttcatgttccagccataagcaattgcctacagatactcagctatgtcactcgacggtgacaaaattcttggatccaattcctgcaatcgccttgacaggctaatggagccgatgaaatatttccctccgctacggttcagcttcaatcatcatttggcgcggatgccataacaataatcaaatggagttcatgatggttttcctcagtacagttccatcggttatcccatcaccctccgtcgattcctcgctccccaactaattgctctatttggcgccttggcgctgtagggactgttgtgcaatgcccatcgtcgtcggcagaggatagccatgaaaa

SEQ ID NO: 115 - DNA, 499 bp, Pseudomonas sp.
  misc_feature 1..499: note = Marker nucleic acid sequence
  source 1..499: mol_type = genomic DNA
tctggtgtttgagccggtgggtggattcgacggcctgtttgcccaactcgatttcctgggcagtgacctgttccggcgtttttatggccaggagcacctgggtgtctggcaacccgaagggcggctggaggcctgccggcaagtggggcacatccgtatcgatgatctgatcaccgagcggctggaggaaagcaactgggcgttgttcagcgaattcctcggcgtcagctccgatgagctggttgcgccatcgctcgagcatgaatacctgagtccgtacctctcggcccacctatatggcttgcaggcctgtcatcagcaggaacgcggctatgcggctggctacaccgattacgtgcaacgcatgatcatggtcatgcaccgcaagcgtatgccggagcccgtctgccagcaggtccaggggctgttgggttcaccgtcggagattcccgagcgtcgagccgtgatcgccctggaaacggaaaaaaatctgaatctg

SEQ ID NO: 116 - DNA, 494 bp, Pseudomonas sp.
  misc_feature 1..494: note = Marker nucleic acid sequence
  source 1..494: mol_type = genomic DNA
atgacatggtggtttcatgcgggttcaaggtaagaaagccccgtgctagcggggcctgtcaggttagacgaatttgattagcagcgtggtgacggtggccaccgtaccgatcaggccggtggcaaccgcgaccgggtaccagaacgtttcgcgagtcatcttgcccgcttcggcgttgagctttttggtctcagccatcaatttggcaatttcgacatggatcttttccaattctgcgccgctcataccgaattcccgcatgtgtgcgtcctttcgggtcatggggcgcgctttgtgcgctgccctgagatccatatcgtgcctttaaggtacggctgcgagttttttcctgcccaagtatagccatttgaattcatctcggttcgccgatcagcatgtacttgggtttcaaggtatgccgagcgcatcgcaatcggttttttcttggcggcgccaagcgtggtcaacaggtcgccaaaacaattttcatgtaa

SEQ ID NO: 117 - DNA, 494 bp, Flavobacterium sp.
  misc_feature 1..494: note = Marker nucleic acid sequence
  source 1..494: mol_type = genomic DNA
caaaaaaattacctcaaaaaatgaaatttaaattacacataaatcagactcttgctcaattactggctcaggaagatactgatggcgacaaaaaaataacgattgacgacaaaggcccaaaaagctttctgctcaaagatgaaaaaggtaattctattgcgattgaaggaacgtatcaactttctaatttgctgcaggagcttgcattatctaaaaaaggagataatgagtttgccgaaatcgacttagccgaaatcacagaagatcccgttaagagaatttccagaaaaataaaagatttgtattggaaaggccttacacgaacgattgacgcagccggagtaaaaaaaatagtagaagacgacaagatagaaaatgcagtttcgtatctgtatgttcctgcgggcgatgcttttgcttttgagtatttcaaaaatttagaacattcaaatcccaggttaaaagtcgttcatttgcccgaagatatttcaccg

SEQ ID NO: 118 - DNA, 491 bp, Flavobacterium sp.
  misc_feature 1..491: note = Marker nucleic acid sequence
  source 1..491: mol_type = genomic DNA
tttttttcatgaaagaatatttgtttacataaagataattaatcgtgattaaattgatgtttttgaaatgagaaaaagctttttttaatcattataaaaatctgattcttaatttaaaaataacctatttcttttcttaaaataattctttggacatttttactcctattatggattctgaattactatttgatttgtacttttataaaatactatcaaagcttaattaatgaaaattaaaatcttaatattttgaaaaagcatcttttattaatcacaattctggctggaaatttagccatgcattctcagaacaaaatcgttacaattacaaactctctttctgtagatcgggaatttgaaacagttgaacttaccaaaaaagacctcggtttgacctcttctgcaaaattggaaaattatgcagtgaaggaaattaattctggtttagcattagaaagccaaactgttgataatgatggagacggcgt

SEQ ID NO: 119 - DNA, 491 bp, Flavobacterium sp.
  misc_feature 1..491: note = Marker nucleic acid sequence
  source 1..491: mol_type = genomic DNA
attaactcctattgcctggaaaaaaattacagccaaagaatatccttcaaaaccaataaaaaaagaagatcaaaaattgctcaaaaagactgttcccggcaatacttatgcgtttaagacaagcaattaccaatattttctgcaggattatgtagacaatcgcaaaaacctatatgccagacgcctcttagttctcgactctaatacaaaagacattataatcgaaaaactctatagccagagcgaaggcacctcaccttctcctctaaactacgaagaaggcgaagacattgtgaaccaatggactggtaaactttttaaagataaatctccggtcgttttcggttttctatatgaatcattcggatgtcctggaatttcaattatcgacaaatcaaacgaagaaatttatcttcaatgcgacaaccgtcattaattatattaagaaaataagaagcagaaaatcctcgtttcaaaagacctttagtccc

SEQ ID NO: 120 - DNA, 487 bp, Flavobacterium sp.
  misc_feature 1..487: note = Marker nucleic acid sequence
  source 1..487: mol_type = genomic DNA
tcatgggaaataccgtatttttttgatgattctgtaaagacttcaaattacagcggctactcattcgtttttaaaagtgaccaaactgtagttgccagtaatggatcagttacagaaacagggcagtgggaaagtactgttctgtatggtgttagaaaattgaaactgaatttttcaacagaattgcttggaaaattaaattttaactgggagttattcgagtttaataattctcagatacgattaagagatgtgggtactacgactaattatctttactttcaaaaaaaataaattcttccttgcacatactaattttgttagcacgaattttatactcaaacaggtgcaaaaaaaatggtttggtcaaattttgtaatgcacaatcttgttatacttttgaaaagggaagccatgtgatatttttaaataaagaaagtctctttgtggtataattaatatttataaaaatttattttccgtttaa

SEQ ID NO: 121 - DNA, 456 bp, Flavobacterium sp.
  misc_feature 1..456: note = Marker nucleic acid sequence
  source 1..456: mol_type = genomic DNA
caatttcctttagcaggtcattggcataatacccatggtctgatacggctgttacttttgcgaatcttgatttattgaaatgattgatagttgtgggtgaggtttcaaaagacaatgtcgccacctggttcagggcaataggcattccctgaatattatttacatacaaatcctttaaggcgtctaaattagagaacttatcccttggcagggtaagagtcacatttctggcatctccgcggtcgtctatgtaattccccatagtcaggccggctacggcaaggcgtacaaccctgtcaatatcgctggttaaaaccccaagtgtgcgtgctttttccttgttaatttttactttaacatcggttttataggtgttaagttcgttattgacgtaaatggttcctttctgtgcgcgcagaatattttctgcttcaaaagaaagttttcgaagcactg

SEQ ID NO: 122 - DNA, 489 bp, Acidovorax sp.
  misc_feature 1..489: note = Marker nucleic acid sequence
  source 1..489: mol_type = genomic DNA
cgatggcggggtgacgccttgcacagcagcggcttgcactgcactgaggccctgcagtgtcatctgctggaccatctccaggcgacgggcacttggtcaagtccagtccgatgacaggcaggtttagagtcgattgcatggcggcctccaggctcagtggttgcgagggttgccactctggcactttgcaactgaactggcgacacccctgtctacgggagggttaccgcggcgcagcgccaaaggtggctggaccatgccatctccgggttttagaaaaatgattcccagaacaagatccgtgttatgcccttcactttgtggcgcggtcagctggacatcatcaaacgctgcacggtccagtacagcgacagcaccagcaacgcgacggagcccccacgcaccaccaccgagcggtaccacgccctgcgcgcaagcactatcgagaccgcgcaccacagggcgaccaccatcagttggcccacttca

SEQ ID NO: 123 - DNA, 494 bp, Acidovorax sp.
  misc_feature 1..494: note = Marker nucleic acid sequence
  source 1..494: mol_type = genomic DNA
tgcgctgcacaggaagacctcccccgggcggccggatacaacgcacagctggttgtagtgcatggaggcgtagtcggtctcgttcgcggagggcagggcgaaggactggcgcgtggcaccttcgaggcgcaccagctctggtgcatagcccaagagcttcctgtcggggctcaagatggcccggttgcacagcacccaggagattggggagcttcctccttcgaacgccatatctgtcacatccatgtaccaggggcgctgatccagcgggggatagttggcggcagtatggacgagctgtggatcgcctaccaccacctgcacttgccccgtggcggatatcgtgccgatcagggaagttcctgaaccgggaggtagccaatccagggtgatgggcagcgtccgtgtcgcaaaccatagcaggcctgtggtgtcggcgcgcagaacgcacatgcctgagaaccccgggtttgcgccaaagtattcgctcctta

SEQ ID NO: 124 - DNA, 494 bp, Acidovorax sp.
  misc_feature 1..494: note = Marker nucleic acid sequence
  source 1..494: mol_type = genomic DNA
acaatggaattcactggtggaggcaactcagacggccggctctgtcgccgcccttggcgagcgccttggcctggatcttagtcaggaaggcaatcgctttcgggcgcgggaggctatcgctgaactgctgcatccctggttcagttcgcaccccttctcgaccatcgccgaggtcttcgacaggtacggggtgtgctggagccgctatcaggggatcgacgaactggcgaaggaccctgcctgctcccctgacaacccattgttcacgcgcacagatcagccgggcgtgggtgagatgctgctggcgggtatccccctgcagttcggtgcggtgccccgtagtcctgcgcggcctgctcctcaacttgggcagcataccgaggaagtgctgtccgagctgctgggcatgggggctgcgcagtatggtcagctgcacgacaagggcgttgtcctgtccggcaagggttgagcgcaattgcatcagtcccgctgca

SEQ ID NO: 125 - DNA, 490 bp, Acidovorax sp.
  misc_feature 1..490: note = Marker nucleic acid sequence
  source 1..490: mol_type = genomic DNA
tcagccagatgaatcactcggctgtgggtaaccaccttggttcgctggttcgcatcccccggctcgggcgtgcggtggtacccgcacaccacgcccagggcggttacaggaccaacgccgtttgtgcggttggctgggaccacttcgaggaagagtcggggcgcggtgtgcatgtactatctggagtgaattggttacaacgtaagacgcattgtgcacggaattctgtgcatgtcaataaatgaatacagaaatccgtgcatcaatgggtacaaggcttcggctagaacgtgagcgcttgaagttgcaccagcctgatatggcagctcttggcgatgtgaaaccacgcacctatcaggactgggagcgcggtgttgccgctgtaagtgccgagttcttggcagttgttgcggcccacggtgtagacgttggctacatcgtcacaggtcagcgtcggggcgggtccgatggcggactatccgaagcggag

SEQ ID NO: 126 - DNA, 497 bp, Acidovorax sp.
  misc_feature 1..497: note = Marker nucleic acid sequence
  source 1..497: mol_type = genomic DNA
gccatccgccgcatcgcaccggctggaccctgcgcgccgcaggcgccgctgacgcgcccgcgctggccgacctgtgcgccgcccacgcggcgtacgagcgcatcccgtacagcgccgacggccatgcccaccggctggcccaggggctggaggcggggcggttgttcgcctggctgggctattggggtgagcaggcagtgggatatgccagcgccacgctggactattcgactctcgccgcgcgctcttacctgcatctggactgcctgtacctggagcctgaagcgcgtggctgcggccggggcgcagagatgatggccgctgtgcagcaccgcgcccaaatgctgggctgcgaggcgatgcagtggcagacgcccgtgtggaacgagggcgccatccgtttctatgaccgcctgggggcaacgcgacttgccaagcaacgctacacgctcgtgtgtgggtgtgaaagcccctgggccaccggcagccccaggggg

SEQ ID NO: 127 - DNA, 495 bp, Bacillus sp.
  misc_feature 1..495: note = Marker nucleic acid sequence
  source 1..495: mol_type = genomic DNA
ttttttgagagtcctttttgaatagtgcgatttttccctctggagtccgctgatcaatcataaaaggatagccattgattgactatccttttgtacatatcttattaaccttttatatggggcataaaacctttttcgatcaattcatcgacggccgtgcataccgcgatcttcacatgggagtaagttagtcctccctgtacatacgcaacgtatggaggcctcaatggcccgtctgccgataattcgatgctcgcaccctgtatgaacgtgcctgcagccatgatgacatcgtcaacataacccggcatatagttcggatatggggtgaaatgagagttcacaggggatgcaaattgaatcgcctgacagaaggcgaccatccgatccctgtccccgaattggacagattgaatcagatcggtccgtggaccctcgggtgccggattcgtatccatcccgagctctgtcaggaatgcgctggtgaagacggcc

SEQ ID NO: 128 - DNA, 497 bp, Bacillus sp.
  misc_feature 1..497: note = Marker nucleic acid sequence
  source 1..497: mol_type = genomic DNA
gaggcaggtgtaggcagtgaaacattctaaagaagttgccgtgatcggcgcggggagctggggttctgccctggccatggtcctcgccgataacgacgtaccggtccgcctatggggacataaacaagaacagatcgacgaaatcaatcgtcatcatacgaacgggaaatatctgaaagatattaaactacctgaaacgatccgcggctatcacgatttggcagaagcccttcaaggggtggacacgatcatccttgcggtcccgacaaaagcgatccgcggggtactcggacggatccaggaagaacaggctggcccgttgacggttgttcatgtgagtaaagggatcgaaccggattcacttttgacgatctctgaaatcatcgaagaagaaatggatgaagtgaacagggaggccatcgttgtcctttcgggaccgagtcatgccgaagaagtaagcttgcgccatccgacgacggtcacggtctcctcgaaga

SEQ ID NO: 129 - DNA, 490 bp, Bacillus sp.
  misc_feature 1..490: note = Marker nucleic acid sequence
  source 1..490: mol_type = genomic DNA
gagggaaatcgtgaaggaagtgtacgacttcttccagctcaatgaggatttctcaaatcttccgagaaaatataagctgtccatctcttcgaatatcaacaatgcatccaatgctgaaattaactgtgcatctttcgttccggccaccaaggtcattgatggaaagaaggtggcaggattccacctgaaggttgggggcggactgtctgccagaccattccttgccgaaacgttggatgtattcatcgaacctcatcaggtaaaggacgtaacgattgctgtaaccacgatcttcagggattttggatacagggagaagaggcatctcgcccgtttgaagttcctcgttgccgactggggacctgaaaagttcaaggaaaaactactggagtatgtcgagctacctgatggcggagaggatgccgttacgggatggaacgcaggctacttttacggagtaaagcctcaaaagcaagaggggctgaactat

SEQ ID NO: 130 - DNA, 497 bp, Bacillus sp.
  misc_feature 1..497: note = Marker nucleic acid sequence
  source 1..497: mol_type = genomic DNA
ggaccgatgcattcacgaggctaccttctgcctcggacttgatggatagggtcgcattatccgttacacgaccgataagggtcgtttcagatactagtcgttcaaaagcttcctggtgttcaggtttgacagtgatgaggaagcgggattgagtttcactgaacagatcagctacaggatttgatcctgagagcgtcacttccgctccaagaccatcggtaccgaaagccgattcagcaagggcgacagacagaccgccttctgcaagatcatgtgcagaggcgacaaggccttcctggatggcttcgaggagttgcatctgacggcgaagctccactttcaggtcgattgccggtgcatggccgaagatcttcccttccgtcattttctgaagctcgctaccgccgaactcttcgagggtttcacccagcagatagatgaggtctccttctgctttgaagctttgggtggtgatgtggtcgatgtcttcgatcaat

SEQ ID NO: 131 - DNA, 486 bp, Bacillus sp.
  misc_feature 1..486: note = Marker nucleic acid sequence
  source 1..486: mol_type = genomic DNA
tctacctcctggaaaggtacaggtttttgccaatgccttccttgggtacgtaaaggatgtaggaatatgcctagatgaataaaggagtttcaactatccctatggaaatggttagagaatgcgatgtttcaatgctgattgggacttaggtcactatcttttcgaccgaaacgtgttgaacattgttggatgtgtacttagtatagaagtatagcgtttccaactctaatcgatgtccatgattatcgtggaacaaaagaggggtgtaccgtgtcactgaaaaaaatcgacaccaagatcctggatggaatccttgagaagatgatcgacacggtcgatgagagcaagggtgaaatctttcagatcggtgagcaatgccggaatgattaccaagacttaatgcaagaactattagatgttaagaataaggtccttcaggtcatcgacgagggggatgagctccacaagaggtcaaggctcgcacgc

SEQ ID NO: 132 - DNA, 304 bp, Enterobacter sp.
  misc_feature 1..304: note = Marker nucleic acid sequence
  source 1..304: mol_type = genomic DNA
gcgttgtcctggaggagaaaggaaataaatctgataattcatgacgatatattttgacttaacgcaaactgcttctaaactttcagaacaataacagcaagtatgcttacggcaggggttgatgtcaccctgccgtttttttctgaagtgcaggtaccggatttaacggctctccggtgccgcaccaattctgcgcagtgcctcctgcacttcatgcagcccaaaaacatcatctgcaggcggattctttcccgacaagctgcatgccgtcagggtcgagttgtatgctgaaacccgctggcga

SEQ ID NO: 133 - DNA, 233 bp, Enterobacter sp.
  misc_feature 1..233: note = Marker nucleic acid sequence
  source 1..233: mol_type = genomic DNA
tgcaggaattcgcgatatcgaacaacagcgcccaaccaaataaaaagcggggacgaatccccgcttgtgtttatcctactttacggtagggaaatgaatgcttaatgcgtgcagcaaaatactgaccttttgacccggcgttaatcaaagcctgatgcactgccgaaggtacgcctgagtattgatagactccaccattatgaaaggcgatttcaagcacgctggaggatgga

SEQ ID NO: 134 - DNA, 308 bp, Enterobacter sp.
  misc_feature 1..308: note = Marker nucleic acid sequence
  source 1..308: mol_type = genomic DNA
gagcgacacctgctataaaatcatctccagcgccagcactgcacgctaacctttataccccggttcagttgggcaaataggggagtagcagagatgcggatttggtggataaacataaacaagaataatgtcacctttatggatatataatatttttatcaagctcagtgatgccgagttcacggattatcatcgactgaaagacaatgtgatctaaccctcggtattgtttttttacagcagttcagctcaggtataccattgtctgacatgcattttagtgttattccataaagacacacagctaa

SEQ ID NO: 135 - DNA, 265 bp, Enterobacter sp.
  misc_feature 1..265: note = Marker nucleic acid sequence
  source 1..265: mol_type = genomic DNA
taatcatgtcccgttaatattttagaggggatactgtcgatttaattagtatatgcactagaatgatggttggtcaatggcttgatttctagtttttacatgttttatgttttgtactgtgcgattactacgttgagtactgtgattttttctagatcgactaactaaggctgcattaagacaggctagcgtaacgcatccctttcaggttcgctccgggcaaaagtagcctatacggtctcaattgacatacttaaggatcggc

SEQ ID NO: 136 - DNA, 496 bp, Variovorax sp.
  misc_feature 1..496: note = Marker nucleic acid sequence
  source 1..496: mol_type = genomic DNA
ggacgtgacgggaggcgtggtgggtgttccggcacccggcaggccgccgaagaagccgccaccgtcgttgccgccaccgcaggcggaaagcgtgcaagccaggatcaatgcggacacgagccgcataggcaatgaatgaagaagcatggagggttcctctctgtgtgattcgtggatatcgatcgggtgttcagggatgcgctgcgggaagccgccgtcggttgccacatgcaagagccagcgcgaaaagcgcgaggcgtgcaggtgtgatgtggtcgggcgcatcggttcagccggtggtctgttgtcgttgggtcgtgaataccggcgcgacaaaaaaaaggcgccatgaaggcaccgcgcaccggacagaccgcaagactatggagaacgcgttacgtcgccgtgaacgggcgatgacagagcgaaggcgctcgcgtgacgaagtgtttcccgagcgccccgcacgggcactcaggctattcgctcagacctt

SEQ ID NO: 137 - DNA, 496 bp, Variovorax sp.
  misc_feature 1..496: note = Marker nucleic acid sequence
  source 1..496: mol_type = genomic DNA
cgcaaatattgcagccgacctgggtgctgtactgaatgcattgacgacgccacacgtcgaatttggttgctggttcagatgccatcagcactggcaccggcaagctacgatcagaacggcagccgcaccaagcacacatgaaggggcaaccgcgtgcagacggtagacgggcaaagccagatcgccggctacgaaccacgaccggcagcgaagctccggcggtatcgaaagccgatgctctgacgatccatcaggctcggcaggtcaaccgccccgtacgctcggtgcatcggacttccataccatcccaaccccgacatgcacgccatcctcatccacggcctcggccgaacacccgtctcgatgctgctgctcgccaggcgcctgcgcgccaagggaatcacgacccatctgttcggctattccgccgccttcgaaggctgggatgcgtgcgtcggccggcttcgcggattcatcgatgcacgcacgcatggcg

SEQ ID NO: 138 - DNA, 481 bp, Variovorax sp.
  misc_feature 1..481: note = Marker nucleic acid sequence
  source 1..481: mol_type = genomic DNA
gggtagcgcagtgcgtgaagggcacgcacgcgatgctcacgcaacttctgcaccacgagcatgcgaacctgtcgctcgcgcagcgctgcagtgcgttgccgggcggcatgcccttgttctccgcgttgctgaattaccgccacggcgcatcgaccgttcccgatcagccggtgcgtgcatgggacggcatggaggtgctctccaacgaagagcgcaccaactatccgttcgtgatgtcggtcgacgacctggaggacggctttgccctggtggcgcagatcgtcggggccgtggatgcgcagcgcatctgccgtttcatggagatggccatcggtgggatcgtggcggcgttgcagaagcagcccgggcaaccgatccgcgaactggagttgctggacgggccggagcaagctcagttggaggcatggggcgagaacgcacgccccgtggactcacagagtccggtgcatcggctgttcga

SEQ ID NO: 139 - DNA, 476 bp, Variovorax sp.
  misc_feature 1..476: note = Marker nucleic acid sequence
  source 1..476: mol_type = genomic DNA
cccaccagggtctcgggcttcacgcccagggcgatcaatcgatgcgccaagtggttcgcgcggcggttcagttcgtcgtagctcagaacctcgtcgccgaacagcagcgcggtggcgtgcggctgtctcttcgcatgtgcttcgatctggcggtgtaccggctgcgcatcgccatgagcctcccggttgtccccgcaattcgacagccataacctctcctcggagctcaggagatccaactcgcacgtcatgcgttcaggctgtctggggaggccgtcggcaatccccttgatcgctgcatgcagatactcgcagacacgttgcgcatccacggcgccgctgacatgcgcgaccagcgcaaagtcttctcccagatcgtccaccgacatgcccaccgggtagttggtctgctcttcgcctttgaggacttccatgccatcccacgcgagggcatcgttgccgttctcggccttggg

SEQ ID NO: 140 - DNA, 498 bp, Variovorax sp.
  misc_feature 1..498: note = Marker nucleic acid sequence
  source 1..498: mol_type = genomic DNA
agcatcttctgccagtgcatatggctgcatctggtccctgatcgcgcgcgtgggtaaccgggccccggctctgaagctcgacgacgacctgctgcgctgcaggacacgttgacggctgtgcgcatcggccgcccggttcagagctgcggttatgagctccatgcgaacggctcagtacctgcgcggccgtgcattgctcgccgagttgttttggtccgaatggatgggcgaggccatcgaattggcctacgtgagggcatcatcccgatgcttttctcgccgcttccctcaacagccatcgcccggatgcggtctggaaaactgcgggtgtgggcacgcggccgaagcggatgctgaatgaggcgcgcatccttcacggcctgctggtctaaggcaggaaaacaaagccgctcgttggcttcgcatgtcacaaagcccggcttgccaggctttttgcttttcggccgagaggctcgccagtgatggaccccgacggct

SEQ ID NO: 141 - DNA, 494 bp, Acidovorax sp.
  misc_feature 1..494: note = Marker nucleic acid sequence
  source 1..494: mol_type = genomic DNA
ctggaaatcaggtgctgcgaactgccgccggtccagcacgccgccgatctccagtgccgcacggcggcctgtggctttgaacccctgctcaaggttcaggtgcacgcggaaatcatcctcggtgtggctgatagcgttgagcggaaagcgggcggcctcggggaagtaccgggtcagttcactggcgagggttgaggcgaaaagctcatccggaccgtagctgcgccacccttggggtgtggccaccagcagtgccgtcccactcccccatttagaccattcggcaacccagaacgtcgcaaagcagctcgccggttcacccgggacctggactccgtcccggtccacctggtgcagtgcaaggccgtaattggcgccgatcaatgccacgttgcgccgcgccgttgcggccattccgttccccatgcccagagcctatcccagcaccgcttaccccggtgagccgcccggcctaagattgcaccgtgccattg

SEQ ID NO: 142 - DNA, 499 bp, Acidovorax sp.
  misc_feature 1..499: note = Marker nucleic acid sequence
  source 1..499: mol_type = genomic DNA
atcagcccgtgcctggcccgcttttgcccaggaactgaccgcattgaccggcatcgacctggagctctcgcagcctggcggcctcatgatctgcctgaccgaggctgaactggccgagcgcgcggccaacctgcaggcgctgcgggattctctggacgagccctaccccttcgaggtgctcgatgccgggcagttgcgcgcgctctcgccgcacatcggccccgaggtagtgggcgccacctacggcgcgctcgatggccacgccagcccgcttcgcttgttgcgcgcgctggtggagggcttccagttgcgcggcggcgagcacgtgtccggcgtgcgctgcgagcgcatcgaacaccgcggcggtgcgttccatgtgtgggccaacggcaccgagcatgtggccgcgcgcctggtgctggccgcaggcctgggcaaccgcgcgttggcgcccatggtggggctcaacgcgccggtcgagcccaaccggggccagatc

SEQ ID NO: 143 - DNA, 495 bp, Acidovorax sp.
  misc_feature 1..495: note = Marker nucleic acid sequence
  source 1..495: mol_type = genomic DNA
gatggcgtcggcagcttgtgcgaaggtgaagccgcgattgagctgcgcacggtaggtgacccggggtacgtccgcagagcacagcgttggcagagcatcggccggcgcttctagtgcggctctccggctgccgcttactgcactgctgatggcgtcgaaccacgggtcgcttgcgagcgtctctagaggcaccgccaggcgttggcgccagttggggtaccgatcttcagtggtcccgggcacgttgagctgttcgcgctggcccgctaggtcttctagctggactcccaacagttggcacggagtccgggccagataggcatgcactgctgctgcaagcaggggtgtcatttcaggggccgactgtgcgtcaaccgttacaccttcaggcagtagctgttcagcgtccagcgccgcaagcagatgcgtgcgatcctgcgcccgagtcagctgcgcctgtacataggcatcgccatcagagagccatcccaacgc

SEQ ID NO: 144 - DNA, 498 bp, Acidovorax sp.
  misc_feature 1..498: note = Marker nucleic acid sequence
  source 1..498: mol_type = genomic DNA
taccaggggcagcacgccccagaagcccacgcccgtggtgttcgaccccgcgtatgcacccaaggtgggtgagctggccgccaacgggccgctcacgcgccagacgctcacggcccgggtgcagatcgacgccgaccatctggccagcgccgccaagggcaacgccttcctcgtggccctggccccgaacggacagatctacacctacaacggatcgaccttcgtgagcatcaacctgctcacccctatcgcggcctggaccaccagcctgcagaaccagagctcggtgctgttctccgagcaggacctgtcggcccttgccggcaccatgctcttcgtcggctacggcctgggcgtggggccatcggaaagcctgaccgatatgctggcggcaaagcgctaccagctggtccataccatccggtgacggacggtggccggctaaggaacaaggcccgcgcaagcgggcctttttttgtgaccacgccgcgctgcatc

SEQ ID NO: 145 - DNA, 500 bp, Acidovorax sp.
  misc_feature 1..500: note = Marker nucleic acid sequence
  source 1..500: mol_type = genomic DNA
ctactttccggtggcgctggagctgcccacctcgcgcgcggtggtcgagtccatcctgcgcaacgcggtggacctcaacacccgctacccggaccactcgggctgcctgggcatcaatggcgtgctggccggctcggacgatgctgagcccgtgcggcgcgcactgatcgacgcgcgtgccaacggcgagaccgcgctgcgcgcgcgcctggagcgcgcccagcaagagggcgacctgccgcccacggccaactgcgcggcgctggccacgtatgtgtgcgcggtgctgcacggcatggcggtgcaggccaaggcaggcttcagccgcgaggtgctgaacgcggtggtggaccaggccttgtcgacctggccgaccgcgcgctgatggtggtgccggggcggcggcgggcctggcccctgccgcgccggacaacatgtccagtgcggcgcccatggaacccgatacgatgaatttccccctctccatcgccacggttcaa

SEQ ID NO: 146 - DNA, 474 bp, Pseudomonas sp.
  misc_feature 1..474: note = Marker nucleic acid sequence
  source 1..474: mol_type = genomic DNA
tttttttcgccgccatgaagaacgccggcagccaccgcgtgcgcgactcggcaatacgactgacgctgcttacgtcatgcaccgaggtgaatggcctggccgggcatggcgatacagctggttattggttgaaacgtggggagatggcgcgcagattcactctatgcgtccgagggacgataaaggacattcaatgtcaggagccgaagacctccggaaacgaaggccttcgcggaaagaatgtgaaatccgctatccagtcaccgtgaagcgacccctggatatttgccgcagagtccattccaaccatttgccacgcaggcaaattagcacgggcggtatttgtacaagagccaacttaaggctcatacagatcggtactttagtgctggttattcatgatccagcccgccagggactcggtgttcccaagaacaccgagccatctggttggaggctgctcaagcttttttt

SEQ ID NO: 147 - DNA, 497 bp, Pseudomonas sp.
  misc_feature 1..497: note = Marker nucleic acid sequence
  source 1..497: mol_type = genomic DNA
atcagggcgcttgagacgccggaagaaccgagccgtcccggtttgcttcaacggttgttcggcggccacgatcactctgaagcgacacccgcgcccgcgccgacacctgaagccgaagcggccccgctgccctccccaccccaggcaacggatacggcagccgtcgcgccgacgccggtatccacagcggaacaagtccacgcacaggacaggactcccgacccgctggtgtccattgaggcggtagacgagcctgatccggcaccggcaccggcaccggcaccggcaccggcaccggcaccagccgtgtcgcctgcccagccgagcatcgtgtcggcgcctaccctcgatgaacccaccgagccggcccccgctgcccagaatcccgacgagctgacgccagaggaaccgccccagccgatcctcgaggctacagccgttccggaagaaccggtcgagcttcccgcagcggtcgttccggatgagtctccctacaa

SEQ ID NO: 148 - DNA, 467 bp, Pseudomonas sp.
  misc_feature 1..467: note = Marker nucleic acid sequence
  source 1..467: mol_type = genomic DNA
cagcagattgtcgattttggtcatgggtcaatctccttcatcagaggccacgcgatacaccgtcgatgcgaccgcgccggggcacaaaacgaacgaccctggagaaatgcgcagcgctccgagcagacgatgagcggtcgcataagtggatgaaatgccgcttgattttccgctcatccggtcgcgacaaggattttcgaaccaagcgttggcgcgccggctcggagctacataacaccgccgcagcccaccgaaaacgaatcggtccttgcggctttcacggcggggtgaagtccaaatctgcctggagttttcgcgatgtgtgaatgtttcgttcagcctgtttcttccaaggattccctagcgttctttgcccaacgggacgcgttcggcgcccaacaaaacccaagcctgtcggccgacagtcttcacgccgcggcagctcctgcactgcatgatcgacaaag

SEQ ID NO: 149 - DNA, 493 bp, Pseudomonas sp.
  misc_feature 1..493: note = Marker nucleic acid sequence
  source 1..493: mol_type = genomic DNA
accgtgtggcacccggcgcattggccggccactgcctgctgatgcgtgaaaaaggctcgaccacccgcacgctcactacaacgctgctacgagaggctggcgttgcgattgggccgctgttggaaattggcagccgcgagtcgattcgcgaagccgtcctgcgcaacatcggcatcagcgtcatcgctcgtcatgaggtgccggagaacccgcagctcaaagtggtggagctggagggcgcgccattaatcgccgagtacctctattgcctgaaggagcgccgccaggctcggctgccttcggcgttcctgggcctggcacgggaaacggccaagtcctgagtcggctacgcaaatttgccgatggcactatcggcaggttttagccaactgcaatcaacccttcgtactgcctgcctaccatgaccctcgtcgagctgaccgctcatcgaggtaacgtcatgacaagaacacgctccgtagacatgcagata

SEQ ID NO: 150 - DNA, 430 bp, Pseudomonas sp.
  misc_feature 1..430: note = Marker nucleic acid sequence
  source 1..430: mol_type = genomic DNA
cggtctcatattgatacccccctgaacgacaaacggtggggttcgtcctatgaaccagcggcggatgtgcctgtgtgaggaagccgaacaagaccatcgaaaccatttaaacaggaatagttatcaacgacttacacatgatcatgcgttgctctcgagtccgtaggctgagtctaggccagcgtaacgcaacgccggtcctgcgcttgggcgttagttgacgcggcttggcacccgcaggaaggaggctttaaggagaactttaaaatcgaccagaaaaatcaatgagataacgttggtaaagggaaatgagtagcgggattacatcgctcctggctcgtcaattaatcgacgagcggcgtatcagcgttggtaaacacgatgatgacgtcaatttatcggcattattggcggcgttgtcccgtttcgc

SEQ ID NO: 151 - DNA, 469 bp, Bacillus subtilis
  misc_feature 1..469: note = Marker nucleic acid sequence
  source 1..469: mol_type = genomic DNA
tggtgtgaaaaggacgattacaatgaaatttgtaggtttaggactaattctagcaataattgaaggagttattggatactttttcagaggaagtgtatcttatgaaacagtatttggtacagtatcaatcattttaataggtatatccgttctaatttcaggtttagcagtaagtggagaccgtcagcgagcaaatcatcattctgaaacaaaagaacacagacagtttagaatcaaaaatactttaaacctcatgatcacagcaataccctctattgttgttcttattttcttactcagcacaaaataaaaaatcttaataaacgtgtttttgaacttgaagctagattgaactactgagtaaagttggcgacgtcgccaactatgagaaacggtatacatataccgatttgtcccaagattcgggtgatacgtaacaccgatatgaaaacggacgacgtcgtccgtt

SEQ ID NO: 152 - DNA, 443 bp, Bacillus subtilis
  misc_feature 1..443: note = Marker nucleic acid sequence
  source 1..443: mol_type = genomic DNA
atataacaatacaataaaaaatatttcttattatgtcatcgacccatcaaaaattttgatgctcacatcataacacataatggggttttaacattaagcgtatagtacatatacatcgagtagttaaaaacggcaaggaatctttaatctattgattaatactaaaaatataaatgcaaaaaatatgtataaaaaacattgattattataagtgatcaggttataatacaattatcaaatacaaaaaatatgtacataaacaggaggcggttaaaatgaatgcacaactttttaatctggagtctagacttgatgaattggaaaatgaaattaatacacaatactgtgagttagatactaatcttgatgctcttaaattcaatcgtattgagctggaatcacagcttgaaaaatttgagtttagtcttacaaatagattacaa

SEQ ID NO: 153 - DNA, 379 bp, Bacillus subtilis
  misc_feature 1..379: note = Marker nucleic acid sequence
  source 1..379: mol_type = genomic DNA
aattatcacggtagaatcttgcaaagaattcgaagtgggcgaagtatttaccgttacagagcgtaataggtggtatgacggtacaggaataagtgtctacgaaactggtattggactgtatcatcatgaataccgcgcactcaaaccgaccgacatcgttcacattgacggtcagcgctacgaaatggccgatcggaaggcaaaagtaggcgagaaagttattacgattactaaatgtgatatttactgtaaaggggagattggaactgttgggtatcaaagtccacctcgctatatttatgttcgatttgaaacgagggcagtcgcatggcgtgtcccacatgaagattaccgcgttcttgttccattagataaatgt

SEQ ID NO: 154 - DNA, 343 bp, Bacillus subtilis
  misc_feature 1..343: note = Marker nucleic acid sequence
  source 1..343: mol_type = genomic DNA
actcaatacttcatctaacattaaagagttatttaagtacaaaactttcatagtcttgatttccttgttcattacaatgtcaatttgtttatcttttagcgaaagaaataaatcaaatatttccacgttgtcctttctgtcttgaaagcaatatcgcttagtttcaagaactttctttccagaaagatagctccaactagtaaactcataaaggaatttaacaatcccttcaaatccattcattttcaaataatatgttatttcctccaccagcctttcattaaaataaaacttttatttagatctctaaatctcatcggctataatgaatccccagagacgt

SEQ ID NO: 155 - DNA, 269 bp, Bacillus subtilis
  misc_feature 1..269: note = Marker nucleic acid sequence
  source 1..269: mol_type = genomic DNA
taggcttaataagacttaatttcattttttccacccgaataagcctaaaaaccttgatattaaaggtttttacgataacgccctctatttactcccctgaaagaacagatttaccttgatatatcaggcattttctcatttatttgcgtagattacgattacctcttaagggggttatttaaaatccattgcaacacagattatctttccagagcggcttaataaaagtggctcttttattatttctgaaaggacgttttaaactagaa

SEQ ID NO: 156 - DNA, 500 bp, Curtobacterium sp.
  misc_feature 1..500: note = Marker nucleic acid sequence
  source 1..500: mol_type = genomic DNA
gctgtgccgatttcgttacgcgcggctcgttcgcttgttcgctcgttcgtcgttcggtgcgaggttccacgctcggtgacgggcgcgcgggctcgcacggagtgcgcaacctcgcaccgagccgacgcgcggtgctgcaccgtgcggtggtcgcgccgcccgccggccgggaggcccgtaccggccccgccccgcgcctcccgtccggtgtccggtcgcgtccgcgggcccgggtcgcctcgtgcgcgccggcccggcccgcagtccgctgcctgctgcccactgcccgcagcccgcggcccgctgtcgcgaaagcgacagtgtgccgccgaacgttcgcgccgatctgtcgctctcgcggaccggacgcagcgacaaaccgcagatgtgtcgctttcgcgggttggtccgccgccggtcaggcctcggtgcgcctcgggtcgctcggtgtcgtgcccgcgacggctgcggcggcggctgctgcggccgcgccctcgcga

SEQ ID NO: 157 - DNA, 497 bp, Curtobacterium sp.
  misc_feature 1..497: note = Marker nucleic acid sequence
  source 1..497: mol_type = genomic DNA
cgcgtggcgggcctcccgtccgcccggaaccaggttccggacaccgaaccacgcgatcgcgcggtgccgtgtccggagcctggttccgtcgtgcggtcgactcccggcatactgggcgcgtgccccggaaccgcaaccgtcccgtgatcaccggcgtcgcggccgtggtggccgccggtctcctcgccggcgggttgttcctgacaacacggcagggcgcggacgacccgaccatcggtgccggctcggcctcacggacgccgagcgccgcgccgaccgccgccggtgacggcaccgtcacgatcacccgtaccgggccggacatgcccggcagcaccgcgctcggccggtgcgacaccacgacccaggcggccgtcgcgcagtacgagaccgaggccctgggccgcgtcaccctgcagtgcggcaccgctgcccaggggtacgagcacatccgggtgcggcacaccgccgactggcaggacgtcgtcaccgggcac

SEQ ID NO: 158 - DNA, 496 bp, Curtobacterium sp.
  misc_feature 1..496: note = Marker nucleic acid sequence
  source 1..496: mol_type = genomic DNA
aggcccggtctggtcgttctgctggtccgtcatgccgccgacggtacgcagggggtcgctgcgggccgtccaggaggctgtcccccgttgcgcggagcggcctgcgcccgccggccgcaccactccagggccgcaggtgcgtgatcctcgtttgtcacggtccggtgacgggcaggctccgattcggtaacacctgtcgttctgttccgatcgaggccctaccgtcgaacggtgactcctcggaccctgctggcgctcggcgccgccgtgctggccttctcggccggtgcgctcgcgttcgacggcaccgccgggctcggggcagacgtggccgtggccgccgagacctcgcacgacgccgctccggtgcacgtgacgaaggcggaactccgacgggtggactcgatcgagctcgacgccgaggcactcgtgctccggaacggcgacgacaccgtggtcgagtcctcgatgcgcgactccggtctgaccgtgagcg

SEQ ID NO: 159 - DNA, 373 bp, Curtobacterium sp.
  misc_feature 1..373: note = Marker nucleic acid sequence
  source 1..373: mol_type = genomic DNA
gcgtatcgtcgacggacccgaaccgcaccgccgcgccacggaaggaccccctccccgcatgaccgtcaccgccgcatccgccaccgcagccgacgccaccgccctcgaacacctgctggggtccgaccaggtcctccgcgacccggagtcgctcgagcgctaccgccacgacgacgccgagtgggccgactccacggcaccgctcgccgtggtcctggcacgcagcaccgacgacgtcgtcaccgccgtccgctgggccgccgccgccggcctccgggtcgtcccccgcggtgccggcaccggcctgtccggcggcgccaacgcgatggccgactcgatcgtcgtgtcgctcgagcggatggaccgggtgctc

SEQ ID NO: 160 - DNA, 332 bp, Curtobacterium sp.
  misc_feature 1..332: note = Marker nucleic acid sequence
  source 1..332: mol_type = genomic DNA
atggagtgagccggccagaagcggccgacgacagtgtagagcccgatgcggtgagtgctccgcttcaggaccaacaatgcctgggtccggcccacattcagacggcggtttaggagtaacacgccagtctcgataaccggtggtgcaccgctacacgacagttgtcgccttcgacggcctccgttgcctactgccgcctgaccgggggtattaccgtatgcctgtcccgcaaaaatgcccggttacggcccggcggattctgatggtcgacgcaacagatggtcgttttagggctggattcagggtagctggagggcgctagctcggcgctt

SEQ ID NO: 161 - DNA, 488 bp, Paenibacillus sp.
  misc_feature 1..488: note = Marker nucleic acid sequence
  source 1..488: mol_type = genomic DNA
gttaggacttggggtcggatcagggtttggtgttggatctacaggtacaggattaggatctggaattgggttgggtgttggatctggtgttggagtagggtccggtgttggccctggatctttactataaaaaaagtcgatttcactgatgtttatagtttcatttgataatcccataaatgatacaaatctaacattttgttctaatggaattgtattgagttgcccactgaaagcactatcgttactatcgtttattccataagatcctaaataaccagtatcatgcccaaaaaaaactattcttgatactttggcatcgcttttaagtttaaaagaatctatttttttgatttcgcctagatcaattacaatcatcttgccagcaggcattgagtattttgtttcttcattattatctgtaacaagagatgtgttttcagcgcttgttgctccatatatatacattgcccttcccgtaatagctg

SEQ ID NO: 162 - DNA, 479 bp, Paenibacillus sp.
  misc_feature 1..479: note = Marker nucleic acid sequence
  source 1..479: mol_type = genomic DNA
agaatttaataaatcgattaataaaatacggaaaaggatagggtgtaggccccatccttgttccagcatgaagatattagaacgtataaaaatatcttcccgaaaatgagagagacgaactccatgttaagcctaaatcctgtacacctgttttccaaatatcaataacagcatctggcaggcttccattatcggctttataaaaagtataagcgacatcattgtcagtgtttcttacagagattttagtattaaacttcggattatcaatagctccttttgttgcgcaatcgcctctttgtagtgaattggaattttcacctgtagagtccgtaaagtttgtccctcttcctgtgccttgaaccttaccgctcgaagttccggtgatgacaatttcattattatgtgctccgtatgtataagtctcaggtgctttgcgtgttccgcgtggttccccaaatgaatactaggagcttgat

SEQ ID NO: 163 - DNA, 465 bp, Paenibacillus sp.
  misc_feature 1..465: note = Marker nucleic acid sequence
  source 1..465: mol_type = genomic DNA
gtttttctcttgaatcccttgattatcaagggattttttatttttagtgattgaaatcatgacttccatatcacagggagcgagcgcctttttcgctcttgggaacggattggggacgaacttttggatcgaagacatcgaggtgtgctgttgttttacgactaatctttttggtgaaatgagcatgggtgtatgaagtcacttgagatgtagaatgtcgcaatcgatgctgaatctccttgataggatgctccctagccaatggcaatgtgggctgaaggcggtgtaggtgtcgatatcggatacataactccgagtgatattagataagtatgctgattgaacaaaagtaagatttatcgtgaaataaaagcgaagactcaaccagtataatagctggtatgagtccttttttatatccaataaaaaataaatatgcaaatatatagattatatttatagatc

SEQ ID NO: 164 - DNA, 450 bp, Paenibacillus sp.
  misc_feature 1..450: note = Marker nucleic acid sequence
  source 1..450: mol_type = genomic DNA
tttcaaactttctttttatggtaatttgtggtggtttcagactttttatttttcgtgtttatcacgtgctctggcaacgcagtaaaatcaacaaaattggttcacgacttttttatcacctgacaaactattgtttagttacattaaagttggtacctttgtacatcgggcttttttattaaattcagaggctactgctttggctcaatcagtgcgtagtatagttacatgaatcctttcctgtattggtgttttaaagtaattgaagcagatgaattccaatcacctataaacgtatggggtaaactgaggagttattaaatccctgattatattcaagctgcgcatcgatgatcgccagctttgaatagatttccggtggttttctttatgtccggaacatggctgactcaatgaatcatcaaaaaaaaacagcccctacagggctgc

SEQ ID NO: 165 - DNA, 356 bp, Paenibacillus sp.
  misc_feature 1..356: note = Marker nucleic acid sequence
  source 1..356: mol_type = genomic DNA
cctttttttgcaataatttcgcttacaggaatgttgcagctggatttactaataactttccagctattgcttgtaagcttttcagattgcagacctcattaggatgaaaacgctgagtatgtagttatttaatattctctttgtataacaacccaatgcagatagcgggacttgtaaaaaatgttttcctgatgacagcgtctacaaacaccaaattgctatgcgtcacatacatcttcacttattttggaccagtaatttacagcgttctactatagagggtatcttcttaaattcgtttttctaaaggctgcctgttccggctaagaaatgaagcatctcctgtccaggagatg

SEQ ID NO: 166 - DNA, 454 bp, Bacillus sp.
  misc_feature 1..454: note = Marker nucleic acid sequence
  source 1..454: mol_type = genomic DNA
tgaattataaatgttaattgtagaaggtgtagagaaggcttataagacaggtgggttattttctagaaaaaagcgaaaaatattaaaaaatattagttttgaatgtaaaagtggggagtgcctaggaattattggagaaagtggaagtggaaaatcaacattaggtcgtctattaataggtattgaacaacctgatgttggaagagttttgtttgaaggaggaaatgtgaatgatagagtaactagatgtgggcgtattagtgctgtattccaaaactatacatcttccattaacccatttttcactgtaaagcaggccattctggagcctctaaaaattaagaaaaagaccaaaatagaaattgaaaataagattgattacctcttggatcaagtagggttaggttcatcgtataaagagaaatatcctcatgagctatcaggagggcaagta

SEQ ID NO: 167 - DNA, 446 bp, Bacillus sp.
  misc_feature 1..446: note = Marker nucleic acid sequence
  source 1..446: mol_type = genomic DNA
agcggcaaagtacatacatactgcaaaaaccaacaatcccccaatagctagggaacctctagctatcatcctactttttcctttctttactaaataatcagaaatggcccctcccgtcattacagtaataaagatacagagccaaggtaagcttgcagcaaatcccatgctacttaacgtaaattgcctagcttctaaaagatacgtaggaagccaaaccaaaaagaaagtaacaatgtatagaacaacaaagtactgaatacctagtgcccaaaaacgtccgttcttcaagaactttttccaaggagctacttttttttcttttgcttggactgtacggttagacaaaattaaattcagttcttctttactaatccaagaatgttcttcaggcttgtctcttcccatcacataccaaattcctgcaattactatcccaatcaaac

SEQ ID NO: 168 - DNA, 479 bp, Bacillus sp.
  misc_feature 1..479: note = Marker nucleic acid sequence
  source 1..479: mol_type = genomic DNA
acctatagggaccgttgttatcttcttatctcttaccatggcctctagtttttcagaacaaatggaagaaggattcattacggaaatcgtttctatcgttatgtttgtcattattcctttactcatgctcattgtctccattagccgtcagtattttaagaagagattaagttcccaataatttttttactacctttaacatgttttatgtaaactacaattgtataacctgtacataacctttttatactaaaatgtattaataaaggtggaatcgaagattacttacaggtggcttaaagtttttgcaccagaaccgttcatttcaaaatcaatttctacgagatataataaatactgattgttaaattatgataattataaatggcgagaggtaaagtttagtagtcctatagaagggcgataaaatcctattatatccattttgcgaaaaataattaaaaaggaggggggaatta

SEQ ID NO: 169 - DNA, 364 bp, Bacillus sp.
  misc_feature 1..364: note = Marker nucleic acid sequence
  source 1..364: mol_type = genomic DNA
atccaaatgctaagactgttatatagatgtttgtaaatgacaataaaagttgtgcccctcccattacgcaacaagcaaacaatagaatgaggatgtgctttttataccgtttaattatcctttttataaatatccctgcaactaatatacttgtaccttctacaaaatacaggactcccaccataaaacctggttggcctttccctacttcaatcacaaataaattgaagcctgaaataaaaatgagaggaataatagatatgactagcacaacttttatagcatgatttactaggataataggaaagatctctttaaatttagtgttagtttttttactatttaccggccatccttcgggaat

SEQ ID NO: 170 - DNA, 441 bp, Bacillus sp.
  misc_feature 1..441: note = Marker nucleic acid sequence
  source 1..441: mol_type = genomic DNA
cataatggaagctaacaaaggaggaaatacagatgattaatggagaaaagaaaattaaacaaccaattcgctgggcaatggtagggggaggacgtggaagtcaaatcggctacatccatcgatcctctgctcttagagaccataacttccaacttgttgcaggtgtttttgatattgatcctgtgagaggaaaagaatttggaatcaacattcatgttgatcctgagcgttgttatcaagattatcaaacgctatttcgagaagaagcaaagcgagaagacggtattcaagcggtttccattgcaactccaaatggaacacactatgaaatatgcaaggcggcgttaaatgcaaatcttcatgttgtatgtgagaaacccctttgctttacaacaaaagaggcagaagaattagaatcactttcaaaagaaaaaaatcgaa

SEQ ID NO: 171 - DNA, 430 bp, Bacillus sp.
  misc_feature 1..430: note = Marker nucleic acid sequence
  source 1..430: mol_type = genomic DNA
catagtgggttcgtagagccccaatctcttaactttaggcaaaattcagagggaatttcaaaaggggttcagaattttttaaatccgaaccccttttgtctacaaactgaaatcacattgacttatctggtacaagataataagaaaaaaagtgatggaggaaaaggaactattagtgtggtctattgtgaacaattctttaacgatagaacttttcacaactgctcccttccgtgtcaaaactcaagacatgatccccacccaagttttcacagccgtcgctaatatcaataaagccagtatgacttgcagcagttttacattcatttttttaccggccatcgccccaagaggagaggccattaaactcgctgccaccatgatcatagcaggatagaagtcaacttgacctgttgagattttccctgct

SEQ ID NO: 172 - DNA, 364 bp, Bacillus sp.
  misc_feature 1..364: note = Marker nucleic acid sequence
  source 1..364: mol_type = genomic DNA
acgagggatgattttgaaatcgcggcggatgccattgcaactggcatgtttgatacctcattgtttatttcaaagatattacccatcgaagaggccaagactggtatgaagattgttgatgagaagctcgaagatgtgataaaggtattattaaaattttaatgatttaatccttcatagtttctatgaaaataacaaaaagttaaaattgttctacaacagtaagaagaattttccaatataagaggtagataaaattgtaaacgtttactccgctatattgctataactatgaccaatgtacaataaatagtccggaactaaggagttgtttaggatgaatgcacatcaattagaacaatct

SEQ ID NO: 173 - DNA, 433 bp, Bacillus sp.
  misc_feature 1..433: note = Marker nucleic acid sequence
  source 1..433: mol_type = genomic DNA
tagaaacagtaatccaaaaaataaaactaaactaacaaaaccgacaccacgcgaaatcggaaaatgaacgttagattcataactttcgtcgtgtcgtttataaattagaaaaccaataaatgcggccagtataataataccaacttgcacataggcagtctgccaaatcaaggtcccaaccaaggctattaatgcaattgtctttctctttatatctggagttaaattttttgacatccccaaaatggcgtgtgcaactactgctactgctactatttttaatccgtggatccagcctgcatttgaaacatccattcctttgaaaaatgatgctaatattactaacgctatcaccgaaggcagtgtaaaaccaaggaaagctaaaattccaccgaagaaacctccccgcataactccgactccaattccaacc

SEQ ID NO: 174 - DNA, 472 bp, Bacillus sp.
  misc_feature 1..472: note = Marker nucleic acid sequence
  source 1..472: mol_type = genomic DNA
atttatcgccccgtttttaatgggatatatgattgaaagcagcggtggttcttacgattcatctttcatattaatgattgcagccatcattgtagcggcaatcatcgcccttacgattggcaatgataccgaaaaagaagattcattaaattcagaaacaatagtggaagcctaatttgaattgccaatttatcaggaagtaaatggattcatttatctttgttgagaatgtttttttacatggtaatagcattatatttagaaaacccttgttgataagaggctatcagatgccgaatcctcgtacattgaaatacagacgctatttttcatatagtgggtaagaaaaaggggggggagatgttgcaattttcagaaaagatattaaagttaaaggaaacatcgttgcttattaggtaacaaaaagggcgtgaatgaacgaaataagttaaatcatctttaagggagtttg

SEQ ID NO: 175 - DNA, 426 bp, Bacillus sp.
  misc_feature 1..426: note = Marker nucleic acid sequence
  source 1..426: mol_type = genomic DNA
gtaggtaaacgatatttagtaacaccgcgccaaatagataaaaaaatccttaaggagactccacagcctcaacagcaaggtaagtatgatggcgaaaagatagcgcctagaaaaaaagccgaattagcccaaaaagcccttatttatatgcaacagctacaacagcttcaagggtttcaagagcttccacagctacaacaacttaaacagtttccgcagcttcagcagcttcaacggcaaactaaagaaaaagtcaaagatgaacttgtagcatctaataaacatgaaaaaaaagctaaagtacaacagagagctaaagatgatgatgaaaaaatagcttctcataaaaaagaaaaaaaggctcataaagccgaaaaaatcaaaaaagccctttatcaaattcaaaagttgcaacaaaaggccata

SEQ ID NO: 176 - DNA, 20 bp, synthetic construct
  misc_feature 12: note = n is a, c, g, or t
  misc_feature 1..20: note = 16S primer
  source 1..20: mol_type = other DNA
agagtttgatcntggctcag

SEQ ID NO: 177 - DNA, 22 bp, synthetic construct
  misc_feature 6: note = n is a, c, g, or t
  misc_feature 1..22: note = 16S primer
  source 1..22: mol_type = other DNA
tacggntaccttgttacgactt

SEQ ID NO: 178 - DNA, 19 bp, synthetic construct
  misc_feature 9: note = n is a, c, g, or t
  misc_feature 1..19: note = 16S primer
  source 1..19: mol_type = other DNA
gtgccagcngccgcggtaa

SEQ ID NO: 179 - DNA, 20 bp, synthetic construct
  misc_feature 11: note = n is a, c, g, or t
  misc_feature 15: note = n is a, c, g, or t
  misc_feature 1..20: note = 16S primer
  source 1..20: mol_type = other DNA
ccgtcaattcntttnagttt

SEQ ID NO: 180 - DNA, 20 bp, synthetic construct
  misc_feature 1..20: note = IS33394_2_NF2
  source 1..20: mol_type = other DNA
atttgcgactgaaagagggg

SEQ ID NO: 181 - DNA, 20 bp, synthetic construct
  misc_feature 1..20: note = IS33394_NES_F4
  source 1..20: mol_type = other DNA
cggcggatgggtaaagaaaa

SEQ ID NO: 182 - DNA, 20 bp, synthetic construct
  misc_feature 1..20: note = IS33395_1_NF1
  source 1..20: mol_type = other DNA
gagcacgagcagaaataaca

SEQ ID NO: 183 - DNA, 22 bp, synthetic construct
  misc_feature 1..22: note = IS33395_F1
  source 1..22: mol_type = other DNA
aacttcgggtattcatcacctg

SEQ ID NO: 184 - DNA, 22 bp, synthetic construct
  misc_feature 1..22: note = IS33395_R1
  source 1..22: mol_type = other DNA
gtagagtagagcgtcaacttgg

SEQ ID NO: 185 - DNA, 18 bp, synthetic construct
  misc_feature 1..18: note = IS33398_2_NF1
  source 1..18: mol_type = other DNA
atctgcaatacgccttct

SEQ ID NO: 186 - DNA, 22 bp, synthetic construct
  misc_feature 1..22: note = IS33398_EXT_F4
  source 1..22: mol_type = other DNA
cgacttcttcacttactctccg

SEQ ID NO: 187 - DNA, 22 bp, synthetic construct
  misc_feature 1..22: note = IS33398_EXT_R4
  source 1..22: mol_type = other DNA
gtttatgagcgctttcttggac

SEQ ID NO: 188 - DNA, 18 bp, synthetic construct
  misc_feature 1..18: note = IS33398_NES_F4
  source 1..18: mol_type = other DNA
cggaatgagaggggcaat

SEQ ID NO: 189 - DNA, 19 bp, synthetic construct
  misc_feature 1..19: note = IS33402_2_NF2
  source 1..19: mol_type = other DNA
tgaaaggacttaacgatgg

SEQ ID NO: 190 - DNA, 22 bp, synthetic construct
  misc_feature 1..22: note = IS33402_F1
  source 1..22: mol_type = other DNA
gaacttcagatgccattcaagc

SEQ ID NO: 191 - DNA, 22 bp, synthetic construct
  misc_feature 1..22: note = IS33402_F2
  source 1..22: mol_type = other DNA
aacacgagattgatacctgctc

SEQ ID NO: 192 - DNA, 22 bp, synthetic construct
  misc_feature 1..22: note = IS33402_F4
  source 1..22: mol_type = other DNA
atgtctcgtgtaaaggatgtgg

SEQ ID NO: 193 - DNA, 22 bp, synthetic construct
  misc_feature 1..22: note = IS33402_F5
  source 1..22: mol_type = other DNA
aattgcatggcgtcaataacag

SEQ ID NO: 194 - DNA, 22 bp, synthetic construct
  misc_feature 1..22: note = IS33402_F6
  source 1..22: mol_type = other DNA
acaagccaatcagatacccttc

SEQ ID NO: 195 - DNA, 22 bp, synthetic construct
  misc_feature 1..22: note = IS33402_F7
  source 1..22: mol_type = other DNA
ctatcagcatctccgccttatc

SEQ ID NO: 196 - DNA, 18 bp, synthetic construct
  misc_feature 1..18: note = IS33402_NES_F4
  source 1..18: mol_type = other DNA
gtaaaggatgtggtgcgt

SEQ ID NO: 197 - DNA, 22 bp, synthetic construct
  misc_feature 1..22: note = IS33402_R1
  source 1..22: mol_type = other DNA
gtcacgcttccttgttatttcg

SEQ ID NO: 198 - DNA, 22 bp, synthetic construct
  misc_feature 1..22: note = IS33402_R2
  source 1..22: mol_type = other DNA
gctctgtgactgcattgaattc

SEQ ID NO: 199 - DNA, 22 bp, synthetic construct
  misc_feature 1..22: note = IS33402_R4
  source 1..22: mol_type = other DNA
tcctcgtacaaagtatcttgcg

SEQ ID NO: 200 - DNA, 22 bp, synthetic construct
  misc_feature 1..22: note = IS33402_R5
  source 1..22: mol_type = other DNA
ggttccttgcttcctagtgtag

SEQ ID NO: 201 - DNA, 22 bp, synthetic construct
  misc_feature 1..22: note = IS33402_R6
  source 1..22: mol_type = other DNA
gtcaattacctgcgaacaagtg

SEQ ID NO: 202 - DNA, 22 bp, synthetic construct
  misc_feature 1..22: note = IS33402_R7
  source 1..22: mol_type = other DNA
cagacaagcatctttcaagcag

SEQ ID NO: 203 - DNA, 22 bp, synthetic construct
  misc_feature 1..22: note = IS33441_F2
  source 1..22: mol_type = other DNA
tccaccatccgatgttaagttc

SEQ ID NO: 204 - DNA, 22 bp, synthetic construct
  misc_feature 1..22: note = IS33441_F3
  source 1..22: mol_type = other DNA
ggttatgtggcatcaatggttg

SEQ ID NO: 205 - DNA, 22 bp, synthetic construct
  misc_feature 1..22: note = IS33441_F4
  source 1..22: mol_type = other DNA
aatcagcttcccatgttctctc

SEQ ID NO: 206 - DNA, 22 bp, synthetic construct
  misc_feature 1..22: note = IS33441_F5
  source 1..22: mol_type = other DNA
aaccatcaaatctacttcccgg

SEQ ID NO: 207 - DNA, 22 bp, synthetic construct
  misc_feature 1..22: note = IS33441_F6
  source 1..22: mol_type = other DNA
tacgaagggaagtttatggcag

SEQ ID NO: 208 - DNA, 22 bp, synthetic construct
  misc_feature 1..22: note = IS33441_F7
  source 1..22: mol_type = other DNA
tggtcaaacgtttaatgttggc

SEQ ID NO: 209 - DNA, 22 bp, synthetic construct
  misc_feature 1..22: note = IS33441_R2
  source 1..22: mol_type = other DNA
catgttagtgattccggtttgc

SEQ ID NO: 210 - DNA, 22 bp, synthetic construct
  misc_feature 1..22: note = IS33441_R3
  source 1..22: mol_type = other DNA
gagtcgtgggttgttctagatc

SEQ ID NO: 211 - DNA, 22 bp, synthetic construct
  misc_feature 1..22: note = IS33441_R4
  source 1..22: mol_type = other DNA
gaattactcgaaacaccttgcg

SEQ ID NO: 212 - DNA, 22 bp, synthetic construct
  misc_feature 1..22: note = IS33441_R5
  source 1..22: mol_type = other DNA
aatacaggtggcaagatggtac

SEQ ID NO: 213 - DNA, 22 bp, synthetic construct
  misc_feature 1..22: note = IS33441_R6
  source 1..22: mol_type = other DNA
gttctgatttctgcacacgatg

SEQ ID NO: 214 - DNA, 22 bp, synthetic construct
  misc_feature 1..22: note = IS33441_R7
  source 1..22: mol_type = other DNA
atcctgcctgataaagttccac

SEQ ID NO: 215 - DNA, 22 bp, synthetic construct
  misc_feature 1..22: note = IS5006_F2
  source 1..22: mol_type = other DNA
gtttcgattgcagtaaagcctc

SEQ ID NO: 216 - DNA, 22 bp, synthetic construct
  misc_feature 1..22: note = IS5006_F3
  source 1..22: mol_type = other DNA
caggagcgaactaagagaactc

SEQ ID NO: 217 - DNA, 22 bp, synthetic construct
  misc_feature 1..22: note = IS5006_R2
  source 1..22: mol_type = other DNA
ctcaacgacatctttgccattc

SEQ ID NO: 218 - DNA, 22 bp, synthetic construct
  misc_feature 1..22: note = IS5006_R3
  source 1..22: mol_type = other DNA
gaaacgaatcaaacgcaggtag

SEQ ID NO: 219 - DNA, 22 bp, synthetic construct
  misc_feature 1..22: note = IS5021_F1
  source 1..22: mol_type = other DNA
aacataaaccctgctctgatcc

SEQ ID NO: 220 - DNA, 22 bp, synthetic construct
  misc_feature 1..22: note = IS5021_F2
  source 1..22: mol_type = other DNA
atcccacacaagatggatcaag

SEQ ID NO: 221 - DNA, 22 bp, synthetic construct
  misc_feature 1..22: note = IS5021_F4
  source 1..22: mol_type = other DNA
atgtaatgagcaacaggtctcc

SEQ ID NO: 222 - DNA, 22 bp, synthetic construct
  misc_feature 1..22: note = IS5021_F5
  source 1..22: mol_type = other DNA
aataggaggtgcagtggaaatc

SEQ ID NO: 223 - DNA, 22 bp, synthetic construct
  misc_feature 1..22: note = IS5021_F6
  source 1..22: mol_type = other DNA
ataattcccgtccttgactgtg

SEQ ID NO: 224 - DNA, 22 bp, synthetic construct
  misc_feature 1..22: note = IS5021_F7
  source 1..22: mol_type = other DNA
gattgacgttgtgctattggtg

SEQ ID NO: 225 - DNA, 22 bp, synthetic construct
  misc_feature 1..22: note = IS5021_R1
  source 1..22: mol_type = other DNA
gtcaacatgccgtcaaatacag

SEQ ID NO: 226 - DNA, 22 bp, synthetic construct
  misc_feature 1..22: note = IS5021_R2
  source 1..22: mol_type = other DNA
aatgcctgtcttctgattctcc

SEQ ID NO: 227 - DNA, 22 bp, synthetic construct
  misc_feature 1..22: note = IS5021_R4
  source 1..22: mol_type = other DNA
cacatcgtcaaattcactcacg

SEQ ID NO: 228 - DNA, 22 bp, synthetic construct
  misc_feature 1..22: note = IS5021_R5
  source 1..22: mol_type = other DNA
tgtcgataccaggaaattcacc

SEQ ID NO: 229 - DNA, 22 bp, synthetic construct
  misc_feature 1..22: note = IS5021_R6
  source 1..22: mol_type = other DNA
gcagcatttccagataaccaac

SEQ ID NO: 230 - DNA, 22 bp, synthetic construct
  misc_feature 1..22: note = IS5021_R7
  source 1..22: mol_type = other DNA
cggtgacaaacaatgacttacg

SEQ ID NO: 231 - DNA, 22 bp, synthetic construct
  misc_feature 1..22: note = IS6635_F1
  source 1..22: mol_type = other DNA
gtcgttgcacagatgattgaag

SEQ ID NO: 232 - DNA, 22 bp, synthetic construct
  misc_feature 1..22: note = IS6635_R1
  source 1..22: mol_type = other DNA
ggcaaattaacagttccgctac

SEQ ID NO: 233 - DNA, 22 bp, synthetic construct
  misc_feature 1..22: note = IS8941_F3
  source 1..22: mol_type = other DNA
tgctaacagatccatttccagg

SEQ ID NO: 234 - DNA, 22 bp, synthetic construct
  misc_feature 1..22: note = IS8941_R3
  source 1..22: mol_type = other DNA
gtcttatgctcgagtttgttgc